European Patent Application EP 4 242 330 A2, published September 13, 2023. Title: Generating Northern Leaf Blight Resistant Maize. Applicant: PIONEER HI-BRED INTERNATIONAL, INC. The sequence listing filed with the application follows.

SEQUENCE LISTING (90 sequences)

SEQ ID NO: 1 - DNA, 21 bp, Zea mays
  source 1..21: mol_type = genomic DNA
gatgggtcctgcgctcgatgt

SEQ ID NO: 2 - DNA, 20 bp, Zea mays
  source 1..20: mol_type = genomic DNA
gctcggtgtacttgtcaacg

SEQ ID NO: 3 - DNA, 20 bp, Zea mays
  source 1..20: mol_type = genomic DNA
gctagcgagcttgtcgagtg

SEQ ID NO: 4 - DNA, 4296 bp, Streptococcus pyogenes
  source 1..4296: mol_type = genomic DNA
atggataagaagtacagcatcggcctcgacatcgggaccaacagcgtcggctgggccgtcatcaccgacgaatataaggtgcccagcaagaagttcaaggtgctcgggaatacagaccgccacagcatcaagaagaacctgatcggcgccctcctgttcgactcgggcgagaccgctgaggccaccagactaaagaggaccgctcgccgccgctacacccgccgcaagaaccgcatatgctacctccaggagatcttcagcaacgagatggccaaggtggacgacagcttcttccaccgccttgaggagtcgttcctcgtggaggaggacaagaagcatgagaggcacccgatcttcgggaacatcgtggacgaggtaagtttctgcttctacctttgatatatatataataattatcattaattagtagtaatataatatttcaaatatttttttcaaaataaaagaatgtagtatatagcaattgcttttctgtagtttataagtgtgtatattttaatttataacttttctaatatatgaccaaaacatggtgatgtgcaggtggcgtaccacgagaagtacccgacgatctaccacctccgcaagaagctggtcgactccacagacaaggccgacctcagactgatctacctggccctcgcgcacatgatcaagttccgcgggcacttcctcatcgagggcgacctgaacccggacaactccgacgtcgacaagctcttcatccagctggtccagacctacaatcaactgttcgaggagaacccgatcaacgcgtccggcgtggacgcgaaggccatcctcagcgcgaggctcagcaaatcaagacggctggagaacctgatcgcccagctcccaggcgagaagaaaaacggcttgttcggcaacctgatcgcgctctcgctcggcctcacgcccaacttcaaatcaaacttcgacctggccgaggacgcgaaactgcagctgtccaaggacacttacgacgacgacctcgacaacctgctggcgcaaatcggtgaccagtacgcagacctcttcctggccgccaagaacctctcggacgccatcctgctgtccgatatcctgagagtgaatacggagatcaccaaggcgccgctcagcgcctccatgattaaaaggtacgacgagcaccaccaggacctgacgctgctcaaggccctggtgcgccagcagctccccgagaagtacaaggagatcttcttcgaccaatcaaaaaacggctacgccggctacatcgacgggggcgcctcccaggaggagttctacaagttcatcaaaccaattctcgagaagatggacggcacggaggagcttctcgtgaagctcaaccgggaggacctcctgaggaagcagaggacgttcgacaacggctcgataccgcatcagatccacctgggcgagctccacgccatcctgcgccggcaggaggatttctatccgttcctcaaggacaacagggagaagatcgagaaaattctgacgttccgcatcccgtactacgtgggccctctcgcgcgcgggaacagccggttcgcctggatgactcggaagtcggaggagacgatcacgccgtggaacttcgaggaggtggtggacaagggcgcctccgcccagtcgttcatcgagcgcatgacgaacttcgataaaaatctgcccaatgaaaaagtgctcccgaagcacagcctcctctacgagtacttcacggtgtacaacgagctcacgaaggtgaagtacgtgaccgagggtatgcggaagccggcgttcctgagcggcgagcagaagaaggccatcgtggacctcctcttcaagacgaaccggaaagtcaccgtgaagcaattaaaggaggactacttcaagaaaatagagtgcttcgacagcgtcgagatctcgggcgtcgaggacaggttcaacgcgtcgctgggcacataccacgacctcctcaagatcattaaagacaaggacttcctggacaacgaggagaacgaggacatcctcgaggacatcgtgctgaccctcaccctgtttgaggaccgggagatgatcgaggagcgcctcaagacgtacgctcaccttttcgacgacaaggtgatgaaacagctgaagcggcgccgctacaccggatggggccggctctcccgcaagctcattaatgggatcagggacaagcagtccggcaagaccatactcgatttcctgaagagcgacggcttcgccaaccggaacttcatgcagctcatccacgacgactccctcactttcaaggaggacatccagaaggcccaggtcagcggacagggcgactcgctccacgaacacatcgccaacctggccgggtcgcctgcgattaaaaagggaatccttcagaccgtcaaggtcgtggacgagctggtgaaggtgatgggcaggcacaagcccgaaaatatcgtcattgagatggcccgggagaaccagaccacgcagaaaggccagaagaacagccgggagcgcatgaaacggatcgaggagggtatcaaggagctgggctcgcagatcctcaaggagcaccctgtggaaaatacccagctgcagaatgaaaagctctacctctactacctccagaacggccgcgacatgtacgtggaccaggagctggacattaatcgcctctcggactacgacgtcgaccacatcgtcccgcagtccttcctgaaggacgacagcatcgacaacaaggtcttgacccgctccgataaaaatcgcgggaagtccgacaacgtgccgtcggaggaggtggtcaagaagatgaaaaactactggcgccagctgctcaacgccaagctaatcacgcagcgcaagttcgacaacctcaccaaggccgaacgcggcggtctctccgagcttgataaggctgggttcatcaagagacagctggtggagacccggcagatcaccaagcatgtcgcccagatcctggactcgcgcatgaatactaagtacgatgaaaacgacaagctcatccgcgaggtgaaggtgatcaccctgaagagcaagctggtctcggacttccggaaggacttccagttctacaaggtccgggagatcaacaactaccaccacgcgcacgacgcctacctgaacgcggtggtgggcacagcccttataaagaagtaccctaagctcgagtccgagttcgtgtacggcgactacaaggtgtacgacgtccgcaagatgatcgcgaagagcgagcaggagatcgggaaggccaccgcaaaatacttcttctactccaacatcatgaacttcttcaagaccgagatcaccctggccaacggggagatccgcaagcgcccgctgattgagacgaacggagagacaggcgagatagtctgggacaagggcagggacttcgccaccgtgcgcaaggttctgtccatgccgcaggtgaacatcgtgaagaagactgaggtgcagacaggcggcttctcgaaggagtccatcctgcccaagcggaacagcgacaagctcatcgcgcggaagaaggactgggaccctaaaaaatatggcgggttcgactcgcccaccgtggcttactcggtcctcgtggtggccaaggtcgagaagggcaaaagcaagaagctgaagagcgtcaaggagctcctcggcatcaccatcatggagcggtccagcttcgagaagaacccgatcgacttcctcgaggcgaagggatataaggaggtgaagaaggacctcatcattaaactgccgaagtactcgctattcgaactggagaatggtcgcaagaggatgctcgcgagcgctggcgagctgcagaaagggaacgagctggctctcccgagcaagtacgtcaacttcctctacctggcctcccactatgaaaagctcaagggctcgccggaggacaacgagcagaagcagctgttcgtcgagcagcacaagcattacctcgacgagatcatcgagcagatctcggagttcagcaagcgcgtgatcctggccgacgccaacctcgacaaggtgctgtccgcatataacaagcaccgcgacaaaccaatacgggagcaggccgaaaatatcatccacctgttcaccctcacgaacctgggcgcccccgccgcgttcaagtacttcgacacaaccatcgaccgcaagcggtacacgagcacgaaggaggtgctggacgccacgttgattcaccagtccatcacgggcctgtatgaaacaaggatcgatctcagccagctcggcggcgactag

SEQ ID NO: 5 - protein, 9 aa, Simian virus 40
MAPKKKRKV

SEQ ID NO: 6 - DNA, 1000 bp, Zea mays
  source 1..1000: mol_type = genomic DNA
tgagagtacaatgatgaacctagattaatcaatgccaaagtctgaaaaatgcaccctcagtctatgatccagaaaatcaagattgcttgaggccctgttcggttgttccggattagagccccggattaattcctagccggattacttctctaatttatatagattttgatgagctggaatgaatcctggcttattccggtacaaccgaacaggccctgaaggataccagtaatcgctgagctaaattggcatgctgtcagagtgtcagtattgcagcaaggtagtgagataaccggcatcatggtgccagtttgatggcaccattagggttagagatggtggccatgggcgcatgtcctggccaactttgtatgatatatggcagggtgaataggaaagtaaaattgtattgtaaaaagggatttcttctgtttgttagcgcatgtacaaggaatgcaagttttgagcgagggggcatcaaagatctggctgtgtttccagctgtttttgttagccccatcgaatccttgacataatgatcccgcttaaataagcaacctcgcttgtatagttccttgtgctctaacacacgatgatgataagtcgtaaaatagtggtgtccaaagaatttccaggcccagttgtaaaagctaaaatgctattcgaatttctactagcagtaagtcgtgtttagaaattatttttttatataccttttttccttctatgtacagtaggacacagtgtcagcgccgcgttgacggagaatatttgcaaaaaagtaaaagagaaagtcatagcggcgtatgtgccaaaaacttcgtcacagagagggccataagaaacatggcccacggcccaatacgaagcaccgcgacgaagcccaaacagcagtccgtaggtggagcaaagcgctgggtaatacgcaaacgttttgtcccaccttgactaatcacaagagtggagcgtaccttataaaccgagccgcaagcaccgaatt

SEQ ID NO: 7 - DNA, 21 bp, synthetic construct
  misc_feature 1..21: note = Ht1-CR2 DNA version of guide RNA
  source 1..21: mol_type = other DNA
gatgggtcctgcgctcgatgt

SEQ ID NO: 8 - DNA, 20 bp, synthetic construct
  misc_feature 1..20: note = Ht1-CR4 DNA version of guide RNA
  source 1..20: mol_type = other DNA
gctcggtgtacttgtcaacg

SEQ ID NO: 9 - DNA, 20 bp, synthetic construct
  misc_feature 1..20: note = Ht1-STH1-CR1 DNA version of guide RNA
  source 1..20: mol_type = other DNA
gctagcgagcttgtcgagtg

SEQ ID NO: 10 - DNA, 37 bp, synthetic construct
  misc_feature 1..37: note = Ht1f3 forward primer
  source 1..37: mol_type = other DNA
atcgggaagctgaagaggaagaatcgcctgtgaagga

SEQ ID NO: 11 - DNA, 38 bp, synthetic construct
  misc_feature 1..38: note = Ht1r4v2 reverse primer
  source 1..38: mol_type = other DNA
atccgacggtagtgtttgatggcaatcagctccttcct

SEQ ID NO: 12 - DNA, 58 bp, synthetic construct
  misc_feature 1..58: note = Forward primer secondary PCR Rxn
  source 1..58: mol_type = other DNA
aatgatacggcgaccaccgagatctacacatacgagatccgtaatcgggaagctgaag

SEQ ID NO: 13 - DNA, 56 bp, synthetic construct
  misc_feature 1..56: note = Reverse primer secondary PCR Rxn
  source 1..56: mol_type = other DNA
caagcagaagacggcatacgagatnnnnnnnnacacgcacgatccgacggtagtgt

SEQ ID NO: 14 - DNA, 21 bp, Zea mays
  source 1..21: mol_type = genomic DNA
gtttggatgtcacatgattgg

SEQ ID NO: 15 - DNA, 23 bp, Zea mays
  source 1..23: mol_type = genomic DNA
gttgtttggtatatgcagagcgg

SEQ ID NO: 16 - DNA, 23 bp, Zea mays
  source 1..23: mol_type = genomic DNA
gctgctcacgtgatcagccaagg

SEQ ID NO: 17 - DNA, 22 bp, Zea mays
  source 1..22: mol_type = genomic DNA
gttggttagaatgaaaactagg

SEQ ID NO: 18 - DNA, 18 bp, synthetic construct
  misc_feature 1..18: note = HT1-CR6 DNA version of guide RNA
  source 1..18: mol_type = other DNA
gtttggatgtcacatgat

SEQ ID NO: 19 - DNA, 20 bp, synthetic construct
  misc_feature 1..20: note = HT1-CR9 DNA version of guide RNA
  source 1..20: mol_type = other DNA
gctgctcacgtgatcagcca

SEQ ID NO: 20 - DNA, 20 bp, synthetic construct
  misc_feature 1..20: note = HT1-CR7 DNA version of guide RNA
  source 1..20: mol_type = other DNA
gttgtttggtatatgcagag

SEQ ID NO: 21 - DNA, 19 bp, synthetic construct
  misc_feature 1..19: note = HT1-CR10 DNA version of guide RNA
  source 1..19: mol_type = other DNA
gttggttagaatgaaaact

SEQ ID NO: 22 - DNA, 25 bp, synthetic construct
  misc_feature 1..25: note = Ht1HR1f1 forward primer
  source 1..25: mol_type = other DNA
attatgttttcaaatggttggcact

SEQ ID NO: 23 - DNA, 29 bp, synthetic construct
  misc_feature 1..29: note = Ht1HR1r1 reverse primer
  source 1..29: mol_type = other DNA
cgattttggaggttatagaattgaattgg

SEQ ID NO: 24 - DNA, 28 bp, synthetic construct
  misc_feature 1..28: note = Ht1HR2f1 forward primer
  source 1..28: mol_type = other DNA
tagacttacctgtccttcgagtgttaga

SEQ ID NO: 25 - DNA, 29 bp, synthetic construct
  misc_feature 1..29: note = Ht1HR2r1 reverse primer
  source 1..29: mol_type = other DNA
gaatgagaatcccaataatatccaaaggt

SEQ ID NO: 26 - DNA, 22 bp, synthetic construct
  misc_feature 1..22: note = hdr2b_f forward primer
  source 1..22: mol_type = other DNA
gatctagagggatgccgtgatc

SEQ ID NO: 27 - DNA, 24 bp, synthetic construct
  misc_feature 1..24: note = hdr2b_r reverse primer
  source 1..24: mol_type = other DNA
ccaggtatctcagatgaaacaagc

SEQ ID NO: 28 - DNA, 17 bp, synthetic construct
  misc_feature 1..17: note = hdr2b_PV probe
  source 1..17: mol_type = other DNA
cagtcaggttcgtcgat

SEQ ID NO: 29 - DNA, 17 bp, synthetic construct
  misc_feature 1..17: note = hdr2b_PG probe
  source 1..17: mol_type = other DNA
cagtcagggtcgacgat

SEQ ID NO: 30 - DNA, 18 bp, Zea mays
  source 1..18: mol_type = genomic DNA
gaagatagaagtaggccg

SEQ ID NO: 31 - DNA, 17 bp, Zea mays
  source 1..17: mol_type = other DNA
gttaacgatgtcaacgt

SEQ ID NO: 32 - DNA, 21 bp, Zea mays
  source 1..21: mol_type = other DNA
gttcgcattagtctaggatta

SEQ ID NO: 33 - DNA, 18 bp, synthetic construct
  misc_feature 1..18: note = NLB18-CR1 DNA version of guide RNA
  source 1..18: mol_type = other DNA
gaagatagaagtaggccg

SEQ ID NO: 34 - DNA, 17 bp, synthetic construct
  misc_feature 1..17: note = NLB18-CR8 DNA version of guide RNA
  source 1..17: mol_type = other DNA
gttaacgatgtcaacgt

SEQ ID NO: 35 - DNA, 21 bp, synthetic construct
  misc_feature 1..21: note = NLB18-CR4 DNA version of guide RNA
  source 1..21: mol_type = other DNA
gttcgcattagtctaggatta

SEQ ID NO: 36 - DNA, 21 bp, Zea mays
  source 1..21: mol_type = genomic DNA
gtacgtaacgtgcagtactgg

SEQ ID NO: 37 - DNA, 24 bp, Zea mays
  source 1..24: mol_type = genomic DNA
gcataatgaggatcgaggatgagg

SEQ ID NO: 38 - DNA, 21 bp, Zea mays
  source 1..21: mol_type = genomic DNA
gctcgtgttggagatacaggg

SEQ ID NO: 39 - DNA, 21 bp, synthetic construct
  misc_feature 1..21: note = 8HR1f1 forward primer
  source 1..21: mol_type = other DNA
cagtccgtggattgaagccat

SEQ ID NO: 40 - DNA, 22 bp, synthetic construct
  misc_feature 1..22: note = PH26NPr reverse primer
  source 1..22: mol_type = other DNA
acccactcagttccatgacaga

SEQ ID NO: 41 - DNA, 20 bp, synthetic construct
  misc_feature 1..20: note = PH26NTf forward primer
  source 1..20: mol_type = other DNA
aacgagccgagtcgagtcaa

SEQ ID NO: 42 - DNA, 23 bp, synthetic construct
  misc_feature 1..23: note = 8HR2r1 reverse primer
  source 1..23: mol_type = other DNA
ctggtagctctgtctccgagacg

SEQ ID NO: 43 - DNA, 21 bp, synthetic construct
  misc_feature 1..21: note = 10HR1f forward primer
  source 1..21: mol_type = other DNA
tggcttgtctatgcgcatctc

SEQ ID NO: 44 - DNA, 24 bp, synthetic construct
  misc_feature 1..24: note = Ht1Pr reverse primer
  source 1..24: mol_type = other DNA
tgacagttgataaagaccggatga

SEQ ID NO: 45 - DNA, 24 bp, synthetic construct
  misc_feature 1..24: note = Ht1Tf forward primer
  source 1..24: mol_type = other DNA
tgaaccggctaggaaagtttagtt

SEQ ID NO: 46 - DNA, 25 bp, synthetic construct
  misc_feature 1..25: note = 10HR2r reverse primer
  source 1..25: mol_type = other DNA
ggacatctatacttgagggcttcac

SEQ ID NO: 47 - DNA, 20 bp, synthetic construct
  misc_feature 1..20: note = 45hr1f1 forward primer
  source 1..20: mol_type = other DNA
gcgtgcgtgcttacatgatg

SEQ ID NO: 48 - DNA, 22 bp, synthetic construct
  misc_feature 1..22: note = PH26NPr reverse primer
  source 1..22: mol_type = other DNA
acccactcagttccatgacaga

SEQ ID NO: 49 - DNA, 20 bp, synthetic construct
  misc_feature 1..20: note = PH26NTf forward primer
  source 1..20: mol_type = other DNA
aacgagccgagtcgagtcaa

SEQ ID NO: 50 - DNA, 30 bp, synthetic construct
  misc_feature 1..30: note = 45hr2r1 reverse primer
  source 1..30: mol_type = other DNA
agtcgacattaaacaatgttagttgtagcc

SEQ ID NO: 51 - DNA, 2658 bp, Zea mays
  source 1..2658: mol_type = other DNA
atggagaacccagacgcgcaggcgaaggcgtgggcggcggagatgcgcgagctggcctacgacatggaggacagcatcgatctcttcacccaccacgtcgaccacgaaccggccgacaccgccaccaccggcgtcaagaggttcttcctccggatcatccggaagcttaagaaactccactaccgccacaggtttgttcaggagatcaaacaactccacgaccttgccaacgaatcgtaccggcgtaggaagaggtacaggattgaggagggcggttcaagcctctcgcacgcggagatcgatcctcggttagaggcgctctacgtggaggtggagaaactcgtgggcatccagggcccaagccaggagatcattggacagctcgtcggcgagaacgcagcggagcgacggagggttgtcgccgttgttggatctggaggttcaggcaagaccacacttgccaaacaggtgtacgagaaaatcaggtgccaattctcttgtgcagcctttgtgtctgtgtcgcaaaagcccaacatgaatagcctcctgtgggagttgctatctcaaatcgggaaccatggtggagatttaggaatgatggcagtaggatattgcagtgacaaacaactgatcgacagactaagatcacatcttgaaaagcagaggtatctcgttgtgatagatgatgtttggacaaactcagcgtgggagaccatacaatgtgcgctccctaaaaatgcccatgcaagtaaaataattctgacaacacgaatcaacagtgtaggccagttctcctgcactccagatgagggttttatctatcagatgaagcctctttgcagaaacgattctgaaaatctgtttctgaaaaggacactatgtgataaagataagtttcctgctcagctggaggggattaaaaacgagataatcgagaaatgcgatggtttgccactggctattgttactctagctagcatgttagctactaaacagagaacaagggaagaatgggagagggcacttgattcaatccattctatgcacaagaaagatagtggcctggaagtgatggacaagatactgtctctgagttacagggatctacctcacaacatgagaaattgcttgctgtatctcagtacatttccagaggaccacacgatttacaaagatgccctagtatggagatggatggctgaagggtttatcgctgaaacacaaggctttactttggagcaggttgccgagggctacttctacgagtttgtgaacaggagtttggttcagcccataaccttgcgttcaagatatgaaatgcgtggagaaggaggttgccgagtccatgacattgtactgaacttcctcatctctcgtgcagctgaagagaactttttaactacgctgtatggcgcccagggggttccatcttcagaccgaaggattcgccggctctctgtctgggacagtccagaacacgcactggcagtctctagagcgaccatgaatctgtcccatctccggtcagttagaatatgcaacgttggagactggcccgtgcctgctgttctagacttacctgtccttcgagtgttagatctagagggatgccgtgatctgaggatcgacgaacctgactgcattctaagcttgtttcatctgagatacctgggtttccgcagcgcaagtggtgtcgtgctaccggctcaaatcggaaatttacaccatctgcagaccatcgatttaagcgggactggagtgacacagctgccagaaagcattgtccagctcaagcgactgatgcatcttgttgggcaacggctcatcatgccagacgggtttggtagcatggaatcccttgaggagttaggtactatcgactgctgcaagtgccccgtcagttttggggaagacctagcacttctgagcaggctgagggtgctccgagtggctttcatcggggtcgaaacaagtgacatggaaaccagaaggaaatctttgatgtcatccctctgcaaactcggaggagacaaccttcggcgtgtcactattatcgacctcgctggcggtggagattgctttgtggagtcgtggcaccctcctcctcgtctcctccagaagttcatccatatcagtcagcaacagcacttctccaggtttccagaatggatcagttcctgcctatgtgatctcacccacctggatataaaggccgaaaagatggaaagggagcatctaagtgttcttgaacacctgcccgccatccgttgcctataccttttcgtgaagcgagtctccgaagacgggctcgccatcagccacggcgcgttccgatgtctacggcgtctcgagttctgcaacgtagatggacctggtttgatgtttgcaggaggcgttccaatgttggaatggctgaggctcgggttcgacgcggatagagcgcaatcgacatacggcggtctggaggttggcatccagcgcctctcgtctctcaaacatgtcgtgctcattgtatggatggtttctgaaggcggtgatgatccagcggagcaagccgtctggtctgccatcaatggccaagtagagatgctccccaactctccgacggttgatatccggtttcgtagacggagtcagctgcaggcaagctcagaataa

SEQ ID NO: 52 - protein, 885 aa, Zea mays
MENPDAQAKAWAAEMRELAYDMEDSIDLFTHHVDHEPADTATTGVKRFFLRIIRKLKKLHYRHRFVQEIKQLHDLANESYRRRKRYRIEEGGSSLSHAEIDPRLEALYVEVEKLVGIQGPSQEIIGQLVGENAAERRRVVAVVGSGGSGKTTLAKQVYEKIRCQFSCAAFVSVSQKPNMNSLLWELLSQIGNHGGDLGMMAVGYCSDKQLIDRLRSHLEKQRYLVVIDDVWTNSAWETIQCALPKNAHASKIILTTRINSVGQFSCTPDEGFIYQMKPLCRNDSENLFLKRTLCDKDKFPAQLEGIKNEIIEKCDGLPLAIVTLASMLATKQRTREEWERALDSIHSMHKKDSGLEVMDKILSLSYRDLPHNMRNCLLYLSTFPEDHTIYKDALVWRWMAEGFIAETQGFTLEQVAEGYFYEFVNRSLVQPITLRSRYEMRGEGGCRVHDIVLNFLISRAAEENFLTTLYGAQGVPSSDRRIRRLSVWDSPEHALAVSRATMNLSHLRSVRICNVGDWPVPAVLDLPVLRVLDLEGCRDLRIDEPDCILSLFHLRYLGFRSASGVVLPAQIGNLHHLQTIDLSGTGVTQLPESIVQLKRLMHLVGQRLIMPDGFGSMESLEELGTIDCCKCPVSFGEDLALLSRLRVLRVAFIGVETSDMETRRKSLMSSLCKLGGDNLRRVTIIDLAGGGDCFVESWHPPPRLLQKFIHISQQQHFSRFPEWISSCLCDLTHLDIKAEKMEREHLSVLEHLPAIRCLYLFVKRVSEDGLAISHGAFRCLRRLEFCNVDGPGLMFAGGVPMLEWLRLGFDADRAQSTYGGLEVGIQRLSSLKHVVLIVWMVSEGGDDPAEQAVWSAINGQVEMLPNSPTVDIRFRRRSQLQASSE

SEQ ID NO: 53 - DNA, 2652 bp, Zea mays
  source 1..2652: mol_type = other DNA
atggagaacccagacgcgcaggcgaaggcgtgggcggcggagatgcgcgagctggcctacgacatggaggacagcatcgatctcttcacccaccacgtcgaccacgaaccggccgacaccgccaccaccggcgtcaagaggttcttcctccggatcatccggaagcttaagaaactccactaccgccacaggtttgttcaggagatcaaacaactccacgaccttgccaacgaatcgtaccggcgtaggaagaggtacaggattgaggagggcggttcaagcctctcgcacgcggagatcgatcctcggttagaggcgctctacgtggaggtggagaaactcgtgggcatccagggcccaagccaggagatcattggacagctcgtcggcgagaacgcagcggagcgacggagggttgtcgccgttgttggatctggaggttcaggcaagaccacacttgccaaacaggtgtacgagaaaatcaggtgccaattctcttgtgcagcctttgtgtctgtgtcgcaaaagcccaacatgaatagcctcctgtgggagttgctatctcaaatcgggaaccatggtggagatttaggaatgatggcagtaggatattgcagtgacaaacaactgatcgacagactaagatcacatcttgaaaagcagaggtatctcgttgtgatagatgatgtttggacaaactcagcgtgggagaccatacaatgtgcgctccctaaaaatgcccatgcaagtaaaataattctgacaacacgaatcaacagtgtaggccagttctcctgcactccagatgagggttttatctatcagatgaagcctctttgcagaaacgattctgaaaatctgtttctgaaaaggacactatgtgataaagataagtttcctgctcagctggaggggattaaaaacgagataatcgagaaatgcgatggtttgccactggctattgttactctagctagcatgttagctactaaacagagaacaagggaagaatgggagagggcacttgattcaatccattctatgcacaagaaagatagtggcctggaagtgatggacaagatactgtctctgagttacagggatctacctcacaacatgagaaattgcttgctgtatctcagtacatttccagaggaccacacgatttacaaagatgccctagtatggagatggatggctgaagggtttatcgctgaaacacaaggctttactttggagcaggttgccgagggctacttctacgagtttgtgaacaggagtttggttcagcccataaccttgcgttcaagatatgaaatgcgtggagaaggaggttgccgagtccatgacattgtactgaacttcctcatctctcgtgcagctgaagagaactttttaactacgctgtatggcgcccagggggttccatcttcagaccgaaggattcgccggctctctgtctgggacagtccagaacacgcactggcagtctctagagcgaccatgaatctgtcccatctccggtcagttagaatatgcaacgttggagactggcccgtgcctgctgttctagacttacctgtccttcgagtgttagatctagagggatgccgtgatctgaggatcgacgaacctgactgcattctaagcttgtttcatctgagatacctgggtttccgcagcgcaagtggtgtcgtgctaccggctcaaatcggaaatttacaccatctgcagaccatcgatttaagcgggactggagtgacacagctgccagaaagcattgtccagctcaagcgactgatgcatcttgttgggcaacggctcatcatgccagacgggtttggtagcatggaatcccttgaggagttaggtactatcgactgctgcaagtgccccgtcagttttggggaagacctagcacttctgagcaggctgagggtgctccgagtggctttcatcggggtcgaaacaagtgacatggaaaccagaaggaaatctttgatgtcatccctctgcaaactcggaggagacaaccttcggcgtgtcactattatcgacctcgctggcggtggagattgctttgtggagtcgtggcaccctcctcctcgtctcctccagaagttcatccatatcagtcagcacttctccaggtttccagaatggatcagttcctgcctatgtgatctcacccacctggatataaaggccgaaaagatggaaagggagcatctaagtgttcttgaacacctgcccgccatccgttgcctataccttttcgtgaagcgagtctccgaagacgggctcgtcatcagccacggcgcgttccgatgtctacggcgtctcgagttctgtaacgtagatggacctggtttgatgtttgcaggaggcgttccaatgttggaatggctgaggctcgggttcgacgcggatagagcgcaatcgacatacggcggtctggaggttggcatccagcgcctctcgtctctcaaacatgtcgtgctcattgtatggatggtttctgaaggcggtgatgatccagcggagcaagccgtctggtctgccatcaatggccaagtagagatgctccccaactctccgacggttgatatccggtttcgtagacggagtcagctgcaggcaagctcagaataa

SEQ ID NO: 54 - protein, 883 aa, Zea mays
MENPDAQAKAWAAEMRELAYDMEDSIDLFTHHVDHEPADTATTGVKRFFLRIIRKLKKLHYRHRFVQEIKQLHDLANESYRRRKRYRIEEGGSSLSHAEIDPRLEALYVEVEKLVGIQGPSQEIIGQLVGENAAERRRVVAVVGSGGSGKTTLAKQVYEKIRCQFSCAAFVSVSQKPNMNSLLWELLSQIGNHGGDLGMMAVGYCSDKQLIDRLRSHLEKQRYLVVIDDVWTNSAWETIQCALPKNAHASKIILTTRINSVGQFSCTPDEGFIYQMKPLCRNDSENLFLKRTLCDKDKFPAQLEGIKNEIIEKCDGLPLAIVTLASMLATKQRTREEWERALDSIHSMHKKDSGLEVMDKILSLSYRDLPHNMRNCLLYLSTFPEDHTIYKDALVWRWMAEGFIAETQGFTLEQVAEGYFYEFVNRSLVQPITLRSRYEMRGEGGCRVHDIVLNFLISRAAEENFLTTLYGAQGVPSSDRRIRRLSVWDSPEHALAVSRATMNLSHLRSVRICNVGDWPVPAVLDLPVLRVLDLEGCRDLRIDEPDCILSLFHLRYLGFRSASGVVLPAQIGNLHHLQTIDLSGTGVTQLPESIVQLKRLMHLVGQRLIMPDGFGSMESLEELGTIDCCKCPVSFGEDLALLSRLRVLRVAFIGVETSDMETRRKSLMSSLCKLGGDNLRRVTIIDLAGGGDCFVESWHPPPRLLQKFIHISQHFSRFPEWISSCLCDLTHLDIKAEKMEREHLSVLEHLPAIRCLYLFVKRVSEDGLVISHGAFRCLRRLEFCNVDGPGLMFAGGVPMLEWLRLGFDADRAQSTYGGLEVGIQRLSSLKHVVLIVWMVSEGGDDPAEQAVWSAINGQVEMLPNSPTVDIRFRRRSQLQASSE

SEQ ID NO: 55 - DNA, 2631 bp, Zea mays
  source 1..2631: mol_type = other DNA
atggagaacccagacgcgcaggcgaaggcgtgggcggcggagatgcgcgagctggcctacgacatggaggacagcatcgatctcttcacccaccacgtcgaccacgaaccggccgacaccgccaccaccggcgtcaagaggttcttcctccggatcatccggaagcttaagaaactccactaccgccacaggtttgctcaggagatcaaacaactccacgaccttgccaacgaatcgtaccggcgtaggaagaggtacaggattgaggagggcggttcaagcctcccgcacgcggagatcgatcctcggttagaggcgctctacgtggaggtggagaaactcgtgggcatccagggcccaagccaggagatcattggacagctcgtcggcgagaacgcagcggagcggcggagggttgtcgccgttgttggatctggaggttcaggcaagaccacacttgccaaacaggtgtacgagaaaatcaggtgccaattctcttgtgcagcctttgtgtccgtgtcgcaaaagcccaacatgaatagcctcctgtgggagttgttatctcaaatcgggaaccatggtggagatttaggaatgatggcagtaggatattgcagtgacaaacaactgatcgacagactaagatcacatcttgaaaagcagaggtatctcgttgtgatagatgatgtttggacaaactcagcgtgggagaccatacaatgtgcgctccctaaaaatgcccatgcaagtaaaataattctgacaacacgaatcaacagtgtaggccagttctcctgcactccagatgagggttttatctatcagatgaagcctctttgcagaaacgattctgaaaatctgtttctgaaaaggacactatgtgataaagataagtttcctgctcagctggaggggattaaaaacgagataatcgagaaatgcgatggtttgccactggctattgttactctagctagcatgttagctactaaacagagaacaagggaagaatgggagagggcacttgattcaatccattctacgcacaagaaagatagtagcctggaagtgatggacaagatactgtctctgagttacagggatctacctcacaacatgagaaattgcttgctgtatatcagtacatttccagaggaccacacgatttacaaagatgctctagtatggagatggatggctgaagggtttatcgctgaaacacaaggctttactttggagcaggttgccgagggctacttctacgagtttgtgaacaggagtttggttcagcccataaccttgcgttcaagatatgaaatgcgtggagaaggaggttgccgagtccatgacattgtactgaacttcctcatctctcgtgcagctgaagagaactttttaactacgctgtatggcgcccagggggttccatcttcagaccgaaggattcgccggctctctgtctgggacagtccagaacacgcactggcagtctctagagcgaccatgaatctgtcccatctccggtcagttagaatatgcaacgttggagactggcccgtgcctgctgttctagacttacctgtccttcgagtgttagatctagagggatgccgtgatctgaggatcgtcgaccctgactgcattctaagcttgtttcatctgaggtacctgggtttccgcagcgcaagtggtgtcgtgctaccggctcaaataggaaatttacaccatctgcagaccatcgatttaagcgggactggagtgacacagctgccagaaagcattgtccagctcaagcgactgatgcatcttgttgggcaacggctcatcatgccagacgggtttggtagcatggaatcccttgaggagttaggtactatcgactgctgcaagtgccccgctgagggtgctccgagtgaccgagtggctttcgtcggggtcgaaacaagtgacatggaaaccagaaggaaatctttgatgtcatccctctgcaaactcggaggagacaaccttcggcgtgtcactattatcgacctcgctggcggtggagattgctttgtggagtcgtggcaccctcctcctcgtctcctccagaagttcatccatatcagtcagcaacagcacttctccaggtttccagaatggatcagttcctgcctatgtgatctcacccacctggatataaaggccgaaaagatggaaagggagcatctaagtgttcttgaacacctgcccgccatccgttatctataccttttcgtgaagcgagtctccgaagacgggctcgtcatcagccacagcgcgttccgatgtctacggcgtctcgagttctgtaacttagatggacctggtttgatgtttgcaggaggcgttccaatgctggaatggctgaggctcgggttcgacgcggatagagcgcaatcgacatacggcggtctggaggttggcatccagcgcctctcgtctctcaaacatgtcgtgctcattgtctgtatggtttctgaaggcggtgatgatccagcggagcaagccgtctggtctgccatcaatggccaagtagagatgctccccaattctccgacggttgatatccggtttcgtagacggagtcagctgcaggcaagctcagaataa

SEQ ID NO: 56 - protein, 876 aa, Zea mays
MENPDAQAKAWAAEMRELAYDMEDSIDLFTHHVDHEPADTATTGVKRFFLRIIRKLKKLHYRHRFAQEIKQLHDLANESYRRRKRYRIEEGGSSLPHAEIDPRLEALYVEVEKLVGIQGPSQEIIGQLVGENAAERRRVVAVVGSGGSGKTTLAKQVYEKIRCQFSCAAFVSVSQKPNMNSLLWELLSQIGNHGGDLGMMAVGYCSDKQLIDRLRSHLEKQRYLVVIDDVWTNSAWETIQCALPKNAHASKIILTTRINSVGQFSCTPDEGFIYQMKPLCRNDSENLFLKRTLCDKDKFPAQLEGIKNEIIEKCDGLPLAIVTLASMLATKQRTREEWERALDSIHSTHKKDSSLEVMDKILSLSYRDLPHNMRNCLLYISTFPEDHTIYKDALVWRWMAEGFIAETQGFTLEQVAEGYFYEFVNRSLVQPITLRSRYEMRGEGGCRVHDIVLNFLISRAAEENFLTTLYGAQGVPSSDRRIRRLSVWDSPEHALAVSRATMNLSHLRSVRICNVGDWPVPAVLDLPVLRVLDLEGCRDLRIVDPDCILSLFHLRYLGFRSASGVVLPAQIGNLHHLQTIDLSGTGVTQLPESIVQLKRLMHLVGQRLIMPDGFGSMESLEELGTIDCCKCPAEGAPSDRVAFVGVETSDMETRRKSLMSSLCKLGGDNLRRVTIIDLAGGGDCFVESWHPPPRLLQKFIHISQQQHFSRFPEWISSCLCDLTHLDIKAEKMEREHLSVLEHLPAIRYLYLFVKRVSEDGLVISHSAFRCLRRLEFCNLDGPGLMFAGGVPMLEWLRLGFDADRAQSTYGGLEVGIQRLSSLKHVVLIVCMVSEGGDDPAEQAVWSAINGQVEMLPNSPTVDIRFRRRSQLQASSE

SEQ ID NO: 57 - DNA, 2667 bp, Zea mays
  source 1..2667: mol_type = other DNA
atggagaacccagacgcgcaggcgaaggcgtgggcggcggagatgcgcgagctggcctacgacatggaggacagcatcgatctcttcacccaccacgtcgaccacgaaccggccgacaccgccaccaccggcgtcaagaggttcttcctccggatcatccggaagcttaagaaactccactaccgccacaggtttgctcaggagatcaaacaactccacgaccttgccaacgaatcgtaccggcgtaggaagaggtacaggattgaggagggcggttcaagcctcccgcacgcggagatcgatcctcggttagaggcgctctacgtggaggtggagaaactcgtgggcatccagggcccaagccaggagatcattggacagctcgtcggcgagaacgcagcggagcggcggagggttgtcgccgttgttggatctggaggttcaggcaagaccacacttgccaaacaggtgtacgagaaaatcaggtgccaattctcttgtgcagcctttgtgtccgtgtcgcaaaagcccaacatgaatagcctcctgtgggagttgttatctcaaatcgggaaccatggtggagatttaggaatgatggcagtaggatattgcagtgacaaacaactgatcgacagactaagatcacatcttgaaaagcagagaactgatttttcaactgcttcacaatctgctcttaggtatctcgttgtgatagatgatgtttggacaaactcagcgtgggagaccatacaatgtgcgctccctaaaaatgcccatgcaagtaaaataattctgacaacacgaatcaacagtgtaggccagttctcctgcactccagatgagggttttatctatcagatgaagcctctttgcagaaacgattctgaaaatctgtttctgaaaaggacactatgtgataaagataagtttcctgctcagctggaggggattaaaaacgagataatcgagaaatgcgatggtttgccactggctattgttactctagctagcatgttagctactaaacagagaacaagggaagaatgggagagggcacttgattcaatccattctacgcacaagaaagatagtagcctggaagtgatggacaagatactgtctctgagttacagggatctacctcacaacatgagaaattgcttgctgtatatcagtacatttccagaggaccacacgatttacaaagatgctctagtatggagatggatggctgaagggtttatcgctgaaacacaaggctttactttggagcaggttgccgagggctacttctacgagtttgtgaacaggagtttggttcagcccataaccttgcgttcaagatatgaaatgcgtggagaaggaggttgccgagtccatgacattgtactgaacttcctcatctctcgtgcagctgaagagaactttttaactacgctgtatggcgcccagggggttccatcttcagaccgaaggattcgccggctctctgtctgggacagtccagaacacgcactggcagtctctagagcgaccatgaatctgtcccatctccggtcagttagaatatgcaacgttggagactggcccgtgcctgctgttctagacttacctgtccttcgagtgttagatctagagggatgccgtgatctgaggatcgtcgaccctgactgcattctaagcttgtttcatctgaggtacctgggtttccgcagcgcaagtggtgtcgtgctaccggctcaaataggaaatttacaccatctgcagaccatcgatttaagcgggactggagtgacacagctgccagaaagcattgtccagctcaagcgactgatgcatcttgttgggcaacggctcatcatgccagacgggtttggtagcatggaatcccttgaggagttaggtactatcgactgctgcaagtgccccgctgagggtgctccgagtgaccgagtggctttcgtcggggtcgaaacaagtgacatggaaaccagaaggaaatctttgatgtcatccctctgcaaactcggaggagacaaccttcggcgtgtcactattatcgacctcgctggcggtggagattgctttgtggagtcgtggcaccctcctcctcgtctcctccagaagttcatccatatcagtcagcaacagcacttctccaggtttccagaatggatcagttcctgcctatgtgatctcacccacctggatataaaggccgaaaagatggaaagggagcatctaagtgttcttgaacacctgcccgccatccgttatctataccttttcgtgaagcgagtctccgaagacgggctcgtcatcagccacagcgcgttccgatgtctacggcgtctcgagttctgtaacttagatggacctggtttgatgtttgcaggaggcgttccaatgctggaatggctgaggctcgggttcgacgcggatagagcgcaatcgacatacggcggtctggaggttggcatccagcgcctctcgtctctcaaacatgtcgtgctcattgtctgtatggtttctgaaggcggtgatgatccagcggagcaagccgtctggtctgccatcaatggccaagtagagatgctccccaattctccgacggttgatatccggtttcgtagacggagtcagctgcaggcaagctcagaataa

SEQ ID NO: 58 - protein, 888 aa, Zea mays
MENPDAQAKAWAAEMRELAYDMEDSIDLFTHHVDHEPADTATTGVKRFFLRIIRKLKKLHYRHRFAQEIKQLHDLANESYRRRKRYRIEEGGSSLPHAEIDPRLEALYVEVEKLVGIQGPSQEIIGQLVGENAAERRRVVAVVGSGGSGKTTLAKQVYEKIRCQFSCAAFVSVSQKPNMNSLLWELLSQIGNHGGDLGMMAVGYCSDKQLIDRLRSHLEKQRTDFSTASQSALRYLVVIDDVWTNSAWETIQCALPKNAHASKIILTTRINSVGQFSCTPDEGFIYQMKPLCRNDSENLFLKRTLCDKDKFPAQLEGIKNEIIEKCDGLPLAIVTLASMLATKQRTREEWERALDSIHSTHKKDSSLEVMDKILSLSYRDLPHNMRNCLLYISTFPEDHTIYKDALVWRWMAEGFIAETQGFTLEQVAEGYFYEFVNRSLVQPITLRSRYEMRGEGGCRVHDIVLNFLISRAAEENFLTTLYGAQGVPSSDRRIRRLSVWDSPEHALAVSRATMNLSHLRSVRICNVGDWPVPAVLDLPVLRVLDLEGCRDLRIVDPDCILSLFHLRYLGFRSASGVVLPAQIGNLHHLQTIDLSGTGVTQLPESIVQLKRLMHLVGQRLIMPDGFGSMESLEELGTIDCCKCPAEGAPSDRVAFVGVETSDMETRRKSLMSSLCKLGGDNLRRVTIIDLAGGGDCFVESWHPPPRLLQKFIHISQQQHFSRFPEWISSCLCDLTHLDIKAEKMEREHLSVLEHLPAIRYLYLFVKRVSEDGLVISHSAFRCLRRLEFCNLDGPGLMFAGGVPMLEWLRLGFDADRAQSTYGGLEVGIQRLSSLKHVVLIVCMVSEGGDDPAEQAVWSAINGQVEMLPNSPTVDIRFRRRSQLQASSE

SEQ ID NO: 59 - DNA, 2930 bp, Zea mays
  source 1..2930: mol_type = genomic DNA
atggagaacccagacgcgcaggcgaaggcgtgggcggcggagatgcgcgagctggcctacgacatggaggacagcatcgatctcttcacccaccacgtcgaccacgaaccggccgacaccgccaccaccggcgtcaagaggttcttcctccggatcatccggaagcttaagaaactccactaccgccacaggtttgttcaggagatcaaacaactccacgaccttgccaacgaatcgtaccggcgtaggaagaggtacaggattgaggagggcggttcaagcctctcgcacgcggagatcgatcctcggttagaggcgctctacgtggaggtggagaaactcgtgggcatccagggcccaagccaggagatcattggacagctcgtcggcgagaacgcagcggagcgacggagggttgtcgccgttgttggatctggaggttcaggcaagaccacacttgccaaacaggtgtacgagaaaatcaggtgccaattctcttgtgcagcctttgtgtctgtgtcgcaaaagcccaacatgaatagcctcctgtgggagttgctatctcaaatcgggaaccatggtggagatttaggaatgatggcagtaggatattgcagtgacaaacaactgatcgacagactaagatcacatcttgaaaagcagaggttagtttaccttttcattccggttagcttaattcggtacaccaactagagatttgtgatttgctattaattacaccaaatttctcctacacaacaataactggtttagcatgatggcgatccaaagtcaaaactatcttctactactagtgtatgccatactcatatagatattttcttttcataaactctcgtagcatttttacatgcattcatattcctattgcctttatacagaactgatttttcactgcttcacaatctgctcttaggtatctcgttgtgatagatgatgtttggacaaactcagcgtgggagaccatacaatgtgcgctccctaaaaatgcccatgcaagtaaaataattctgacaacacgaatcaacagtgtaggccagttctcctgcactccagatgagggttttatctatcagatgaagcctctttgcagaaacgattctgaaaatctgtttctgaaaaggacactatgtgataaagataagtttcctgctcagctggaggggattaaaaacgagataatcgagaaatgcgatggtttgccactggctattgttactctagctagcatgttagctactaaacagagaacaagggaagaatgggagagggcacttgattcaatccattctatgcacaagaaagatagtggcctggaagtgatggacaagatactgtctctgagttacagggatctacctcacaacatgagaaattgcttgctgtatctcagtacatttccagaggaccacacgatttacaaagatgccctagtatggagatggatggctgaagggtttatcgctgaaacacaaggctttactttggagcaggttgccgagggctacttctacgagtttgtgaacaggagtttggttcagcccataaccttgcgttcaagatatgaaatgcgtggagaaggaggttgccgagtccatgacattgtactgaacttcctcatctctcgtgcagctgaagagaactttttaactacgctgtatggcgcccagggggttccatcttcagaccgaaggattcgccggctctctgtctgggacagtccagaacacgcactggcagtctctagagcgaccatgaatctgtcccatctccggtcagttagaatatgcaacgttggagactggcccgtgcctgctgttctagacttacctgtccttcgagtgttagatctagagggatgccgtgatctgaggatcgacgaacctgactgcattctaagcttgtttcatctgagatacctgggtttccgcagcgcaagtggtgtcgtgctaccggctcaaatcggaaatttacaccatctgcagaccatcgatttaagcgggactggagtgacacagctgccagaaagcattgtccagctcaagcgactgatgcatcttgttgggcaacggctcatcatgccagacgggtttggtagcatggaatcccttgaggagttaggtactatcgactgctgcaagtgccccgtcagttttggggaagacctagcacttctgagcaggctgagggtgctccgagtggctttcatcggggtcgaaacaagtgacatggaaaccagaaggaaatctttgatgtcatccctctgcaaactcggaggagacaaccttcggcgtgtcactattatcgacctcgctggcggtggagattgctttgtggagtcgtggcaccctcctcctcgtctcctccagaagttcatccatatcagtcagcaacagcacttctccaggtttccagaatggatcagttcctgcctatgtgatctcacccacctggatataaaggccgaaaagatggaaagggagcatctaagtgttcttgaacacctgcccgccatccgttgcctataccttttcgtgaagcgagtctccgaagacgggctcgccatcagccacggcgcgttccgatgtctacggcgtctcgagttctgcaacgtagatggacctggtttgatgtttgcaggaggcgttccaatgttggaatggctgaggctcgggttcgacgcggatagagcgcaatcgacatacggcggtctggaggttggcatccagcgcctctcgtctctcaaacatgtcgtgctcattgtatggatggtttctgaaggcggtgatgatccagcggagcaagccgtctggtctgccatcaatggccaagtagagatgctccccaactctccgacggttgatatccggtttcgtagacggagtcagctgcaggcaagctcagaataa

SEQ ID NO: 60 - protein, 16 aa, Zea mays
VSFGEDLALLSRLRVL

SEQ ID NO: 61 - DNA, 2064 bp, Zea mays
  source 1..2064: mol_type = other DNA
tccacctcgtctaccacgtcttctccccgccatggctgctcaccagcctcacctctccgtcctcctcctcgtcctcctcgctgcccatgtcgtctccacctccgcccatggcgagcctcctcttccgagcccttacaacacctccgcccatggcgagcctcctcttccgagcacttacaacgcctccatgtgctcgtcgttctggtgtggcggcgtcgagatccgctacccgttctatcttgccaacgcaatcgccgactacagcgggagctactactcctgcggctacaccgacttgagcgtttcctgcgaactcgaggtcgaggggtcgccgacgacctggacccctaccatccgtctcggcggcggcgactacaccgtcaagaacatctcctacctctacgaccagcagaccatctcactggcggacagagatgtgctcggaggcggcggctgccccgtcgtccgccacaacgtcagcttcgacgagacgtggctgcacctgcacaacgccagcgccttcgacaacctcaccttcttcttcggatgccactgggggccacggaatacaccgcctgaatttgccgactacaacatcagctgcgccgggttcaatactccaactatcagcggtggaaggtccttcgtgttcaagactggagatcttgacgaacaagaggagcaggagttggctttacactgcgacgaggttttctccgtgccagtgagaagagatgctctgcaggcgatcgtcagcaacttcagcctcacacgggacgggtacggcgaggtgcttaggcaggggttcgagttggaatggaatcggacatcggaggatcagtgtggccggtgcgagggatcgggctccggcggatggtgcgcctacagccagaagagagaattcctgggctgcttgtgcagcggagggaaggtgggcagcccgttctgcaaaccatcgagatcaaaaaggaaagaaggacctattgttggtgctgttgccgttgcattcctgtgtctagtcattctcacatgcttcttggcttgtagacatggttcgctgcccttcaaatcggagaacaaaccagggacaaggattgagtccttcctacagaagaacgagagtatacatccgaaaagatacacctacgcggacgtgaaaagaatgacaaaatccttcgctgtgaagctaggccaaggtgggtttggtgctgtatacaaaggcagcctccacgatggccgacaggtagcagtcaagatgctgaaggacacccaaggtgacggcgaggaattcatgaacgaggtggctagcatcagcaggacttctcatgtcaacgtcgtgacacttctagggttttgcttgcaagggtcgaaaagagcactgatctacgagtacatgcccaatggttcgctcgaaaggtatgccttcaccggtgacatgaacagtgagaatttgctaacctgggaaaggctatttgacatagcaattggcacggccagagggctcgaatacctacaccggggatgcaacactcggatcgtgcattttgacatcaagccacacaacatcctgttagaccaggatttctgtcctaagatctctgactttggactggccaagctatgtctgaacaaagagagcgctatctccattgctggcgcaagagggacgatagggtatatcgccccggaggtctactcaaagcaatttggaataataagcagcaagtctgatgtctatagctatgggatgatggtccttgagatggttggagcaagggacaggaatacaagcgcagatagtgaccatagcagccaatatttccctcagtggctttatgaacatttggacgactattgtgttggtgcttccgagattaatggtgagaccacagagctcgtgaggaagatgatagttgtaggtctgtggtgcatacaagtgattccgactgatcgaccaacaatgacgagagtcgtcgagatgttggaagggagcacaagtaatctagagttgccacccagagttctcttgagctgacaaagcgtagatatttttcctatcaaatg

SEQ ID NO: 62 - protein, 667 aa, Zea mays
MAAHQPHLSVLLLVLLAAHVVSTSAHGEPPLPSPYNTSAHGEPPLPSTYNASMCSSFWCGGVEIRYPFYLANAIADYSGSYYSCGYTDLSVSCELEVEGSPTTWTPTIRLGGGDYTVKNISYLYDQQTISLADRDVLGGGGCPVVRHNVSFDETWLHLHNASAFDNLTFFFGCHWGPRNTPPEFADYNISCAGFNTPTISGGRSFVFKTGDLDEQEEQELALHCDEVFSVPVRRDALQAIVSNFSLTRDGYGEVLRQGFELEWNRTSEDQCGRCEGSGSGGWCAYSQKREFLGCLCSGGKVGSPFCKPSRSKRKEGPIVGAVAVAFLCLVILTCFLACRHGSLPFKSENKPGTRIESFLQKNESIHPKRYTYADVKRMTKSFAVKLGQGGFGAVYKGSLHDGRQVAVKMLKDTQGDGEEFMNEVASISRTSHVNVVTLLGFCLQGSKRALIYEYMPNGSLERYAFTGDMNSENLLTWERLFDIAIGTARGLEYLHRGCNTRIVHFDIKPHNILLDQDFCPKISDFGLAKLCLNKESAISIAGARGTIGYIAPEVYSKQFGIISSKSDVYSYGMMVLEMVGARDRNTSADSDHSSQYFPQWLYEHLDDYCVGASEINGETTELVRKMIVVGLWCIQVIPTDRPTMTRVVEMLEGSTSNLELPPRVLLS

SEQ ID NO: 63 - DNA, 2061 bp, Zea mays
  source 1..2061: mol_type = other DNA
tccacctcgtctaccacgtcttctcctcgccatggctgctcacctaccacgcctccccgtcctcctcctcgtcctcctcgctgctcatgtcgtctccacctccgcccatgccgagcctcctcttccgagcccttacagcacctccgcccatggcgagcctcctcttccgagcacttacaacgtctccatgtgctcggaatcgttctggtgcggcggcgtcgaaatccgctacccgttctatcttgccaacgcaaccgccgactacagcgggagctactactcctgcggctacaccgacttgagcgtttcctgcaaactcgaggtcgaggggccgacgacgacatggacccctaccatccgtctcggcggcgacaactacaccgtcaagaacatcttgtacgactatcataccatctcactggcggacagcgatgtgctcggaggcggcgagtgccccgtcgtccaccacaacgtcagcttcgacgagacgtggctgcacaaccccagcgccttcgacaacctcaccttcttcttcggatgccactgggggccacgcgatacactgcctgaatttgccggcaacaacatcagctgcgccgggttcagtactccagctatcagcggtggaggctccttcgtgttcaagcctgaagatcttgacgaacatgcggagcaggagttggcttcacactgcgacgaggttttctccgtgccagtgagaagcgaggctctgcagcaggcgatcgtcagcaacctcagcctcggggacgggtacggcgagctgcttaggcaggggatcgagttggaatggaaacggacatcggaggatcagtgtggccagtgcgaggaatcgggctccggcggacggtgcgcctacagccagaagagagaattccttggctgcttgtgcagcggagggaaggcgggcaacccgttctgcaaaccatcaagatcaaaaaggaaagaagcatctattgttggtgctgttgccgttgcattcctgtgtctagtcattctcacatgcttcttggcttgtagacatggttcgctgcccttcaaatcggagaacaaaccagggacaaggattgagtccttcctacagaagaacgagagtatacatccgaaaagatacacctacacggacgtgaaaagaatgacaaaatccttcgctgtgaagctaggccaaggtgggtttggtgctgtatacaaaggcagcctccacgatggccgacaggtagcagtcaagatgctcaaggacacccaaggtgacggcgaggaattcatgaacgaggtggctagcatcagcaggacttctcatgtcaacgtcgtgacacttctagggttttgcttgcaagggtcgaaaagagcactgatctacgagtacatgcccaatggttcgctcgaaaggtatgccttcaccggtgacatgaacagtgagaatttgctaacctgggaaaggctatttgacatagcaattggcacggccagagggctcgaatacctacaccggggatgcaacactcggatcgtgcattttgacatcaagccacacaacatcctgttagaccaggatttctgtcctaagatctctgactttggactggccaagctatgtctgaacaaagagagcgctatctccattgttggcgcaagagggacgatagggtatatcgccccggaggtctactcaaagcaatttggaacaatcagcagcaagtctgatgtctatagctatgggatgatggtccttgagatggttggagcaagggaaaggaatacaagcgcaagcgcagatagtgaccatagcagccaatatttccctcagtggatttatgaacatttggacgactattgtgttggtgcttccgagattaatggtgagaccacagagctcgtgaggaagatgatagttgtaggtctgtggtgcatacaagtgattccgactgatcgaccaacaatgacgagagtcgtcgagatgttggaagggagcacgagtaatctagagttgccacccagagttctcttgagctgacaaagcgtagatatttttcctatcaaatg

SEQ ID NO: 64 - protein, 666 aa, Zea mays
MAAHLPRLPVLLLVLLAAHVVSTSAHAEPPLPSPYSTSAHGEPPLPSTYNVSMCSESFWCGGVEIRYPFYLANATADYSGSYYSCGYTDLSVSCKLEVEGPTTTWTPTIRLGGDNYTVKNILYDYHTISLADSDVLGGGECPVVHHNVSFDETWLHNPSAFDNLTFFFGCHWGPRDTLPEFAGNNISCAGFSTPAISGGGSFVFKPEDLDEHAEQELASHCDEVFSVPVRSEALQQAIVSNLSLGDGYGELLRQGIELEWKRTSEDQCGQCEESGSGGRCAYSQKREFLGCLCSGGKAGNPFCKPSRSKRKEASIVGAVAVAFLCLVILTCFLACRHGSLPFKSENKPGTRIESFLQKNESIHPKRYTYTDVKRMTKSFAVKLGQGGFGAVYKGSLHDGRQVAVKMLKDTQGDGEEFMNEVASISRTSHVNVVTLLGFCLQGSKRALIYEYMPNGSLERYAFTGDMNSENLLTWERLFDIAIGTARGLEYLHRGCNTRIVHFDIKPHNILLDQDFCPKISDFGLAKLCLNKESAISIVGARGTIGYIAPEVYSKQFGTISSKSDVYSYGMMVLEMVGARERNTSASADSDHSSQYFPQWIYEHLDDYCVGASEINGETTELVRKMIVVGLWCIQVIPTDRPTMTRVVEMLEGSTSNLELPPRVLLS

SEQ ID NO: 65 - DNA, 5930 bp, Zea mays
  source 1..5930: mol_type = genomic DNA
gatattgaatccaattcaattctataacctccaaaatcgatatcctaacatagcatgatagtttttttgagaggtgtgatttaacatattagatgaattttctttttttaatacgctatgttctagatgtctgacgatgaatggagccgctctgcatataccaaacgctatctaagtttgtgaacaaatgactaaattatccacacgaccacaattgggcgctgataagatccacacttgctggttttaattcatccggtctttatcaactgtcacatcagttatagatcattatcaacttttatctacaattgatgttgtaatacacggtcacttaagaccatgtttaggtacaatgtctctcaaaactatgattttacttatgatgacaataccgtagttttgaatagctctaaaaatatcatggttctaaaaatattgtttggattcaacattataaatcgtggtattaagcaaaagctagtcatgttataaaaactttaggttgaagtagagttttcaatactaaaaaaatatcatggtatttagaatatcatgattttaaaaatatagttcttacgaatgcaaccaaacaccttatgatataaaataatatggtattgcctacaaactacaaaaataaatcactcccaagcattacataaacatcatttttataaactttttagtaaaataaagcgcaatgtttttattaaatagaaatttatacaagtatatataattaagcaaataaaaactacgttattcataaaaagctaataaaaagtaaaaagtaaaaactatataattcataaaaaaatcgttatctttctcttccatcttattatctatttttagttgttttgtcaaatttaaggctattttatgggttctttttatctttgtacatgtcgtgagccaataacttattgaattggtcaatcaatttaggttgagttttacttttaactaacctagtatagtttgttcaacacctttttttcataatcggggactcattccacttgttgttgacccattttttcttctactgagttcttgcccttttgcaatcaataggacgtggtgagcccatatttttaggtgttatggatttataatcaccgttcaaatttgaatgaatattttgtttttattattgaagtcttcgtcaatcgttatcatgcctcgcataccacttagaccgacgaagtccaacatatttctcccccgacgaggagagattcttcgtaaaattgctactggtattactggtattgaatagaagataagggtgcgtttggttgcatgcatctacgcgtgcttgcatcacggaatgcgggttggtgctgtttggttgctataagctagactatacatatgcaagttttgtgtttggttggctgcatgcagatttcgatccaaactcgcacgatccacacagcaccctgggccaggcttaccagatacgagtagattggtcgcatctttggagccaggctttagcggtccgcggtcctggctgacacggccagattgccgagagaaaccaaccaaacagggtctaaatgtccaatcgtttgactgctactggatgaaaaaagaatgtcacaactttaaaatgtgtatttatttatactcctacacatgaaataactactatactcagatttcttttacattcagattttttctcagccactgaaacataccagccctttactaccaaaaacaggaactccacggtccaatgattatgtgagtcggaggagaggggaggaagaatcgcctgtgaaggagggagggagggagggacgtccgatccgaagatggaaggagctggggaggggagcgccttgacggggatgatgggtcctgcgctcgacaagctcgctagcctcgttgacaagtacaccgagctcagaaacgtgaggaagaagatggagcagctgaggaaggagctgattgcgatcaacctcgcgcttgagaagcacgcggccatggagaacccagacgcgcaggcgaaggcgtgggcggcggagatgcgcgagctggcctacgacatggaggacagcatcgatctcttcacccaccacgtcgaccacgaaccggccgacaccgccaccaccggcgtcaagaggttcttcctccggatcatccggaagcttaagaaactccactaccgccacaggtttgttcaggagatcaaacaactccacgaccttgccaacgaatcgtaccggcgtaggaagaggtacaggattgaggagggcggttcaagcctctcgcacgcggagatcgatcctcggttagaggcgctctacgtggaggtggagaaactcgtgggcatccagggcccaagccaggagatcattggacagctcgtcggcgagaacgcagcggagcgacggagggttgtcgccgttgttggatctggaggttcaggcaagaccacacttgccaaacaggtgtacgagaaaatcaggtgccaattctcttgtgcagcctttgtgtctgtgtcgcaaaagcccaacatgaatagcctcctgtgggagttgctatctcaaatcgggaaccatggtggagatttaggaatgatggcagtaggatattgcagtgacaaacaactgatcgacagactaagatcacatcttgaaaagcagaggttagtttaccttttcattccggttagcttaattcggtacaccaactagagatttgtgatttgctattaattacaccaaatttctcctacacaacaataactggtttagcatgatggcgatccaaagtcaaaactatcttctactactagtgtatgccatactcatatagatattttcttttcataaactctcgtagcatttttacatgcattcatattcctattgcctttatacagaactgatttttcactgcttcacaatctgctcttaggtatctcgttgtgatagatgatgtttggacaaactcagcgtgggagaccatacaatgtgcgctccctaaaaatgcccatgcaagtaaaataattctgacaacacgaatcaacagtgtaggccagttctcctgcactccagatgagggttttatctatcagatgaagcctctttgcagaaacgattctgaaaatctgtttctgaaaaggacactatgtgataaagataagtttcctgctcagctggaggggattaaaaacgagataatcgagaaatgcgatggtttgccactggctattgttactctagctagcatgttagctactaaacagagaacaagggaagaatgggagagggcacttgattcaatccattctatgcacaagaaagatagtggcctggaagtgatggacaagatactgtctctgagttacagggatctacctcacaacatgagaaattgcttgctgtatctcagtacatttccagaggaccacacgatttacaaagatgccctagtatggagatggatggctgaagggtttatcgctgaaacacaaggctttactttggagcaggttgccgagggctacttctacgagtttgtgaacaggagtttggttcagcccataaccttgcgttcaagatatgaaatgcgtggagaaggaggttgccgagtccatgacattgtactgaacttcctcatctctcgtgcagctgaagagaactttttaactacgctgtatggcgcccagggggttccatcttcagaccgaaggattcgccggctctctgtctgggacagtccagaacacgcactggcagtctctagagcgaccatgaatctgtcccatctccggtcagttagaatatgcaacgttggagactggcccgtgcctgctgttctagacttacctgtccttcgagtgttagatctagagggatgccgtgatctgaggatcgacgaacctgactgcattctaagcttgtttcatctgagatacctgggtttccgcagcgcaagtggtgtcgtgctaccggctcaaatcggaaatttacaccatctgcagaccatcgatttaagcgggactggagtgacacagctgccagaaagcattgtccagctcaagcgactgatgcatcttgttgggcaacggctcatcatgccagacgggtttggtagcatggaatcccttgaggagttaggtactatcgactgctgcaagtgccccgtcagttttggggaagacctagcacttctgagcaggctgagggtgctccgagtggctttcatcggggtcgaaacaagtgacatggaaaccagaaggaaatctttgatgtcatccctctgcaaactcggaggagacaaccttcggcgtgtcactattatcgacctcgctggcggtggagattgctttgtggagtcgtggcaccctcctcctcgtctcctccagaagttcatccatatcagtcagcaacagcacttctccaggtttccagaatggatcagttcctgcctatgtgatctcacccacctggatataaaggccgaaaagatggaaagggagcatctaagtgttcttgaacacctgcccgccatccgttgcctataccttttcgtgaagcgagtctccgaagacgggctcgccatcagccacggcgcgttccgatgtctacggcgtctcgagttctgcaacgtagatggacctggtttgatgtttgcaggaggcgttccaatgttggaatggctgaggctcgggttcgacgcggatagagcgcaatcgacatacggcggtctggaggttggcatccagcgcctctcgtctctcaaacatgtcgtgctcattgtatggatggtttctgaaggcggtgatgatccagcggagcaagccgtctggtctgccatcaatggccaagtagagatgctccccaactctccgacggttgatatccggtttcgtagacggagtcagctgcaggcaagctcagaataaggagcacgaaaaagacgatgatgttggatgtcgcctgctagctgtagtatgttgctgcttctgcttgttgccaacacattttttttgggttagggtggggtacaaccataaaatgtgtgtggatgtgcttgtaagcattacttgtatgtttttttttgtaaagcacaatatagatagatgcatatatgtgtgcgtgcaaagctatgattatcgacactcacacttgtacattagctagatgaaggtctcgacagagcagagcatagtacacatctctgggagttggactggacactataacggggatgctgcagccgaaactcaaaagctacatgcatgtcacttggctcatcggcgcaggaagcaacgcaggtccatcacgcgcagcaccttgaacccgtccaggctacaccccagcagcagcctcggcttcttcggcgccggcgggcagcgcggggggcgttcggttccagcgccactcgccgtcgccgacgacagcggcgagagcttccgtggaccttcttcgtcctcgtcgccgccgcgggagtaagaccgcttcagcttcagcggccgcagctccaccagctgcggaatgctaacatcttcttcaggcacctgccgggtggttctctttcccagaatcttccgctggagacccatggcgagctcggttcggtttaacctgcaattaatgcgcaatagcggagtaggaagcgagattgttagctcaggcgagcagagatgaaccggctaggaaagtttagttgctcgtgcatgctaccagctagcttgttggaggctcttgctttggacaccaagcaacggatatgacagcagaatgtgcgtgcttataagcaagcaagcagagcagcagttgcaaagaagggaaaaggtggagtggaaaaaggagttgccattgaagtgcacgagtgagcgagcatcatgtcaaggaaccaggagggaagttgcacaacagatgaaaagcggagagctgtttccg

SEQ ID NO: 66 - DNA, 13125 bp, Zea mays
  source 1..13125: mol_type = genomic DNA
tgaactcgtgctatcgcaaagtaagggcacctgatgaaaatacaagccaaaatcccataaagtagccatcatccaaatcagctgcgagcaatagttagcggcaacgacatactcggctagatagtggcaacaacaactagcgacttgatgttgatctgcccttttagatctggtttggtgataggagaattagagggaatctatgggaaaggaaatctcttggtactcaattttaaatagtaagggatttactctccatagtttccctctaaatcagttgtctcccaaccaacaagtcccaaagatatgtagtgtccaacatcaactataagactgtatccagcagtttacgcatatggtcactcaaattattgttttgtactgtaaattgtactgttctgcacttttcgcagagtgaggtttgaatgtgtgtatgtggatgggcaagatgctagagctaggccaaggcgcatatcatactagtctccgacgttgacatcgttaacgagtaagcggtcgcaatcggctgcccgcgcctccacgtgaacctcaccttcgacatcgtctggctacggcttgcaccctccagctccaacatcacattcctctacaattgcaagaagaacattagaccatctccaacaggtcgtgtaaatacccgtgcaaaatacaattttgtattatggattacactgtttgcagagtaaagtttaagataaagagttggataaggaatcagctgaacatattaccctaccctctgtcgtggaactgagtgggtgcccacaacaacaagaagatagaagtaggccgtggatggcgggatcatgggtgctgaggcgtacgtatacatgtccaaataggcaggtcgagccgacctggcccgagcctggctaggctcggcacggattgggatcatgttggcctgacccggattagtaagcgggtcgtgtcgtgcctgtccacgggtctcgaacgaggctcagacacaacatgctaagatattaaccgtgtcgggtcggcccacggcccgacaggcctaacaagtctataatagtatatggcatttaaatgataaaacatatgttaaaatatacatatatgaaagtttaaaccatagttattagctctaacacctatttacacccacataaccaacaaaacaaatatttttactgtattttatactatatattcaagtataatgtatgtatttgtattaaaaaataggaaaaaaattaaaaacgggtcatgtctagcctgtcgtgccgcgtcttagacccagacacgacttagtcaccaggccgagccaaccagtgcctgagtttcggaccgcccgacccgcctggacatctattggcgtacaagcacgggtgcgagggcgtggtggtggcgctgcctgtgctggatgtacccaagaagggcttgttcggttctaccttccatatggattgagggggattgaggggtttcaactctagtaagtcaaaaactcttctaatccatatcaatctcctctatctatatggattgaaaataggcaccactggcggtccgcctccggaacgggtcgctccgtcggttgctgcaggacgggttcgagctgaactacaacactcactccgagcagtgcgaccgatgcgagggctccgccggatggtgtgtggctaccagcgcgaggagacgcccgccggcgggatgacattcgcctgtttctgcgacggcggccagaccacgggccgatgcggtgccggtatgtctctgtttttttttcttcgaacaaggtttggcatgtgttctaccgtttcaactagtaaatgattacattgagctagccacacattttcttgaatgattttctttgattaaactgatgttttctttcatgacgtgaacaacgggcctgcaagctgccacatacctagggagactatttcgtgaccttctttacacgtcttctctactcgccactgggagttgacgccgctcggtcgtcccactttgtgacgttcaaccagagtctagagatgtaattctctgcgaatacaggactagttggagctaacaacgcagcttgacgagggtgaacccagctccacacctcgtctaccacgtcttctcctcgccatggctgctcacctaccacgcctccccgtcctcctcctcgtcctcctcgctgcccatgtcgtctccacctccacccgtgccgagcctcttcttcccagcacttacaacgtctccatgtgctcggaatcgttctggtgcggcggcgtcgagatccgctacccgttctatcttgccaacgcaaccgccgactacagcgggagctactactcctgcggctacaccgacttgagcgtttcctgcgaactcgaggtcgaggggccgccgacgacctggacccctaccatccgtctcggcggcgacaactacaccgtcaagaacatcttgtacgactatcataccatctcactggcggacagcgatgtgctcggaggcggcgagtgccccgtcgtccgccacaacgtcagcttcgacgagacgtggctgcacaacgccagcgccttcaacaacctcaccttcttcttcggatgccactgggggccacgcgatacactgcctgaatttgccggctataacatcagctgcgacgggttcagtactccaactatcagcggtggaggctccttcgtgttcaagactgaagatcttgacgaacaagaggagcaggatttcgcttcacactgcgacgaggttttctccgtgccagtgggaagcgaggctctgcgggcgaccgacaccttcagcctctcaaggtacgggtacggcgagctgcttaggcaggggttcgagttggaatggaatcggacatcggaggatcagtgtggccagtgcgagggatcgagctccggcggacggtgcgcctacaaccagaagagagaattcctgggctgcttgtgcagcggagggaaggcgggcaacccgttctgcaaaccctcaagtaaagtcctgaaccgagcctcccttattttttttcattttttgcaatcaccagagagcacgcatcggttgcgtcagtagcttgcaacctcgtagctagccccgcagtgtcccctgtgtgcgagtaccgcgctgctccagcttgcctcctgctaacgcctaacggtgaatgcttcatgcttgacatgatctagctagtctacactttgcttggggtttgcctgggagctggaaattctgtggctcctgtttgcatcactcgacaaggacgctttcagacttgcgagtctcgttctgcttttgcaccaaatccgtgttttttcatttcgtgatcgagattaatccagcatagagatgacaataggtatccgaaactcaaaactcaataggtttttactctattatggtacaagtttgagtcaattttcatatcatagatttgttaataggcacaaatctatatccaacaggttcatagatacgggtttgttcctacaataatcaaatccgtaaacccatgagttttttagacccgaccaaacctagtgcatattgtcattttattttataaacgaacaatattatctctctatttactttctattttttatcggttggtgaatgtataagtagttggtgagagtgttgcttgcttgctattataatatttagttatttactagtgttatatatgtggtgatggataacttagtgcaaggtcacttgattatacaacttattatttgtattcattctttctactaataatttttataccaaatcatgaactcggtgtttatcatataaattttggaccatgatctcattaatcatcacgatagttattgattatgagaaaaacaaacatattggagataaaatcctcggctaacccgttaacccgatgggtacgggtttgaacagaatttcaaacccattatgaatataagttttttaacaaatatagatatgtttcacggatagagtttgagatgacaaaatccaacggatttgttgccatctctatccggcggcccttaccgtgctccacgagcagaggtcgtatccctcttcccgtgtcgcctgcttcgcgttgccgaacggagacgtttggtagcgttggccggctctagcagtcgggtcaatttttttgttgttgttttcgatgttgttggatttttgttccgtataagccatgttttagtaatttatttagtccagccgaatccgagacgtgtttgctgggttggagacttggagttgctagtcatgatatgctttctactcggtttgatttcaacccagttaggctatatttgatactccagtatttattccaatataaatggtttgaaagggattaaggtataaattagtttaatttatatctttaattcctctcaacccatatgtattgggctgaatactaagtatccaaacaaacccttatttaagatgcatttcctttaggtctcgtttgtttcgttggaattgaattctattttaataattataatatatttatatatgaaatatatttgaatattatcctaaatcatatgagagagatagttatatactacatttatgttatatcgaagcaagtaaaagagtgtgatataagttgtgcatcggaaaaatagtatgtaaatctataaaatcaatttccatctctcacccaatgaatttgagataggataatatgataactttgtaaagtggtggaatatcacattctaaaaaaatagtctattccattagtaagattccaattcctcaaaatgaaagggaaacaaacgggaccatagttacacgtggccactgttgtgtgggggtgggggtgaggggggacaggccaatcctactcgtcagtgctcattcgagagcaaagataccgaaggagattagagagactaaaaactttttactatttaaaattagataataagacgatttaatcccgttccatatctttgctctaaacaaaccctcaatgatcatatatctcgaaagatccggccggctgttctttatttatcaagtgatgactgctgaccgcttatagaatatatattttaaagcaaaatttcttctacagcagtaaaaggactagacgaaacaatgatgcatttctctaacaaaagaaagtagaattatcaagcggagagccaagaccaaaagccttgcatctatgggcgtcaaccaatgataccgcgacggaaccaccccagctggtctatactgtctgtcacgacccagcgagtaaccgtgtggctacgctgttagcttaggactcgacgaaatgctcgattcattaacaaaccagctcacgagttaaatgatttattatataacgaaattatatgcatattatttaccagtgtgacgacagagggcataggtgggcaatattcagctcctctaattctatagggattgttaatttctttagctaattatcatgtaaacgatataaaaaatgtttctaacagcacctcggtccaccctaatcttagaccctagcttcgcccatgtcatttacgtaacaattggtaaatatgttatacatgtgtagtgtctatgtcctatgaattaaactaatgattgatgaattgtgcttatatattaaattggtctatgcgaatataactatgtgttaaactgatgaatatgtgtgtgaattgtgaattgataagtgacgagttgtgtctaatttagtgttatattgatgtgttttatgaaactatgagtataattaatattttctataattaaatttgtttgaaattaactagaaattgattattatatatatatattgttttctgctctaattcgcaagctaaacaagcaagctcaagctcgtaaacgagccgaaccgagctgactctgtggctcattaacttaacaacccgagccgggccaacttgttagcttaacgagccagctcgaatacggacgagttgagccgagctggcatgatatccagccttaattaggctcgtaccagtgcaacatatccctctcgcctttgtcacgtccagacatgtcaatgggccccgattcccgcaaggaattcctctattaagagatgaggatgagaaagtttctccccacggaaaaattctctcctgacgcataaacggggacaacactccacatccccattcctcgtggggacctattaaacttacatatggtgatgttttcatgtaaaagttaatgataaaaataaataattacgttgtcaagatatcactttttgtacaaatgtgctcattctgatgtaggcatattttttcttacatctaacaatgtgtataagtgagaatgttttgtattaataacaaagtaagtatgtcctaattataatttaagcggggccgggtatccccgatggggatttatacccttgggaaacgaagatggggaagaaatgtcctacacaagttttcatggcgatcctcgcggggaactttttcgtcgtggggatagggatggggagctaaaacccgatgaggaattcctcgttgccatccccagtcacatcaactctcgactccactattgtctatgctgcatagtctatggtagactatagcctcagcctatagcacatcagcttttctatttcagaattaagtaattcatgcagttttatttcaacgctcgaaaattacacaacataatattttttattgaattaaaaattataaagtgcatacaaatcaaaataaaaaaatattataattaaaacatatataaatctaatcggagacctcgatcttatcctcgtcttccaccacctctttccgttttgcttctggttcctcttcttcgtcatcaaccagaccacgtccttttttcgaacatctttatggccttggcatgggtttatctttcggctaggtccatatccctggttgaatggctctttagaatattccgttgctttaaaagcttggtcttcactaatccaccccacaagttcttcattttaaatgcttcacttgttgaccgttgcttgtggcttccttccctttccccttcaccttcatctttaacgcagccgcctttgccctatcacgccctactgatcggggcacttccttcttggtatctttagtgcctccagaactatattcactagagactccgagtcgggttatcttattcgtagtcccattttatcctagaacctcgtcattgctgcctccatgaccattgcctcgtctgctccgctctgatgcaacttttcttctcgaaggtagtatccattaaacttggtcacctcctggttgtaggtgccctaatgatttttaagttgcttggcggtttgaggatatcaagggtcggaggtggagttatatgttgtcgctatttgactccaaaaacatgatccaaacttattattgacgggggttgaattattagaatgcatattccaagaattaacctataatataagtaaactacaaatataaatattaaataaatgagaaatgattcactcaccaacttttcctcatcgtcattcatccattctagcctctttggacgcttttctttcggcccaggattttcctcagcttggttttcaaatccaacatattggacatgtatgtgaaattggaggaggtggtccatacagaggtggagcatatgcaggaggggcatacggaggtactgagaaagaagtttgacttccatccgcagcaggtggagggcatacagacgtaccgaggaaaaagcttgaattctggcttgggaagttggaggttgaccatatgaaggcggcgagtatgaatacagatgataggaaaaggttatggtagtggtggacgcgcaactgaaaatagtgcatggggactgaagctgaagcatcagagcgacaatgtagtggagagactcatcaaacggaggggtttgtgacccatcggactacaagagatctatgaaggtgttcaaatctagggaccaacccgacattgtgtgaacagaggggagtttggaagagagaaacgaaatgaaatggtgtgtggaatgagatcaacccaagtagaggtacttacaaagggattgggatgaaatttgtgatttttttgcaattttttattttttggattccaaacgatcaaaaacaactagttgcaatagctagcacacgtgaaccaattgaaagcccccaccttgctctcgttcgcgccagcgcgtcacccacccactgcgccctctcatcctccttgcccgagaacgtgcttcagagcaggcgagagtggggcgatatcgcccactctcattgggcacgggcggtatcgcccgagggatgcatctctccctcctctcaccccgggccaggctacaacagccccctactgcccaaccactcgccctcgttggcaccaaccatactaccacaacactccaatgcacagtttttaatgttagcctatagtcaccttagcatcacatcatatttcttctacaaaatcatatttagaacgaaacatgatgttttgcttggaattttttcggtggagtagaaaaaatataatccaaaaaaattacgtaaaatacgtaaaataaaaaatatagctcctaaaagttaaaattactcatcattatcaccctcctcgttttcttcctcgtctagttttaattgcgtgatcaatttttcagaaccaacctagaccctcctcataccagtggtggattgtttcagtaacttggtgaactggtcgtacaattttttgattgatttctcgtgtcactaaccttgaataactgctttgttatggttttcttctggacaagggactcattggtactcattcatggtccctaacccttgttttgtgctcttgcccaatcacgaccaatagggtgtggtggtttggcactatcagacgatgtagagttataatcaccctccacgttgaggcaagatcatttgctctcattgctagagtttgaatcaccatgtcacgtgcaccacttgaattgatgatgaagagcacaccattagtttcatcgagcctgttgtggaagagtagcatcacattatttgatctgcttggtaggttatacgtggtcgatatttggcaccaaaaggtcaaacatttttgttgtttccctcaaaccttttttggcctcaaaaaggtcaaaccttttttggctttccatccctgtccccacgaacagtcacgagtaactttttatcccatccacgttcgcgtgggggaatttatccccatgggaaatctatccctgttagagaatgtaatattttcgaggcaaggtcaaattgataaaccaatataaattgaacaaataagatttaaaattacaagagaaatctactttagagttgagcttgctattttataaaaggctatgtgttgaatttttattataactttaacatatcaatggattgattttagattaagagaagttcgtggggcggatatgcgaggaacagggatggggaatggttcaccattctcgtcccacgaacccggcaaggactaaatttttctcgtttcaatctccgtggggactaaattacacctattcccgtccactaataaagggataccccgcggggaattagggatcacgtccccatttcacatttttagacttctcacattgagcaacaacaaaacattttatgaatttgtagccattttacttatctaaaacaattactattgaatcttaatcattttgtgcaaaataaagaatgaactaaattttgggtcgggtgtgggtcacccgtaggttgaaataaaaactcgcacccacaacgtgaaactttgggtcagatgcgggttacacccgcggattaaaatctctacccatacccacacccgtcagatcgagtacccaaagattttgggtttgcgggttaaattgtcatccctagacacgagcgtgatggaggatttggaagtttcgcaatgcgtacttaccaagtgtttggttctatggattaaactttagcatgtgtcgcattagatgattgaatgcctattatgagtattaaatattgtctaattattaatcaaattacacaagtgaaggctaaacaactagacaaatttattaagcctgattaatttatgattagcaaatatttatagtagcagcatcttagtgaatcatgaactaattaggtttaataggttcgtcttaacgtttagttcttatctatgtaattagttttataagtaaactatatttaatattcctaattagcctccaaacatccgatataacatagactaaaatttagtggtggtgctgctggctccttttcatttcatccgacataatgttttcctcccaatttattgtgttgttttgtttgtgctttaaaaatgacttgtcctctgcttgctgtatcaaggtcgtgatgtgtgcttaacttattcccttccttgctagctgcccttagcatttatataggggtatttggttacagggactaaagtttagtttagtccgtatccaattataaaactaattacataattaaatactaaaataccaaaatacgagaaaaattattaaacctaattaatttattatttggcaaatgtttattgtaacatcacataagaaaagcatagactaatttagtttaataggttcgtcttatcatttagtcttgatctgtataattagttttgtaattagactatatttactatttttaactagtatccaaacacattaaatgtgacatggattaaaatttagttagtgaccttaggcttttagagttgagttagttgtagcttggtttagttacttgtttgttctcttacgtttatttaggacctctctataatgttttatcaccttcttaatacaaattaaaatacgcagctcttgcgtattgcaggcgtgtgtgttcctatattttttagctcaattatgaaggaaattattctcagcgagcatataaccgttttcgaggtaaaatgaactaaaagcatatgggcctgcctgttcgcataagtacaccctccgtctaaaaagaataaaaatctcatttcttgatgagtcaaagaagttcaaatttaagaaaatatatgttacgacacgaatatttataatgcgtaataagtactgctagattaattttaaaataaaattttcataataaacctatttgaagatacaagtattggtactatttctaataaatctaatcaaactggtgttatatcttttgtaacaaatttgtgctttatgtttctggttgacgtgaatcagcttaatcttgctgaaatctaacattgtcttttgttcgttggcatacaggatcaaaaaggaatgaaggacctattgttggtaagagcctatagccaatacccatgttcatttcgtctaaaagagcagaagaaaagcatatgatgaattattgccatgtcttgtttaaaatacagaattctcaaaaacaaaaacaaaaaaaacttggaatccactaaccactgatagcattgtagaaaatttcatcctccctttgggcaatacactgatgagtttacatgctgactagtggtgcatttgttctttgccaattgagtttttagaatgctttgcagctgaattcacttgtggtgttttttttttgtgtgatgcaggtgctgttgttgccgttgcattcctgtgtctagtcattctcacatgcttcttggcttgtagacatggttcgctgcccttcaaatcgaagaacaaaccagggacaaggattgagtccttcctacagaagaacgagagtagtatacatccgaaaagatacacctacgcggacgtgaaaagaatgacaaaatccttcgctgtgaagctaggccaaggtgggtttggtgctgtatacaaaggcagcctccacggccgacaggtagcagtcaagatgctgaaggacacccaaggtgacggcgaggaattcatgaacgaggtggctagcatcagcaggacttctcatgtcaacgtcgtgacacttctagggttttgcttgcaagggtcgaaaagagcactgatctacgagtacatgcccaatggttcgctcgaaaggtatgccttcaccggtgacatgaacagtgagaatttgctaagctgggaaagactatttgacatagcgattggcacggccagagggctcgaatacctacaccggggatgcaacactcggatcgtgcattttgacatcaagccacacaacatcctgttagaccaggatttctgccctaagatctctgactttggactggccaagctatgtctgaacaaagagagcgctatctccattgttggcgcaagagggacgatagggtatatcgccccggaggtctactcaaagcaatttggaacgataagcagcaagtctgatgtctatagctatgggatgatggtccttgagatggttggagcaagggacaggaatacaagcgcagatagtgaccatagcagccaatatttccctcagtggctttatgaacatttggacgactattgtgttggtgcttccgagattaatggtgagaccacagagctcgtgaggaagatgatagttgtaggtctgtggtgcatacaagtgattccgactgatcggccaacaatgacgagagtcgtcgagatgttggaagggagcacaagtaatctagagttgccacccagagttctcttgagctgacaaagcgtagatatttttcctatcaaatgctgcttccaggtcacacaaatgcaaatatttgtggagacgagtgcccagtaacctcatacactgtatctgtatgacaaaagtcccacgactcactggacacggaaatgtcgcttgactacgccaattttctaaaaagattggcacaattaatggggcttatagcggtaactttggttcgcattagtctaggattagggttgaatattgatcaaactcgacgcagcttggtcgagctcaagctagctccgctcagcttattaaagaatccagctagagaatcaacccaggtcgtttacgagttaatttgctggctcgtttaggtcgtaaatcacaacaaaaacaatatacacatatatacaataatataattaatactagttaattctagacta

SEQ ID NO: 67 - DNA, 500 bp, Zea mays
  source 1..500: mol_type = genomic DNA
agtgtccaacatcaactataagactgtatccagcagtttacgcatatggtcactcaaattattgttttgtactgtaaattgtactgttctgcacttttcgcagagtgaggtttgaatgtgtgtatgtggatgggcaagatgctagagctaggccaaggcgcatatcatactagtctccgacgttgacatcgttaacgagtaagcggtcgcaatcggctgcccgcgcctccacgtgaacctcaccttcgacatcgtctggctacggcttgcaccctccagctccaacatcacattcctctacaattgcaagaagaacattagaccatctccaacaggtcgtgtaaatacccgtgcaaaatacaattttgtattatggattacactgtttgcagagtaaagtttaagataaagagttggataaggaatcagctgaacatattaccctaccctctgtcgtggaactgagtgggtgcccacaacaacaagaagatagaagtagg

SEQ ID NO: 68 - DNA, 201 bp, Zea mays
  source 1..201: mol_type = genomic DNA
ttagggttgaatattgatcaaactcgacgcagcttggtcgagctcaagctagctccgctcagcttattaaagaatccagctagagaatcaacccaggtcgtttacgagttaatttgctggctcgtttaggtcgtaaatcacaacaaaaacaatatacacatatatacaataatataattaatactagttaattctagacta

SEQ ID NO: 69 - DNA, 492 bp, Zea mays
  source 1..492: mol_type = genomic DNA
tgaactcgtgctatcgcaaagtaagggcacctgatgaaaatacaagccaaaatcccataaagtagccatcatccaaatcagctgcgagcaatagttagcggcaacgacatactcggctagatagtggcaacaacaactagcgacttgatgttgatctgcccttttagatctggtttggtgataggagaattagagggaatctatgggaaaggaaatctcttggtactcaattttaaatagtaagggatttactctccatagtttccctctaaatcagttgtctcccaaccaacaagtcccaaagatatgtagtgtccaacatcaactataagactgtatccagcagtttacgcatatggtcactcaaattattgttttgtactgtaaattgtactgttctgcacttttcgcagagtgaggtttgaatgtgtgtatgtggatgggcaagatgctagagctaggccaaggcgcatatcatactagtctccgacg

SEQ ID NO: 70 - DNA, 13643 bp, Zea mays
  source 1..13643: mol_type = genomic DNA
tctaacgccgacaccgtcgacgagtaagaggtcgtggccggctgcccacacgtctgtgtgaacctcaccatcgacaccaccgtccgcctgcggcctacggcctcgaactccaacatcacattcctctacaactgcatgaagaacattaccctaccctctgtcatggaactgagtgggttcccacaacaacaagaagatagatgtaggtcgtacgtgctgtgggatggcgggatcacgggtgctcaggcgtacgggtatgggtgcgaggacttggtggtagcgtcggagctggatgtacacaaaaagggagaaggcgatccacctccggaacggatcgctccatcgggttgccgcatgacgggatcgagctgaactacgacactcactctaagcagtgggacctagggatgaaaacggtcggtaaacactaaagcaattaccgttttcatattttttttatcgaaaacaaaatcgaaaacggtaactccggaaatggaaacgatatcggtatttcggaaacatcgcaaacgaaagttcggtgcgaaaaatacacaagtaacggtcgaaatctaaaatacgatcgataaacatatcaaacttcataatacaacaaagttgacaaaagatcacaaagaccacaagttcacaattcatgatataacaagtttaaaatataacaagttcacaaggatcacaaatttataatataaaaaaattacaaagatcacaagttcacaatataacaagttcacagtataacaagttcataaagatcacaagttcacaaactcaaggttcacaattcacaatatccactcgatttagctgacatggcatgcttactcatgaaatattttttcctcaaataaagagtttttcacagactcgtaggaaaaccctaaaatctagtatgtggaaaagacagactgtcggctctatcattatatattactaatacataacatgtggacagaaaatggtggattcgttcgagagaccaaatcgttaatctcaactgccttccaacaccatctatcaaaaaaaatcttaaggcgtccaaaaaatacaaaaaataagtaatccttatctagagacgtacaggcgatgcgaaaaaaatcacatgctgaataattccgaaaaaaattccggaaaattctgagacataaatccggtaatttccgacaaaaaccggtaaccgaaggaaacagtcggtaaaacaccacgccgattccgataccgactctaatagaaatttccgaaaaccgatttcgttttcgaaaaatactgttaccggtgaatacaatcgaaaaatttcgaaatcggtttccggaataccaaaaaattgtgaaactgttttcatcactagtgggaccgatgtgatggctccgacggatggtgtggctaccagcgtgatgagacgcccaccggcgggatgacattcgcatgtttttgcaaacgcagcccgatcacatgtgcacaatcgttagtggcgcgttttaaaaaagacgtaactacgaaaaaaaatagcgacatgtttttagccagtgtcacaaacgtcatcttcgagcacttttgatgtagtgtatacaatctactagtcaaattaaaaagaataacatacacgaaatggttcataacttttatatagttaaacaataataaatttataaaaatccctaaacaaacaacaaaacgttggacacctccccgctatttatggcggatggcccgcccaattgacgtaatttccacatcgaagtcgaagaaccggtcgctgtgaccagtcaccccaacctccgtcacttgtctctcacgcgcgcgcaacatcgccgagaaaaccagaacagacctccggattggtctctcccccgttcacacgagcacattgcgatggctcctctgctcctgctgctcctcttccccgtccagctccccctcgcagtagccgacgccgtctccggtccctgcaccagagccacatgcgccggccaggacgtccattacccgttctggctcaagtcctccgcgcccgactgcgtctatcccggtgtcggccttgtggcccttgtctgcgagggcaactcgacgctgatcctccccttcaagtcccacagatacgtagtgctcagcatcgactacaagacgcgtaccgtgctggtctccgacgccgacatcgtccacgagtacgacgcggccggctgcccgcgcgtccgcgtgaacctcaccatcgacaccgcctggctgcggcccacggcctccgactccaacatcaccttcctctacaactgcaagaagaacatcaccctgccctccgccgtggaactgagcgggtgccagcagcagcagcaacaagacggcagcaggtcgtattcgtacgtgctgccggacggcggggtcacgggcgctgaggcgcaccagtacgggtgcgaggacttggtggtggcgccggtgctggacgtccacaggagggcgatcttgagggcgcctggcggcccgactctggagaacgggtcgctccgtcggttgctgcagggcgggttcgagctgaactacgacactcactccgagcagtgcgaccgatgcgaggcctccggcgggtggtgtggctaccagcgcgacgagacgcccgccggctggatgacgttcgcctgcttctgcgacggcgggccgacgaccacggcccgatgcggtgccggtatgtcttttttttttcttcgaacaaggtgtggcatgtgttctaccgtttcaactagtaaatgattacattgagctaggcagctagccacacattttcttgaatgattttctttgatgaacctgctgtttgcttttatgacgtgaacaacggggcctgcaagctgccacatacctagggagactagttcgtgaccttctttacacgtcttctctactcgccactgggagttgacgccgctcggtcgtcccactttgtgacgttcaaccagagtctagagatgtaattctctgcgaatacaggactagttggagctaacaacgcagcttgacgagggtgaacccagctccacctcgtctaccacgtcttctcctcgccatggctgctcacctaccacgcctccccgtcctcctcctcgtcctcctcgctgctcatgtcgtctccacctccgcccatgccgagcctcctcttccgagcccttacagcacctccgcccatggcgagcctcctcttccgagcacttacaacgtctccatgtgctcggaatcgttctggtgcggcggcgtcgaaatccgctacccgttctatcttgccaacgcaaccgccgactacagcgggagctactactcctgcggctacaccgacttgagcgtttcctgcaaactcgaggtcgaggggccgacgacgacatggacccctaccatccgtctcggcggcgacaactacaccgtcaagaacatcttgtacgactatcataccatctcactggcggacagcgatgtgctcggaggcggcgagtgccccgtcgtccaccacaacgtcagcttcgacgagacgtggctgcacaaccccagcgccttcgacaacctcaccttcttcttcggatgccactgggggccacgcgatacactgcctgaatttgccggcaacaacatcagctgcgccgggttcagtactccagctatcagcggtggaggctccttcgtgttcaagcctgaagatcttgacgaacatgcggagcaggagttggcttcacactgcgacgaggttttctccgtgccagtgagaagcgaggctctgcagcaggcgatcgtcagcaacctcagcctcggggacgggtacggcgagctgcttaggcaggggatcgagttggaatggaaacggacatcggaggatcagtgtggccagtgcgaggaatcgggctccggcggacggtgcgcctacagccagaagagagaattccttggctgcttgtgcagcggagggaaggcgggcaacccgttctgcaaaccatcaagtaaagtcctgaaccgagcctcccttatttttttttcattttttgcaatccaccagagagcacgcatcggttgcgtcagtatcttgcaacctcgtagctagccccgcagtgtcccctgtgtgcgagtaccgcgctgctccagcttgcctcctgctaacgcctaacggtgaatgcttcatgcttgacatgatctagctagtctacactttgcttggggtttgcctgggagctggaaattctggctcctgtttgcatcactcgacaaggacgctttcagacttgcgactctcgttctgcttttgcaccaaatccgtgtttttttcatttcgtgatcgagattaatctagcttagagatgacaatgggtatccgaaactcgaaacttgatggatttttactccattagggtataggtttgaatcaattttcatatttatggatttgttaataggcataaatatatatccaacaggtttatagatacgagtttgtttctacagtactcaaatccgtgaacacatgaggtttttaaacccgaccaaacctagtgcatattgtcattttattttataaacgaacaacaaaattgttatctctatttacttcctattttttatcgattggtgaatgtataagtagttggtgagaatgtttcttgcttgctattatagttttactagcgttatatatgttgtgggtggataacttagtgcaatgtcacttgattatacaacttattatttgtattcattctctctactaataatttttataccaaatcatgaactcggtgtttattatataaattttggaccataatctcattaatcatcacgatagttattgattatgagaaaaaacaagcatattggagataaaaccctcggctaacccgttaacccgatgggtacgggtttgaacaaaatttcaaacctattatgaatataagttttttaacaagtatagatatatttcacggatagagtttaagatgacaaaatccaacggatttgtatccattgccatctctatccggcggcccttacccggcggcccttaccgtgctccacgagcagaggtcgtatcgtccctcttcccgtgtcgcctgcttcgcgttgccgaacggagacgtttggtagcgttggccggctctagcagtcgggtcaactctttttgttgttgttttcgatgttgttggatttttgttccgtataagccatgttttagtaatttatttagtccagccgaatccgaagacgtgtttgctgggttggagactttggagttgctagtcatgatatgctttctactcggtttgatttcaacccagttaggctatatttaatactctagtatttatttcaatataaatggtttgaaacggattaaggtataaattagtttaatttatatatttaattcctctcaatccatatgtattgggctgaatactgaggtagtgtttggttgaagagccatatagaacggagccgttctgttccagttttgttgttgtttggttataaagtaactagaacggaatgacttcaattaaggaatattcttctcagatccagaaccattccgctctaaaaaatcaaccggacggagccgctccgtttccatcctgctcttacagtcacgctccgttccgttcactctgcaaccaaacaaaaaacagagccgctccgttccaaattaccaaacacagaacagagcggcttcattcctagaattaggaatggaacgactctgttctacttgactcctcaaccaaacactacctaagtatccaaacaagcccttatttaagatgcatttcctttacagttacacatgaccactattgtgtgggggcaggctgaacaagcccttatttaagatgcatttcctttagagttacacgtggccactattgtgggggggggggggggggggcaggccgatcctactcgtcagtgctcattcgagagcaaagataccgaaggagattagagagactaaaaactttttactatttaaaattagataataagacgatttaatcccgttccatatctttgctctaaacaaaccctcaatgatcatatatctcggaagatccggccggctgttctttatttatcaagtgatgactgctgaccgcttatagaatatatattttaaagcaaaatttcttctacagcagtaaaaggactagacgaaacaatgatgcatttctctaacaaaagaaagtagaattatcaagcggagagccaagaccaaaagccttacttctatgggcgtcaacaaatgataccgcgacggaaccatcccagcaggtctatactgtctgtcacgacccagcgagtaatcgtgtggctacgctattagacttaggattggatgaaatgctcggtttattaatgagccagctcgtgagttaagagtgtttggtttgatgaatgaagtaattcatcttcttttcactccccacttttttatttggtttgtgtaatagaatgagttgatccatcaccaccacattcatcataagctaataattagtatatacatgagtagtgagttgattccaccaaaattgatgaaatgaacttatgatgcatcatctcatgaagcatagagtgactccacaaaccaaacacaccataaatgatctattacataacgaaattatatgcatatcatttatcagggcgacgacagggggcatagggaggcaatatccccctaatgctccccaaattctatagggattgttagtttcttttagctaattctcatgtaaacaatataaaaaatgcttctaacagtccctcctaattataatttggtccaccctaatcttagatcctggcttcgtccgtgccatttacgtaacaattggtaaatatgttatacatgtgtggtatctatggcctatgaattgaactaatgattgatgaattgtgcttatgtgttaaattggtctatgcgaatataactatgggttaaacggatgaacatgtgtgttcattgttaattcatgagtgatgaattatgtataatttggtgttatattgatgtgttttgtgaaactatgtgtataattattattttctataattaaatttgtttgaaattaactagaaattgattattatatatatatatatatatatattgtttttctgctctagtctgcaagctaaacgagcaagctcaagctcgtaaacgatccgaaccgagctgactttgtggctcattaacttaacaagccgagttgggccaacttgttagcttaacgagtcagctcgaatacggacaagttgagccgagttggcatgatatccagccctaattaggcttgtaccagtgcaacatatccctctcgcctttgtcacgtccagacatgtcaatgggccccgattcccgcaaggaatttctctattaagggatgaggatgggaaagtttctccccccacagaaaaattctctcccgacggataagcggggacaacactccccatccccattccccgtggggacctattagacttacatatggtgatgttttcatgtaaaagttaatgataaaaataaacaattaccttgttgtcggcgtttcgaccccggagggtccctggaccgacgagtaaattgtcgctgcgtgtcccagcccagatgggtcgacgcgagacggaacacaagggggaaacaataaggggaatcgcggcctcgtgttgtcctgcgcccagggcggatgcgcttgcagtaaggggttacaagcgttcgcgagggagagagagagagagcctgtgcgccagcccgtcctcccgcgcggccaccttctcgtacgagggccctggacctttcttttatagatgtaaggagagggtccaggtgtacaacagggagcgtagcaatgtgctaacgtgtctagcagagggaagccagaatcctatgtacaggccgacgtgactgtcgaagaggttttggcgccctgttcatgtgatgtcgtggccgtcggaggagcgcttgagccctgtaggagcacagctgtcggagctgtcgggtccttgctgacgtctcattgcttccatagggagctgagaaccgccgtcgtcatggagcacgcggggtgccatcattacttgttttaccgggacgagccagatgggacgctggtcttgttcccagtagcctgaggtagctagaggtagggtaatgatgtgccctcctgcgacgtggtcggtccgagcccaaggtcgggcgaggcggaggctcctccgaggtcgaggctgagtccgagacctggggtcgggcgaggcggagaccgtcgtccgaggtcgaggttgagtccgagccctggggtcgggcgaggcagagtccatcgtccgaggtcgaggttgagtccgagccctggggtcgggcgaggcggagacagtcgtccgaggtcaaggttgagtccgagccctggggtcgggcgaggcggagttcgtcttccgaggtcgaggtggagtctgagccctagggtcaggcgaggcggagaccgtcgtccgaggtcgaggttgagtccgagctctggggtcgggcgaggtggagcttcctatggcgcctgaggccggacttggcggctgtcagcctcaacctgacgggtggcacagcagtcgaagcagcgcaggcggcgctgtttttctatcaggtcagccagtggaggggcgaagtgactgcggtcacttcggctctgtcgactgaagagcgtgcgtcaggataaggtgtcaggcgatccttgcattgaatgctcctgcgatccggtcggctggcgaggcgatcttggctaaggttgcttctccgcgaagcctgcctgagctgggcctcgggcgagtcggaggtgcgcccgttgcttgaggaggccctcgggcgaggcgtgaacctgcctgggcctgctgtttctgcccgaggctgggctcgggtgaggcgagatcgtgtcccttgagcggacagagctttgtcctgtgttgcgcccatcaggcctttgcagctttgtgctgatggtgtttaccagccgagtttaagagtcttgggggtacccctaattatggtccccgacacttgtcaagagatcactttttgtacaaatatattcattctgatgtacacatatttttttcttacatctaacaatgtgtataagtgagaatgttttatattaataacaaatgaagtatgtcctaattagacttctcacattgagcagcaacaaaacattttatgaattagtaaccattttacttactaaaataattactattgtatcttaatcattttgtgcaaaataaagaatgaaccaaattttgggtcaggtgtgggtcactcgcaggttgaaataaaaacccgcacccacactcgtgaaactttgggtcagatgcgggttacacccgcggattaaaatctctacccatacccacactcatcagatcgagtacccaaagattttaagtttgcgggttaaattgtcatccctcgacaccaacgtgttggaggatttggaagtttcgcgatgcgtacttaccaagtgtttggttctatgataaaagtttagcctgtgtcgcattagatgattgaatgtctattatgagtattaaatattgtctaattattaatcaaattacacaagtgaaggctaaacaacgagacaaatttattaagcctaattaatctatgattagcaaatgtttacagtagcaccatctagtagcaccatctgagcgaatcatgaactaattaggtttaataggttcgtcttaacgtttaattcttatctatgtaattagttttataagtaaattatatttaatacttctaattagcctccaaacattcgatataacatagactaaaatttagtcagtggtgctgctgctggctcttttccttcatccgacgtaatgttttcctcccaatttattgtgttgttttgtttgtgctttaaaactgacttgctctctgcttgctgtatcaaagtcgtgatgtgtgcttagcttattcccttccttgctagctgcccttagcatctatatagggatatttggttatagggactaaagtttagtttagtccgtgtccaattataaaactaattacataactgaatactaaaagacgagaaaattttattaaacttaattaatttatgattagcaaatgtttattgtaacatcacataagtaaattatagactaattttgtttaataggttcatcttatcatttagtcttcatctatgtaattagttttgtaattagactatatttactatttctaactagtatctaaacattaaatgtgacatggattaaaatttagttagagcaactccagtagttttctaaaagacttcctaaatcaataatttaggtagttaacatgaaaactattctccaacagttctctaaataaactttctaaatttaacaacttgtcatctaacctcattttctctctacatttggcaaccatttaataactccctaatcaaaaatgttgactgcattatatagtttttgtgacttattttttatgtggataaatacaaaataaaattacaacctatatttagagaactattggagaacccacttatttttatttcaaaagtcatttagcaacttcttaaatctgtaatttagaaagctaaaatttacataactattagagttgctcttagtgacgttaggcttttagagttgagttggtcgtagcttggtttagttacgtgtttgttctcttgcgtttatttaggacctctctataatgttttatcaccttcttaatacaaattaaaatacgcagctctcttgcgtattggaggcgtgtgttcctatattttttaggctcaattatgaatgaaattattctcagcgagcatataaccgttttcgaggtaaaatgaactaaaagcatatgggcctgcctgttcgcataagtacaccctccgtctaaaaaagaataaaaatatcatttcttgatgagtcaaaaaagttcaaatttaagaaaatatatgttacgacaccaatatttataatgtgtaataagtactgctgattaattttaaaataaaattttcataataaacctatttgaagatacaagtattggtactatttctaataaatctaatcaaactggtgttatatcttttgtaacaaatttgtgctttgtgtttctggttgacgtgaatcagcttaatcttgctgaaatctaacattgtcttttgttcgttggcatacaggatcaaaaaggaaagaagcatctattgttggtaagagcctatagtcaatacccatgttcatttcgtctaaaagagcagaagaaaagcatatgatgaattattgccatgtcatgtttaaaatacagaattctcaaaaacaaaaacaaaaaaaacttggaatccactaaccagtaaccactgatagcattgtagaaaatttcatcctccctttgggcaatacactgatgagtttacatgctgactagtggtgcatttgttctttgccaattgaatttttagaatgctttgcagctgaattcacttgtgatttttttttgtgatgcaggtgctgttgccgttgcattcctgtgtctagtcattctcacatgcttcttggcttgtagacatggttcgctgcccttcaaatcggagaacaaaccagggacaaggattgagtccttcctacagaagaacgagagtatacatccgaaaagatacacctacacggacgtgaaaagaatgacaaaatccttcgctgtgaagctaggccaaggtgggtttggtgctgtatacaaaggcagcctccacgatggccgacaggtagcagtcaagatgctcaaggacacccaaggtgacggcgaggaattcatgaacgaggtggctagcatcagcaggacttctcatgtcaacgtcgtgacacttctagggttttgcttgcaagggtcgaaaagagcactgatctacgagtacatgcccaatggttcgctcgaaaggtatgccttcaccggtgacatgaacagtgagaatttgctaacctgggaaaggctatttgacatagcaattggcacggccagagggctcgaatacctacaccggggatgcaacactcggatcgtgcattttgacatcaagccacacaacatcctgttagaccaggatttctgtcctaagatctctgactttggactggccaagctatgtctgaacaaagagagcgctatctccattgttggcgcaagagggacgatagggtatatcgccccggaggtctactcaaagcaatttggaacaatcagcagcaagtctgatgtctatagctatgggatgatggtccttgagatggttggagcaagggaaaggaatacaagcgcaagcgcagatagtgaccatagcagccaatatttccctcagtggatttatgaacatttggacgactattgtgttggtgcttccgagattaatggtgagaccacagagctcgtgaggaagatgatagttgtaggtctgtggtgcatacaagtgattccgactgatcgaccaacaatgacgagagtcgtcgagatgttggaagggagcacgagtaatctagagttgccacccagagttctcttgagctgacaaagcgtagatatttttcctatcaaatgttgcttccaggtcacacaaatgcaaaatatttgtggagacgagtgcctatttacctcatacactgtatctgtatgacaaaagtcccacgactcactggacgcggaaatgtcgcttgactacgccaattttctaaaaagattggcagcaattaatggaggcttatagcggtaactttggttcgcattaatcctaggactagggttgaatatcgatctaactcgacgcggcttggtcaagctcaagctagctccactcatctcattaaagaatccagctagaaaatcaacccaagtcgtttacgaaacgagtttgagctgactcgtttagatcgtaaatcacaacaaaaacaatatgcacatatatacaataatataatcaatactagttaattctagactagtttaacactagaaaagagtaatgatactcataatttcacatacaatgtcaatccaacaccaatttaacacacttcatcacttattagttcatccaaccaagtgtaggctttgatttactaacaaatggttgctcgttcgagctagcgagcttgcttgttaacaaactgagttgagatgctagcttaacttgtgacaaaattaaaacgagccgagtcgagtcaagttgagctcacgatgagtcgagcaagctcacaatccacgagtatttttttagtcctatctaagactaaagtttaatcctaaaactaaattttaatctctatttgtttggttctataaactaaacaggttcagaaaacataaaatacattatagaaaacctgaaatacccttctatacttaaggcatcactaagagagagcaataaataaagggtagagagaggaataaatctgctttattcccttttagctaccctttgagagagtaaacactaaaatgaaaggatccttgaggattttgatgttttggatgacaactaacacaattaaaggtctaattaggatgttaa

SEQ ID NO: 71 - DNA, 35391 bp, Zea mays
  source 1..35391: mol_type = genomic DNA
tgttggattaatgtggccttggcctaaattaatattcaataatagtcaatgctaatggcccactttaatgttatggtgtactaattatttagtaccatatttgaagttcaaaggacaaatcaatcaacttaaataggtggaccattggtgcatctattgagaagttgagaaaaggatgaaggactgccacacgcgcgcgcgcgccgcgtgctgctgttcttcttcccggcgaccgttcgagggactgcacagcgtatatcttcctgcaccgacttcgtacggctacatcgaacaaacacacgagatgtctcgtgtgaatggttgtgcatatttcattgctgtttactacttatgcgagtagttatacacacatgcacatacatgtcatcacatatatcgcactgtttttctggattaaattaaaactaaaaatgcctaactttctaacaatccaaaaatctgatattaggcatttttctgttagtggttttgctgctgcgttaaaaccaagtgaaccttttgatgggacgttttacaagagatggcgtagtaagatgatactgtggttgaccgcaatgaactgctatcacgccgcacaggggaaacccgaacagttcactcctgaagaggagagaatgttcgacgttgccgataacctgtttcgaggcgccgtgattggtgctcttgccaacaagtatgttgattcttatctaacgtgcacatctgcaaaagagttatgggatgcattagatgagaagtttggtgtttctgatgctgatagcgagctgtacatcatggagcagctatttgactataagatggtggaaaaccgtcctgtagttgaacaggctcatgaaatacaggcactggctaaagaactcgaacaattcccatgtgtcttgcctgacaagttcgtggccggcggtattatcgctaaactgccaccttcttggacggactttgctaccactctaaaacataagagacaagagtttagcgtggctgagcttattggttctcttgatgttgaggagagggcgagagcaaaagacactcgtggaaaaggagttgagacttctagtgccaatatggtacaaaagaagaactccaatgcatcacataataataaaaagaagaacaagcaacagaatgccacgaagcccaagcaggcagcctcgttcaaaaagaagaacaaaggagctggttgctttgtttgcgggagtactgatcattgggcaagcgcttgtccagactgcaaatttaagcaagagaaaaaaccagctcaagagaagaaaacagtaaacatggttgttagcgagactgcagaaggaacatcggggtatggtaatcttttacctactgttctttcagtgtgtcaatcccctgagtggtgggctgataccggtgctaatattcatgtgtgtgctgatatttctttattttcttcttatcagtgcaaagggactggagccttgctgatggggaacggatcacatgcgcgtgttcttggtgttggtacagtcattctgaagtttacttcgggaaagacggtgctattgaagaacgtgcagcatgtcccctccatcaaaaagaatctagttagtggctctcaattgtgtcgagatggctacaaaattgtctttgagtctaataaatgtatactgtctaagtatggaacgtttgttggaaaaggctatgacagcggaggcttgttccgcttatctttgcatgatgcgtgtaataagtctgtgaacaatgttgtttcgaatgagtcgtatatttggcattcacgactttgtcatatcaattttggttgtgtgtcgcggttagcagatttaaatttaatcccgaaatttgatttagtcaaaggttctaagtgccaggtgtgcgtgcaatctaagcaacctcgcaagcctcacaaggctgcagaggcgaggaatttggcaccactagacttaatacattccgatttatgtgagatgaacggaatattgactaaaggaggcaagcgatattttattacttttatcgatgactctactagattttgttatgtgtatctcttaaaatcaaaagatgaagctttgcattattttaagacctacaaagctgaagttgaaaatcaactcgagaggaaaattaaacggttaaggtctgatcgtggtggagaatatttttcgggtgatttttctgatttttgtgtggaacatggtattattcatgagaggacaccgccatactcaccacaatccaatggggttactgaaagaaagaaccgtactctaactaatttggttaacgccatgttagagacttcagggctatctaaggaatggtggggtgaggcgatcttgacggcgtgtcatgtcctgaataaagttcccacaaagaacaaagaaatcacaccattcgaggaatgagaaaagaagaaattaaatatctcctatttgcgcacctggggttgtttggataaagtgaatgtgccaattaacaagaagcgcaaattaggaccgaaaactgttgattgtgttttccttgggtatgctttccacagcattggatataggtttttaattataaactctggagtaccggacatgttggttggtacaattatggagtccagagatgctacgttttttgaggacgaatttcccatgaaagctacacatgatacgtctaatgatgaaccaacgataccccatgagcattttattccggtagaacacactgaggaatcccatatacataatcatgtggaaaatgacaatgtatcaactcgaaagagtaagagaccaaggattgcaaagtcctttggtgatgattacattgtatatcttgtggatgacacaccaagtaccattgaagaggcatattcctctcctgatgctgacttttggaaggaagcaataaggagtgagatggattctattatgtctaatgcaacttgggaggtagttgagcgtccttatgggtgtaagcccattggaagtaaatgggtgttcaaggaaaaacttaggcctgatggtactattgaaaggtacaaggcgaggcttgtaattaaaggctattcacagaaggaaggtgaggatttctttgatacttattcacctgtggctcgattgaccacaattcgtgtgctactttctttggctgcctctcatggtctactcgtccatcaaatggatgttaagacagcattcctaaatggagagctagatgaggaaatttacatggagcagccagctgggtttgtagcaaacggtcaagaaggcatggtgtgtaaattattgaaatctttatatggcctaaaacaagcacctaagcaatggcatgaaaagttcgatagaactttgacatctgccggttttgttgtgaacgaagcagacaagtgtgtatactatctgtcggggaccataattaggggtaccctcaagacgcctaattctcagctggtaacccccatcagcataaagctgcaaaggcctgatgggtacgattaagtcagggatcggtccacacgagtgactcgatcacgcttcacccgagcctagcctcggccaagggcagccgacctcgagagacttctgtctcgcccgaggccccctttttacggcggacacatcaccggctcgcccgaggccttggcttcgctcagaagtaaccctgactaaatcgccacaccgactgaccaagttgcaggagcatttaacgcaaaggtggcctgacacctttatcctgacacgcgccccccccccccccggcagagccgaagtgaccgccgtcactccaccgctccactgaccagtctgacagaaggacagcgccgcctgcgccactccgactgcagtgccactcgacagagtgagtctgacaagcagtcgggccctgccaaaggcgccatgggaaactccactccgcccgaccccagggctcggactcgggctaaaacccggaagacggcgaactccgctccgcccgaccccagggctcggactcgggctaagacccggaagacggcgaactccgctccgcccgaccccagggctcggactcgggctaagacccggaagacggcgaactccgctccgcccgaccccagggctcggactcgggctaaaacccggaagacggcgaactccgctccgcccgaccccagggctcggactcgggctaagacccggaagacggcgaactccgctccgcccgaccccagggctcggactcgggctaagacccagaagacggcgaatctccgcctcgcccgaccccagggctcggactccgccctggcctcggccaaacgatctccgcctcgcccgacccgggggctcgggctcggcctcggcaacggaaggcaaactcgacctcgacttcggaggagcccccacgtcgccctgcctagggcacaggtccgccacgtcaacaggaagcgccatcaccaacctaccccgagccgacttgggacacgaaggacaagaccggcgtcccatctggccagctccgccggatgggcaatgatggcgcccccaagctctgtgacgacggcggctcttagctctcttacggcagcagagcgacgtcagcaaggactcgaccgctccaacagctgtccctccgccaggctccgtcgctcctccgacagccacgacatcacgccagcaaggtgccaagacctctccggctgccacattggcatgtacccagggcgctagctctctctctctctccgctagacacgtagcactctgctaccccccattgtacacctggatcctctccttacgactataaaaggaaggaccagggccttcttagagaaggttggccgcgcgggaccgaggacgggacaggcgctctcttggggccgctcgcttccctcacccgcgtggacgcttgtaaccccctactgcaagcgcacctgacctgggcgcgggacgaacacgaaggccgcgggacttccacctctctcacgctcgactccggccacctcgcctctccccccttcgcgctcgcccacgcgctcgacccatctgggctggggcacgcatcacactcactcgtcggcttagggaccccctgtctcgaaacactgacagttggcgcgccaggtagggcctgctgcgtgctgacgaacagctccccgtcaagctccagatgggcagtctccagcaacctctccggcccggggcggtgcttcgtttcgggactcttgagttcatgtccttcgacggcagctacgacatgatacttcttccaccgccgcgcgacgacgacaatggcggccgacagcccgcccgccggcggcggaatcgacgacatcttccccgcgtggtggaagagcaacattcgagctcactccgttctctcccccgccaacggaggaggaggcggggccgtcaaggccaggcgggaggccgcgcttcgttggccgtcgggcgaatcgacgcccccgacgccccgacggaaggcacgccggacgtcgacctcgcgttcaagacggaggcaagcgccgtccccccgcgacacgccgaccccaaacaagaagacgacgccagcgcgctcgcggaaagcctgcaggacgtcgccctcgtacctgagatgacggtgcaaccagtccccgatgtgactacgtcgctcctcgtcgaccaaaaggtaccaactaactcccatcttgcgtcatttcgactcggcctcgacccgccaaacgacctcgttttggcgggcgctctcattgaggcgagtgcaaccccactggggtttcgtatgcggtcgccttgggaccggctgacggacgtctcgacctacgggccctctgggtccgaggaagatgacgatcccagcatctgttgggatttctccggacttggcaaccccagtgccgtgcgggacttcatgaccgcatgtgactactgcctctccgactgttccgacgaaagccgcagccttggcgacgagagctgcggcccaagccgcgaatgtttccacatcgagctaggggatccctccgaaggcaaccatctcggcatgccggaggacggtgatcttcctaggccggtgcctcgcgccgacatcccacgggagctagctgtggtccccgctccggcgggggttacgacccacaactcgagcaagtccgcgaggtgcaggccaggctcaacgagggaacaggagcgcttgagccgatccgtcgggacgtcggacaggcatgggcgggccaacccctggccggagaaatatgccacctgccccaaggtctccagcaccgcgtcgccaacgatgtcagggtcaggccgccgcccgcatccagcggggttggtcagaacctggcagccgcagcgatgctcctccgcgcgatgccggagccatcaaccaccgagggtcagcgaatccagggagagctcaagaatcttctggaaggcgctgcggcccgacgggccgagagcactgcctcccgaaggcaaggataccctcggaacctcacgccgcgacttcccgattcatgcgggaagcctcggtctacaccgagcgcacgcgcaacaccgcgcctgcggccccgggccacctcggcaacgagcaccatcgacgcgaccgtcgggctcacctcgacgaaagggtgcgccgaggctaccaccccaggcgtgggggcgctacgacagcggggaggatcggagtccctcgcccgaaccacccggtccgcaggccttcagtcgggccatccgacgggcgccattcccgacccggttccgacccccggctactatcacgaagtactcgggggaaacgagaccggaactgtggctcgcggactaccgccttgcctgccaactgggtgggacggacgacgacaacctcatcatccgtaacctccccctgttcctctccgacactgcccgcgcctggttggagcacctgcctccggggcagatctccaactgggacgacttggtctaggccttcgctggcaatttccagggcacatacgtgcgccccgggaattcctgggaccttcgaagctgccggcaacagccaggggagtcgctttgggactacatccggcgattctcgaagcagcgcaccgagctgcccaacatcaccgactcggatgtcatcggcgcgttcctcgccggacgccggcaccacttgccgcgacctggtgagcaagctgggtcgcaagacccccaccagggcgagcgagctgatggacatcgccaccaagttcgcctctggccaggaggcggtcgaggctatcttccgaaaggacaaccagccccagggccgcccatcggaagaggctcccgaggcgtctgctccgcgcggcgtcaagaagaaaggcaagaagaagtcgcaatcgaaacgcgacgctgctgacgcggaccttgtcgccgccgccgagtacaagaaccctcggaagcccccggaggtgcaaacctcttcgacaagatgctcaaggagccgtgcccttaccatcaggggcccgtcaagcacaccctcgaggagtgcgttatgcttcggcgtcacttccacagggccgggccacccgccgagggtggcagggcccgcgacgacgacaagaacgaagatcaccaagcaggagagttccccgaggtccgcgactgcttcctgatctatggagggcatgcgacgaatgcctcggctcggcatcgcaagcaagagcgccgggaggtctgctcggtgaaggtggcggcgccagtctacctagactggtccgacaagtccatcaccttcgaccaggccgaccaccccgaccatgtgccgagcccggggaaatacccgctcgtcgtcgaccccgttgtcggcaatggcaggctcaccaaggtcctgatggatgggggcagctgcctcaacatcatctacgccgagaccctcaagctcctgcgcgtcgatctatcctccgtccgagctggcgctgcgcccttccacgggatcatccctgggaagcgcgtccagccctcgggcgactcgacctccccgtctgcttcgggacgccctccaacttccgaagggagaccctgacgttcgaggtggtcgggttccgaggaacctaccacgccgtactagggaggccatgctacgcgaagttcatggccgtccccagctacacctacctgaagctcaagatgccgggccccaacggggtcatcaccgtcgaccccacgtacaaacacgcgttcgaatgcgacgtggggtgcgtggagtacgccgaggccctcgccgagtccaaggccctcatcgccgacctggagaacctctccaaggaggtgccagacgtgaaacgccatgccggcaacttcgagccagcggagacggtcaaggccgtccctcttgaccccggtggcgacaccaccaagcagatccggatcggttccgggcccgaccccaaataggaagcagtgctcgtcgactttctccgcgcgaacgccgacgtctttgcgcggagtccctcggacatgcccggcataccgagggatgtcgccaaacactcgctggatatccgggccggagcccgacccgtcaggcagcctctgcgccgatttgacgaggagaagcgcaaagtgattggcgaagagatccacaagctaatggcagcagggttcatcaaagaggtattccatcccgaatggcttgccaaccctgtgcttgtgaggaagaaagggggaaatggcggatgtgtgtagactacactggtctcaacaaagcatgtccgaaggttccctaccctctgcctcgcatcgatcaaatcgtggattccaccgctgggtgcgaaaccctgtccttcctcgatgcctactcagggtatcaccagatccggatgaaggagtccgaccagcttgcgacttccttcatcacgccgttcggcatgtactgctacgtcaccatgccgttcggtttgaggaatgcgggcgcgacgtaccagcggtgcatgaaccatgtgttcggcgaacacatcggtcgcacagtcgaggcctacgtcgatgacatcgtagtcaagacaaggaaggcttccgacctcctctccgaccttgaagtgacattccgatgtctcaaggcgaaaggagtcaagctcaatcctgagaagtgtgtcttcggggtgcccgaggcatgctcctagggttcatcgtctccgagcgaggcatcgaagccaacccggagaagatcgcggccatcaccagcatgggacccatcaaggacttaaaaggtgtacagagggtcatgggatgcctcgcggccctgagccgcttcatctcgcgcctcggcgaaagaggtctgcctctgtaccgcctcttaaggaaggccgagtgtttcgcttggacccctgaggccgaggaagccctcggcaacctgaaggcgctccttacaaaggcgcatgtcttggtgcccccggcggatggagaagccctcttggtctacgtcgccgcgaccactcaggtggttagcgccgcgatcgtggtcgagaggcaagaggaagggcatgcattgcccgttcagaggccggtttacttcgtcagcgaagtgctgtccgagaccaagatccgctacccacaagttcaaaagctgctgtatgcagtgatcctgacaaggtggaagctgcgacactacttcgagtctcacccggtaactgtggtgtcatccttccccctgggggagatcatccagtgccgagaagcctcgggcaggatcgcaaagtgggcggtggaaatcatgggcgaaacgatctcgttcgcccctcggaaggccatcaagtcccaggtgttggcggacttcgtggccgaatgggtcgacacccagttgccgacggctccgatccaaccggagctctggaccatgtttttcgacaggtcgctgatgaagacaggagccggcgcgggcctgctcttcatctcgcccctcgggaagcacttgcgctacgtgctgcgcctccatttcccggcgtccaacaatgtggccgagtacgaagctcttgtcaacgggttgcggatcgccatcgagctaggggtcagacgcctcgacgcccgcggtgattcgcagctcgtcatcgaccaagtcatgaagaactcccactgctgcgacccgaagatggaggcctactgcgacgaggttcggcgcctggaagacaagttcttcgggctcgagctcaaccacatcgctcggcgctacaacgaaaccgcagacgagctggctaaaatagcctcggggcgaacgacggtcccccggacgtcttctcccgggatctgcatcaaccctctgtcaagatcgacgacgcgcccgagcccgaggtaccctcggctcagcccgaggcaccctcggcacagcccgaggtaccctcggcccccgagggcgaggcactggacgtcgaggaagagcagagcggggccacgccagatcgagattggcaggccccgtacatgcagtatcttcgccgaggagagctacccccgaccaagtcgaggctcggcgggtagcgcgactgatagtcgcctagaggggggtgaatagggcgaaactgaaatttacaaatataaacacaactacaagccgggttagcgttagaaatataaacgagtccgcgagagagggcgcaaaacaaatcgcgagcaaatgatgaagtgtgacacacggatttgttttaccgaggttcggttctctcaaacctactccccgttgaggaggccacaaaggccgggtctctttcaacccttccctctctcaaacggtccctcggaccgagtgagcttctcttctcaaatcaaagccgggaacaaaacttccccgcaagggccaccacacaattggtgcctcttgccttgattacaatggagttgtgatctcaagaacaattgagaaagaaaagaagcaatccaagcgcaagagctcaaatgaacacggcaaatcactctcactagtcactagggctttgtgtggaattggagaggatttgatctctttagtgtgtctagaattgaatgctagagctcttgtagtagttgagaagtggaaaacttggatgcaatgaatggtgggtggttggggtatttatagccccaaccaccaaacttgaccgttggctggaggcgtctgctcgatggcgcaccggacagtccggtgcacaccggacagtccggtgcccctgccacgtcatcactgccgttggattctgaccgttggagcttctgacttgtgggcccgcctgggtgtccggtgcacaccggacatgtactgtttgatgtccggtgcaccggcatgggcgattctgacttctgcgcgcgctgagcgcgcattaaatgctccgcagggagccgttggcgccgaaaagagccgttgctccgctgttacaccggacagtccggtgcacaccggacagtccggtgaattttagcggagcggctgccgcgcgaacccgaggctggcgagttctggagaccgcgcttccttggagcaccggacatgtccggtgcacaccggacagtccggtgaattatagcgcgccggctctcgagaattcccgagggcgaagagtttgagtctgagtcccctggtgcaccggacaggtactgttcactgtccggtggcacaccggacagtccggtgcgccagaccaggggtgccttcggttccccctttgctcctttattgaatccaaaacttggtctttttattggctgagggtgaaccttttacacctgtaaaatctatacacttgggcaaactagttagtccaattatttgtgttgggcaattcaaccaccaaaattatttaggaactaggtgtaagcctaattccctttcaatctccccctttttggtgattgatgccaacacaaaccaaagcaaatagagaagtgcataattgaactagtttgcataatgtaagtgtaaaggttgcttggaattgagccaatataactactttacaagatatgcatggaatgtttctttctttatttagcattttggaccacgtttgcaccacgagatttgtttttgcaaattcttttgtaaatccttttcaaagttcttttgcaaatagtcaaaggtaaatgaataagagtttgcaaagcattttcaatttcttttgacttaacaaaactccccctaaaagagatccacctcttagtgttcaagagggttttgatataccatttttgaaatactactttctccccttttgaacacaatagtataccaaatgataaatacttttggaaagcactaagtttttgaatttggtggtggtggtgcggtccttttgctttgggctcatttctccccctttttggcatgaatcgccaaaaacggaatcattagagccctcgaagtaatttcttcccctttggtcataagtaaatgagttaagattataccaaagacgaaatccggtccttttgctttgggcttttactttctcccccaaagataaggtccgtttagtggagcgatggcgaaggatgagttacggagtggaagcctttgtctttgccgaagactccaattccctttcaatacacctatgacttggtttgaaatagactcgaaaaacacattagtcatagcatatgaaagagatatgatcaaaggtattcaatgagctatgtgtgcaagctaacaaaagaaatttctagaatcaagaatattgagctcatgcctaagtctggtaaaagattgttcatcaagaggcttggtaaagatatcggctaattgatctttagtattaatgtaagaaatctcgatatccccttttgttggtgatccctaagaaaatgataccgaatggctatgtgcttagtgcggctatgctcgacgggattgtcggccattttgattgcactctcattatcacatagcaaagggactttggttaatttgtaaccatagtcccgcagggtttgcctcatccaaagcaattgcgcgcaacaatgacctgcggcaatgtactcggcttcggcggtggaaagagcgaccgaattttgcttctttgaagcccaagacaccaaggatcttcccaagaactggcaagtccccgatgtgctcttcctattgattttgcaccccgcccaatcggcatccgaataaccaatcaaatcaaatgtggatccccgagggtaccaaagcccaaacttaggtgagtaagccaaatatctcaagattcgttttacggccgtaaggtgggattccttagggtcggattggaatcttgcacacatgcatacggaaagcataatgtccggtcgagatgcacataaataaagcaatgaaccaatcatcgaccggtataccttttgatccacggacttacctcctgtgtcgaggtcgagatgcccattggttcccatgggagtcttgatgggcttggcatccttcattccaaacttggttagaatgtcttgagtgtacttcgtttggctaatgaaggtgccctcttggagttgcttgacttggaatcctagaaaatacttcaactcccccatcatcgacatctcgaatttctgtgtcatgatcctactaaactcttcacatgtagactcgttagtagacccaaatataatatcatcaacataaatttggcatacaaataagtcattttcaagagttttagtgaagagtgtaggatcggccttgccgactttgaagccattagaaataaggaaatctcttaggcattcataccatgctcttggggcttgcttgagcccataaagcgccttagagagcctatagacatggttagggtactcactgtcttcaaagccgggaggttgctcaacgtagacctcttccttgattggtccgttgaggaaggcacttttcacgtccatttgatagagcttaaagccatggtaagtagcataggccaataatatgcgaattgactcaagcctagctacgggtgcataggtttcaccgaaatccaaaccttcgacttgtgaataccctttggccacgagtcgagctttgttccttgtcaccacaccatgctcatcttgcttgttgcggaagacccatttggttcctacaacattttggttaggacgtggaactaaatgccatacctcattcctcgtgaaattgttgagctcctcttgcattgccatcacccaatccgaatcttgaagtgcttcctctaccctgtgtggctcaatagaggaaacaaaagagtaatgttcacaaaaatgtgcaacacgagatcgagtggttaccccttatggatgtcgccgaggatggtgtcgacggggtgatctcgttggattgcttggtggactcttgggtgtggcggccttggttcttcctcatcctccttttcttgatcatttgcatctccccttgatcattgccattatcttgaggtggctcatcttcttgattttgcccttcatcaacttgagcctcatcctcattttgagttggtggagatgcttgcatggaggaggacggttgatcttgtgcatttggaggctcttcggattccctaggacacacatccccaatggacatgttccttagtgctatgcatggagcctgttcttcacctatctcatcaagatcaacttgctctacttgagagccgttagtttcatcaaacacaacgtcacatgagacttcaactagtccagtggacttgttaaagaccctatatgcccttgtgtttgagtcataaccaagtaaaaagccttctacagttttaggagcaaatttagattttctacctcttttaacaagaataaagcatttgctaccaaaaactctaaagtatgaaatgttgggctttttaccggttaggagttcatatgatgtcttcttgaggattcagtgaagatataaccggttgatggcgtagcaggcggtgttgaccgcttcggcccaaaaccggtccggtgtcttgtactcatcaagcatggttcttgccatgtccaatagagttcgattcttcctctccactacaccattttgttgtggcgtgtagggagaggagaactcatgcttgatgccctcctcctcaaggaagctttcaatttgagagttcttgaactccgtcccgttgtcgcttcttattttcttgatctttaagccgaactcattttgagcccgtctcaagaacccctttaaggtctcttgggtttgagatttttcctgtaaaaagaatacccaagtgaagcgagaataatcatccactattacaagacaatacttactcccgccgatgcttatgtaagcaatcgggctgaaaaggtccatgtggagtagctcaagtggcctgtcggtcgtcatgatgttcttgtgtggatgatggactccaacttgcttccctgcctggcatgcgctacaaatcctgtctttctcaaaatgaacatttgttaatcctaaaatgtgttctccctttagaagcttgtgaagattcttcatcccaacatgggctagtcggcggtgccagagccaacccatgttagtcttagcaattaagcatgtgtcgagctcagctctatcaaaatctactaagtatagctgaccctctaacacacccttaaatgctattgaatcatcacttcttctaaagacagtgacacctacatcagtaaagagacagttgtagcccatttgacataattgtgaaacagaaagcaagttgtaatctaaggaatcaacaagaaaaacattggaaatagaatggtcaggagatatagcaattttaccaagtcctttgaccaaaccttgatttccatccccgaatgtgatagctcgttggggatcttggtttttctcatatgaggagaacatccttttctccccggtcatgtggtttgtgcacccgctgtcgagtatccaacttgagcccccggatgcataaacctacaaaacaattttagttcttgactttaggtacccaaacggttttgggtcctttggcattagacacaagaactttgggaacccaaacacaagtcttggaacccttgtgtttgcccccaacaaacttggcaacgaccttgccggatttgttagtcaaaacatatgatgcatcaaaagtcttaaatgaaatgctatgttcatttgatgcattagaaattttctttctaggcaacttggcacgggttggttgcctagagttagatgtctcacccttatacataaaagcatgattagggccagagtgagacttcctggaatgaattttcctaattttgctctcgggataaccggcagggtacaaaatgtaaccctcgttatcctgaggcatgggagccttgcccttaacaaagttagacaaatttttaggaggggcattaagtttgacattgtctcccctttggaagccaatgccatccttaatgccagggcgtctcccattataaagcatgctacgagcaaatttaaatttctcattttctaggttgtgctcggcaattttagcatctagttttgctatatgatcattttgttgtttaattaaagccatatgatcatgaatagcatcaatatcaacatttctacatctagtacaaatagatacatgctcaacaatagatgtagatggtttgcaagaatcaagttcaacaatcttagcatgaagaatatcatttttatctctaagattggcaatggtaactttgcaaacgtcaaaatctttagccttagcaatcaaactttcattctctaatctaaggctagcaagagaaatgtttaattcttcaatcctagcaagcaaatcatcattattatttctaggattgggaattgaaacattacaaacatgagaatcaaccttagcatttaaactagcattttcatttctaaggttgtcaatcatctcacggcaagtgcttagctcactagataatttttcacatttttctacttctagagcataagcctttttaaccttaacatgtttcttgttttctttaattagacaatcctcttgggagtccaaaaggtcatccttttcatgaatagcactaactaattcatttaatttttctttttgagctatgttaaggttggcaaaaagggaacgcaaattatcctcctcatcactagcattatcatcactagaagattcatatttagtggaggagttagatttaacctttttccgtttgccgtcctttgccatgaggcacttgtggccgacgttggggaagaggagtcccttggtgacggcgatgttggcggcgtcctcgtcgtcggaggagtcgcttgagctttcgtcggaatcccattcccgacaaacatgggcatcgccgcccttcttcttgtagtaccttttcttctcctttcttctccccttcttgtcgtcgcctcggtcactgtcactagatataggacatttagcaataaaatgaccgggcttaccacacttgtagcaaaccttcttggagcgggacttgtaatccttccccctcctttgcttgaggatttggcggaaactcttgatgacgagcgccatttcctcattgtcgagtttggaggcgtctattggttgtcgacttggtgtagactcctcctccttctcctccgttgccttgaatgcaacgggttgggcttcggatgggtcgccaagctcgttgattttcctcgagccttctatcatgcactcaaaacttacaaaatgcccgataacttcctcgggggtcattttagtatatctaggattgccatgaatcaattgaacttgagtgggattaagaaaaatgagagatcttaaaataacatttaccacttcgtggtcgtcccacttcttgctcccgaggttgcgcacttggttcaccaaagtcttgagccggttgtacatgtgttgtggctcctcccctttgtgaagccggaaccgaccgagctccccctcgatcgtttcccgcttggtgatcttggtgagctcatctccctcgtgcgcagttttgagcacatcccaaatctccttggcgctcttcaacccttgcactttgttatactcttctctacttaaagaggcgagaaatatcgttgtcgcttgagagttgaagtgctcgatttgggccacctcatcctcatcatagttctcatcccctatggatggtacctgcgcaccaaactcaacaacatcccatatgcttttgtggagcgaggttagatgaaatcgcattaaatcgctccacctagcgtaatcttcaccatcaaaagttggtggtttgcctaatgggacggaaagtaaaggtgtatgtttggaaatgcgagggtagcgtagggggatcttactatacttcttgcgctcttggcgcttaaaagtgacggagggcgcatcggagtcggaggtcgatgttgatgaagtgtcggtctcgtagtagaccaccttcctcatcctcttgtgcttgtcgcctttccgatgcggcttgtgggaagaagatttttccttcttctctttgtggtgagaagaagatttcttctccttccctttgtgggaggagctcttcttcttctccctccttttggtgcgggactcttccgatgaagtgctcccgtggcttgtagtgggcttttcgccggtctccatctccttcttggcgtgatctcccgacatcacttcgagcggttaggctctaatgaagcaccgtgctccgataccaattgatagtcgcctagaggggggtgaatagggcgaaactgaaatttacaaatataaacacaactacaagccgggttagcgttagaaatataaacgagtccgcgagagagggcgcaaaacaaatcgcgagcaaatgatgaagtgtgacacacggatttgttttaccgaggttcggttctctcaaacctactccccgttgaggaggccacaaaggccgggtctctttcaacccttccctctctcaaacggtccctcggaccgagtgagcttctcttctcaaatcaaagccgggaacaaaacttccccgcaagggccaccacacaattggtgcctcttgccttgattacaatggagttgtgatctcaagaacaagtgagaaagaaaagaagcaatccaagcgcaagagctcaaatgaacacggcaaatcactctcactagtcactagggctttgtgtggaattggagaggatttgatctctttagtgtgtctagaattgaatgctagagctcttgtagtagttgagaagtggaaaacttggatgcaatgaatggtggggtggttggggtatttatagccccaaccaccaaacttgaccgttggctggaggcgtctgctcgatggcgcaccggacagtccggtgcacaccggacagtccggtgcccctgccacgtcatcactgccgttggattctgaccgttggagcttctgacttgtgggcccgcctgggtgtccggtgcacaccggacatgtactgtttgatgtccggtgcaccggcatgggcgattctgacttctgcgcgcgctgagcgcgcattaaatgctccgcagggagccgttggcgccgaaaagagccgttggcgccgaaaagagccgttgctccgctgttacaccggacagtccggtgcacaccggacagtccggtgaattttagcggagcggctgccgcgcgaacccgaggctggcgagttctggagaccgcgcttccttggagcaccggacatgtccggtgcacaccggacagtccggtgaattatagcgcgccggctctcgagaattcccgagggcgaagagtttgagtctgagtcccttggtgcaccggacaggtactgttcactgtccggtggcacaccggacagtccggtgcgccagaccaggggtgccttcggttccccctttgctcctttattgaatccaaaacttggtctttgatagtcgcctagaggggggtgaatagggcgaaactgaaatttacaaaaaataatcacaactacaagccggggttagcgttagtaataataaatgagtcctcaagagagggcgcaaaacaaatcgcaagcaaataaagagagtgacacgtggatttgttttaccgaggttcggttcttgcaaacctactccccgttgaggaggccacaaaggccgggtctctttcaacccttccctctctcaaacggtccctcggaccgagtgagctttccttcttctcaatcaaccgggaacaaagcttccccgcaagggccaccacacaatcggtgcctcttgccttggttacaattgagtgttgatcacaagagcataagagaaagaaagaatgcgatccaagcgcaagagctcaaaagaacacggcaaatcactctcactagtcactagggttttgtgtggaattggagaggatttgatctctttgaatgtgtctagaattgaatgcctagctcttgtaagtggttgagaagtggaaaacttggatggctatgaatgtggggtggttggggtatttatagccccaaccaccaaacatgaccgttggctggaggcttctgttcgatggcgcaccggacagtccggtgcacaccggacagtccggtgcccctgccacgtcatcgttgccgttggattctgaccgttggagcttctgacttgtgggcccgcctgggtgtccggtgcacaccggacatgcactgtttgatgtccggtgcaccggtatgggcagccctgacgtctgcgcgcgctgcgcgcgcatttaatgcaccgcagggagccgttggcgccgcagggagccgttgctccgctggcacaccggacagtccggtgcacaccggacagtccggtgaattatagcggagcggctgccgcgcgaacccgaggctggcgagttcaggaggccgagcttccttggagcaccggacatgtccggtgcacaccggacagtccggtgaattatagcgcgccggcctccacgaattcccgagggcgaagggttggagtctgagtcccctggtgcaccggacaggtactgttcactgtccggtggcacaccggacagtccggtgcgccagaccaggggtgccctcggttgcccttttgctcctttattgaatccaaacttggtctttttattggctgagtgtgaaccttttacacctgtataatctatacacttgggcaaactagttagtccaaagatttgtgttggacaattcaaccaccaaaattatataggaactaggtgtaagcctaattccctttcaatctccccctttttggtgattgatgccaacacaaaccaaagcaaatatagaagtgcataattgaactagtttgcataatgtaagtgtaaaggttgcttggaattgagccaataaaactacttacaagatatgcatggaatgtttctttcttatataacattttggaccacgtttgcaccacttgttttgtttttgcaaaaccttttgtaaatccttttcatagatcttttgcaaatagtcaaaggtaaataaatgagagtttgcaaaagcattttcaagatttgaaatttcctccccttgtttcaaatgctttttcctttgactaaacaaaactccccctaaaagagatccacctcttagtgttcaagagggttttgatatactactttctcccctttttgagcaaaataggataccaaatgataaatatttttagaaagcactaagtttttaaatttggtggtggtggtgcggtccttttgctttgggctcatttctccccctttttggcatgaatcgccaaaaacggaatcattagagcccttgaagtgcaatcttcccctttggtcataaataagtgagttaggattataccaaagacgaagtccttttgcgtttgagcttttactctctcccccaaggatgaagtccttttccttgatgctcatttctcccccaaagacgagagagttgctcggagtgatggcgaagtatgagttacggagtggaagcctttgtcttcgccgaagactccaattccctttcaatatacctatgacttggtttgaaataaacttgaaaacacattagtcatagcatataaaagagatatgatcaaaggtattcaaatgagctatgtgtgcaagcttagcaaaagaaatttctagaatcaagaatattgagctcatgcctaagtctggtaaaagattgttcatcaagtggcttggtaaagatatcggctaattgatctttagtgttaatgtaagaaatctcgatatccccttttgttggtgatccctaagaaaatgataccgaatggctatgtgcttagtgcggctatgctcgacgggattgtcggccattttaattgcactctcattatcacatagcaaagggactttggttaatttgtaaccgtagtcccgcagggtttgcctcatccaaagcaattgcgcgcaacaatgtcctgcggcaatgtactcggcttcggcggtggaaagagcgaccgaattttgcttctttgaagcccaagacaccaaggatcttcccaagaactggcaagtccccgatgtgctcttcctattgattttgcaccccgcccaatcggcatccgaataaccaattaaatcaaatgtggatcccctagggtaccaaagcccaaacttaggagtgtaagccaaatatctcaagattcgttttacggccgtaaggtgggattccttagggtcggattggaatcttgcacacatgcaaacggaaagcataatgtccggtcgagatgcacataaataaagcaatgaaccaatcatcgaccggtataccttttgatccacggacttacctcccgtgttgaggtcgagatgcccattagttcccatgggtgtcttgatgggtttggcatccttcatcccaaacttagcaagaatgtcttgagtgtacttcgtttggctaatgaaggtgccctctcggagttgcttgacttggaatcccagaaaatatttcaactcccccatcatcgacatctcgaatttctgtgtcatgatcctactaaactcttcacatgtagactcgttagtagacccaaatataatatcatcaacataaatttggcatacaaacaagtcattttcaagagttttagtaaagagtgtaggatcggccttgccaactttgaagccattagcaataaggaaatctcttaggcattcataccatgctcttggggcttgcttgagcccataaagcgccttagagagcctatagacatggttaggatacttactgtcttcaaagccgggaggttgctcaacatagacctcttccttgattggtccattgaggaaggcacttttcacgtccatttgataaagcttaaagccatggtaagtagcataggctaataatatgcgaattgactcaagcctagctacgggtgcataggtttcaccgaaatccaaaccttcgacttgtgaataccctttggccacgagtcgagctttgttccttgtcaccacaccatgctcatcttgcttgttgcggaagacccatttggttcctacaacattttggttaggacgtggaactaaatgccatacctcgttcctcgtgaaattgttgagctcctcttgcatcgccaccacccaatccgaatcttggagagcttcctctaccctgtgtggctcaatggaggaaacaaaagagtaatgttcacaaaaatgagcaacccgagatcgagtagttacccccttatgaatgtcgccgaggatggtgtcgacggggtgatctcgttggattgcttggtggactcttgggtgtggcggtcttggttcttcctcatcctccttttcttgatcatttgtatctcccccttgatcattgctatcatcttgaggtggctcgtcttcttgattttgctcttcatcattttgagcctcatcctcattttgagttggtggagatgcttgcatggaggaggatggttgatcttgtgtacttggaggctcttcggattccttaggacacacatccccgatggacatgttccttagcgcgatgcatggagcctgttcttcacctatctcgtcaagatcaacttgctctacttgagagccgttagtttcatcaaacacaacgtcacaagagacttcaactagtccagtggacttgttaaagaccctatatgcccttgtgtttgagtcataaccaagtaaaaaaccttctacagttttaggagcaaattttgattttctacctcttttaataagaatgaagcatttgctaccaaaaactctaaaatatgaaatattgggctttttaccggttaggagttcatatgatgtcttcttgaggatttggtgaagatataaccggttgatggcgtagcaggcggtgttgactgcttcggcccaaaaccggttcggtgtcttgtactcatcaagcatggttcttgccatgtccaatagagttcgattcttcctctccactacaccattttgttgtgacgtgtagggagaagagaactcatgcttgatgccctcctcctcaaggaagctttcaatttgagagttcttgaactccgtcccattgtcgcttcttattttcttgatccttaagccgaactcattttgagctcgtctccagaatccctttaaggtctcttgggtttgagatttttcctgtaaaaagaatacccaagtgaagcgagaataatcatccacaataactagacagtacttactcccgccgatgcttatgtaagcgatcgggccgaatagatccatgtgtaggagctccagtggcctgtcagtcgtcattatgttcttgtgtggatgatgagtgccaacttgcttccctgcttggcatgcgctacaaatcctgtctttctcaaaatgaacattggttagtcctaaaatgtgctctccttttagaagcttatgaagattcttcatcccaacatgggctagtcggcggtgccagagccaacccatgttagtcttagcaattaaacatgtgtcgagctcagctctatcaaaatctactaagtatagctgaccctctaacacacccttaaatgctattgaatcatcacttcttctaaagacagtgacacctatatcagtaaaaagatagttgtagcccatttgacataattgggaaacagaaagcaagttgtaatctaatgaatcaacaagaaaaacattggaaatggaatggtcaggtgaaatagcaattttacccaaacctttgaccaacccttgatttccatccccaaatgtgatagctcgttggggtctttgtttttctcatatgaggagaacatccttttctccccggtcatgtggtttgtgcacccgctgtcgagtatccaacttgagcccccggatgcataaacctacaaaacaaatttagttctttgttttaggtacccaaacggttttgggtcctttagcattagatacaagaactttgggtacccaaacacaagtcttggagcctttgtgtttgcccccaacaattttggcaactaccttgccagatttgctagtcaatacataagatgcatcaaaagttttaaatgaaatggcatgatcatttgatgcattaggagttttctttctaggcaacttggcacgggttggttgcctagagctagatgtctcacccttatacataaaagcatggttagggccagagtgagacttcctagagtgaattctcctaattttgctctcgggataaccggcagggtacaaaatgtaaccctcgttatcctgaggcatgggagccttgcccttaacaaaattagacaaatttttaggtggggcattaattttgacattgtctcccctttgaaagccaatgccgtccttaatgcccgggcgtctcccattatagagcatgcttctagccaatttaaatttttcattttctaagtcatgctctctaattttagcattaagttgtgctatgtgatcattttgttttttaattaaggcaaggtgatcatggatagcatcaacattaatatctctacatctagtgcaaatggacacatgctcaatagtagatgtagagggtttgcaagactttaattcaataaccttagcatgcaacaaatcattcttagttctaaggtcagaaatagtagtattgcaaacatcaaaatccttagccttagcaattaatttctcattctcatttctaaggctagcgatggaagcattcaattcatcaatcctagcaagcaaatcaacatcatcatttctaggatcaatgcaaacatgagaatcaaccttagccaacaaattagcattttcatttctaaggttgtctagaatctcatggcaagtgcttagctcactagataatttttcacatttttctctttctagagcataagcatttttaaccttaacatgtttcttattttccttgattaggaaatcctcttgggagtccaagagatcatccttttcatggatagcactaattagctcatttaatttttccttttgttccatgttaaggttggcaaaaagaatacgcaagttatcctcctcatttttatcatcctcatcactagatgtttcatatttagtggaggactttgattttaccttctttttgccgtccttggccatgaggcacttgtggccgacgttggggaagaggaggcctttggtgacggcgatgttggcggcgtcctcgtcgtcggaggagtcgcttgagctttcgtcggagtcccactcccgacaaacatgggcatcgccgcccttcttcttgtagtacttcttcttctccttcctcttgcccttcttgtcgttgtccctgtcactgtcacttgataatggacatttagcaataaagtgaccgggcttaccacacttgtagcaaaccttcttggaacgggatttgtagtccttccccttccgttgcttgaggatttgccggaagcttttgatgattagggccatctcctcgttgtcgagcttggaggcgtcaattggttgtctacttggtgtagactcctcctccgttgccttgaaggccacgggttgcgcctcggatgtggaaggctcatcaagctcgttgatcttcttggagcccttaatcatgcattcaaaactaacaaaattcccgatgacttcctcgggggtcatttgtgtatatctaggattgccacgaattaattgtacttgagtagggttaaggaaaataagggctctcagaataaccttaaccacttcgtggtcatcccattttgtgctcccgaggttgcgcacttggttcaccaaggtcttgagccggttgtacatgtcttgtggctcctccccttggcgaagacggaagcgaccgagctccccctcgatcgtttcccgcttggtgatcttggtgagttcatcaccttcatgcgccgtcttgagtaggtcccaaatctccttggcgttcttcaacccttgtactttgttgtattcctccttgcttaaagaggcaaggagaatggttgtggcttgagagttgaagtgctcgatttgggccacttcgtccgtgtcgtagtcctcatcccctacggatggtacctgtacaccatactcaacaacatcccataatcttttgtggagagaggttagatgaaatcgcatcaaattactccacatagcataatcttcaccattaaaagttggtggtttgcctaatgggacggaaagtaaaggtgtatgtttaggaacgcgagggtagcgtaggggatcttactatacttcttacgctcttggcgtttagaagtgacggacgccgcgtcggagccggaggtggagatcgatgaagtgtcggtctcgtagaagaccaccttcctcatccttttgtgcttgtccccactccgatgcggcttgtgagaagatttttccttcttctccttatggtgagaagaggaagatcttttctccttccgcttggaggatttcttcttcttctctcttctcttggtgcgggattcttccgatgaagatgaagtgctcccttggcttgtagtaggcttgtcgtcgccggtctccatctccttcttggcgtgatctcccgacatcacttcgagcggttaggctctaatgaagcaccgggctccgataccaattgatagtcgcctagaggggggtgaatagggcgaaactgaaatttacaaaaaataatcacaactacaagccggggttagcgttagtaataataaatgagtcctcaagagagggcgcaaaacaaatcgcaagcaaataaagagagtgacacgtggatttgttttaccgaggttcggttcttgcaaacctactccccgttgaggaggccacaaaggccgggtctctttcaacccttccctctctcaaacggtccctcggaccgagtgagctttccttcttctcaatcaaccgggaacaaagcttccccgcaagggccaccacacaatcggtgcctcttgccttggttacaattgagtgttgatcacaagagcataagagaaagaaagaatgcgatccaagcgcaagagctcaaaagaacacggcaaatcactctcactagtcactagggttttgtgtggaattggagaggatttgatctctttgaatgtgtctagaattgaatgcctagctcttgtaagtggttgagaagtggaaaacttggatggctatgaatgtggggtggttggggtatttatagccccaaccaccaaacatgaccgttggctggaggcttctgttcgatggcgcaccggacagtccggtgcacaccggacagtccggtgcccctgccacgtcatcgttgccgttggattctgaccgttggagcttctgacttgtgggcccgcctgggtgtccggtgcacaccggacatgcactgtttgatgtccggtgcaccggtatgggcagccctgacgtctgcgcgcgctgcgcgcgcatttaatgcaccgcagggagccgttggcgccgcagggagccgttgctccgctggcacaccggacagtccggtgcacaccggacagtccggtgaattatagcggagcggctgccgcgcgaacccgaggctggcgagttcaggaggccgagcttccttggagcaccggacatgtccggtgcacaccggacagtccggtgaattatagcgcgccggcctccacgaattcccgagggcgaagggttggagtctgagtcccctggtgcaccggacaggtactgttcactgtccggtggcacaccggacagtccggtgcgccagaccaggggtgccctcggttgcccttttgctcctttattgaatccaaacttggtctttttattggctgagtgtgaaccttttacacctgtataatctatacacttgggcaaactagttagtccaaagatttgtgttggacaattcaaccaccaaaattatataggaactaggtgtaagcctaattccctttcagtctttttattggctgagggtgaaccttttacacctgtaaaatctatacacttgggcaaactagttagtccaattatttgtgttgggcaattcaaccaccaaaattatttaggaactaggtgtaagcctaattccctttcagcgacgcgccaagtcgttcgtcttgctgggcgatgaagaggagctctaccatcgcagcccctcgggcatcctccagcgatgcatctccatcgccgaaggtcgggaactgctgcaagaaatacactcgggggcttgcggccatcacgcagcaccccgagcccttgtcgggaatgctttccgacaaggcttctactggccaacggcggtggatgacgccactagaattttccgcacctgcgaagggtgccaattctatgcgaagcagacccacctgcccgctcaggctctgcagacaatacccatcacctggcccttcgctgtatggggtctggacctcgtcggtcccttgcagaaggcgcccggggctacacgcacctgctggtcgccatcgacaaattctccaagtggatcgaggtccgacctctgaacagcatcaggtccgagcaggcggtggcgttcttcaccaacatcatccatcgcttcggggtcccgaactccatcatcaccgacaacggtacccagttcaccccgtcgcattaactctgcggcgggacacgcggcgcctctggcgggagaagcgcgcgacgcttcgccttcgccgtaataaccgcgtcaaaaagaggtacgccacgtcgttcggtttcgtatcctcttcctttttcctctttctctatctcttgcaacagggaccgggaaaggggataccccgaaaaggacccttctccgcgaaggaaccgggctccgagcccccctactgatcaggggttcgaagactggccctccgaagggttcaacagtcgccttagatcgcgtgggcccgacacccactactggtcaggggttcgaaggccagcccccaaagggttctatggccgcctcaggctactcgggctccgcgcccattactgatcaggggttcgaaggctggcccccgaagggttcacagtcgcctcagacaccgagcgagggatgaccaggggtacgttcgatacataaccgaggctcgggctgcgctcccgaggtaccctaggacatttccgagaccagcgggaacgatcttgtaacggaatcccatcggagggaggcatcgagccctcggaccccgtcgccaggggaccgggtccggcaaatcacccgcaggtacttttgggcgtgcctctgggcccctagccgacccccaacgaacggggcacggacgtccactcggattacccgcttgcagctcaccggagacaccatgttcgatgcccatcgagggtaacatggcgcactcccccctcctccttgcggaaaggcgacgtaggggcgtatgtaaaaagccgagtctgtccctgatcgtcctctcgccctgtgcagaggctcgggggctgctctcgcgaaaaccggctccggccgaaccgttgacagcgtcaacataccagcccgagagcttgggccccgaccgtgcacccgggctacggccagttcgcatgagggaacgaccagaccagccgaagcgttacgcaaggtattaagacctcgaaggagtgtaaccactcctccgaggcctcggggctacacccggcgggtgcgctcgcgcgcacccaccggaacgaaatgcaaccgagaaaggctggtccccttgcaaaaaagtgcgacgaaagcctccaagcgagtgctaacactcccttcgaggctcgggggctactgtcggggaccataattaggggtaccctcaagacgcctaattctcagctggtaacccccatcatcataaagctgcaaaggcctgatgggtacgattaagtcagggatcggtccacacgagtaactcgatcacgcttcacccgagcctagcctcggccaagggcagccgacctcgagagacttccgtctcgcccgaggcccccctttttacggcggacacatcaccggctcgcccaaggccttggcttcgctcagaagtaaccctgactaaatcgccacaccgactgaccaagttgcaggagcatttaacgcaaaggtggcctgacacctttatcctgacacgcgccccccggcagagccgaagtgaccgccgtcactccaccgctccactgaccagtctgacagaaggacagcgccgcctgcgccactccgactgcagtgccactcgacagagtgagtctgacaagcagtcgggccctgccaaaggcgccatgggaaactccgctccgcccgaccccagggctcggactcgggctaaaacccggaagacggcgaactccgctccgcccgaccccagggctcggactcgggctaagagccggaagacggcgaactccgctccgcccgaccccagggctcggactcgggctaagacccggaagacggcgaactccgctccgcccgaccccagggctcggactcgggctaagacccggaagacggcgaactccgctccgcccgaccccagggctcggactcgggctaagacccggaagacggcgaactccgctccgcccgaccccagggctcggactcgggctaagacccggaagacggcgaactccgctccgcccgaccccagggctcggactcgggctaagacccggaagacggcgaatctccgcctcgcccgaccccagggctcggactccgccctggcctcggccaaacgatctccgcctcgcccgacccggggctcgggctcggcctcggcaacggaaggcaaactcgacctcgacttcggaggagcccccacgtcgccctgcctagggcacaggtccgccacgtcaacaggaagcgccatcaccaatctaccccgagccgacttgggacacgaaggacaagaccggcgtcccatctggccagctccgccggatgggcaatgatggcgccccccaagctctgtgacgacggcggctcttagctctcttacggcagcagagcgacgtcagcaaggactcgaccgctccaacagctgtccctccgccaggctccgtcgctcctccgacagccacgacatcacgccagcaaggtgccaagacctctccggctgccacattggcatgtacgcagggcgctagctctctctctctctctctccgctagacacgtagcactctgctacccccattgtacacctggatcctctccttacgactataaaaggaaggaccagggccttcttagagaaggttggccgcgcgggaccgaggacgggacaggcgctctcttggggccgctcgcttccctcacccgcgtggacgcttgtaaccccctactgcaagcgcacctgacctgggcgcgggacgaacacgaaggccgcgggacttccacctctctcacgctcgactccggccacctcgcctctccccccttcgcgctcgcccacgcgctcgacccatctgggctggggcacgtagcacactcactcgtcggcttaggacccccctgtctcgaaacgccgacactatcggtatggtggggcgagggagtaattttatgcctatatgttgatgacattctaatcttggggacgagtcttgatgtgattaaagagacaaaagactttctgtctaataattttgaaatgaaagatttgggagaagctgatgttattcttaacattaagctactgagagaaggcattggtgggatcacacttgtgcaatcccattatgtggaaaaggttttgagtcgctttggttttagcgaatgtgaacctgctccaacgccttatgatcctagtaagctattaaagaaaaatcgaaggatagttagggatcaattgagatattcccaaataattggttcactcatgtatttagctagcgctacgaggcctaacatctcatttgctgtgagcaaacttagtcgatttgtttcaaatccgggagatgatcactggcgtgctcttgagagagttttgcgctatctaaagggtactatgagtttaggcatccattataccgggtacccaacagttctggagggttattgtgatgcaaactggatatctgatgctgatgagatatatgccacaagtggatatgtgttttcacttggaggtggtgctgtttcatggaagtcttgcaagcagaccatcttaacgaggtcgactatggaagcagaactcacagcattagataccgcttcagttgaggctgagtggcttcgtgaactccttatggatttaccggtggttgaaaaacctgtgccggctatttccatgaactgtgataatcagactgtgataattaagataaacagttctaaggataatatgaagtcgacaaggcacataaagaggcgtttgaaatctgtcaggaaattgagaaactccggagtaatagcgttggattatgtccatacgtctaaaaatctggcagatcaatttactaaggggctatcacgtagtgtgatagatagtgcatcaagtgagatgggcatgagacccacctaaagtttatcatagtggtaacctgttctatgtgatcggagatcccgtgaattagaatggtgaaacaagctagtggtagactgagaggaaagacccttaataaggctcatttcagatgcatatctttccttactgtaaggtaggttggtgtttacaccttaatatgttccaagtggctttgtgaagcaaagatgttgtcctacagaacatctttagaggaacatacctatatgggttaactgctagtcacagtttatgagatctgggtggtttctagatacccatgaaaggctatggagtttgacttatatgctccaaccagaggggatgcgttcaacaatctagtactggtaaagagtttagatgaaactcattccacgcaaaactgccaattcaaggcctagtccattgtgcagttgtggtcaagtgtagtctaagttctaggtggatgttcaacttaacagtctccatctaaacaccagtatatcaaacgtttgagatgatgagagcttttttgtgtgacttagcatttggtggggattgttggattaatgtgggcttggcccaaattaatattcaataatagtcaatgctaatggcccactttaatgctatggtgtactaattatttagtaccatattggaagttcaaaggacaaatcaatcaacttaaataggtggaccattggtgcatctattgagaagttgagaaaaggacgaaggactgccacacgcgcgcgccgccgccgccgccgccggccgggccaggccgggccgtgtccgtgttcgaatattcctttcaaacggttgcgcattttgcctggagcgatgaccgtcatgataaccgcccgtttcttgtcttatggctagtaacggacgtcagttactgtcgtcagtttccagttctaatgcgcgaccgtttctgtccgttgttcttctccctccttctgaccgcctataagaatggagagggagggctcttccagttatgcgaattatctcacacgaattgcaaacaacacattcccgtcccatcttctgcgagcacagagagagtgggagagcaggcctccgaaatcaccgaccgcagagatacacttgcacgggtgtgcgggcgatcagatttttggggagcgtcttcgcgactgctcgcgtgatctgtttgtccagctgcttcgttcacagcttgttgttcgtcgccttcccgagttgacgcgtgctgctgttcttcttcccggcgaccgttcgagggactgcacagcgtacatcttcctgcaccgacttcgtacggctacatcgaacaaacacacgagatgtctcgtgtgaatggagccactgatgccttgagcatcggtccctccgctgggtacactctgttcttcgtatttgtacatgtttcattgctgtttactacttatgcgagtagttatacacacatgcacatacatgtcatcacatatatcgcactgtttttctggattaaattaaaactaaaaatgcctaactttctaaca

SEQ ID NO: 72 - DNA, 5966 bp, synthetic construct
  misc_feature 1..5966: note = Cas9 expression construct
  source 1..5966: mol_type = other DNA
gtgcagcgtgacccggtcgtgcccctctctagagataatgagcattgcatgtctaagttataaaaaattaccacatattttttttgtcacacttgtttgaagtgcagtttatctatctttatacatatatttaaactttactctacgaataatataatctatagtactacaataatatcagtgttttagagaatcatataaatgaacagttagacatggtctaaaggacaattgagtattttgacaacaggactctacagttttatctttttagtgtgcatgtgttctcctttttttttgcaaatagcttcacctatataatacttcatccattttattagtacatccatttagggtttagggttaatggtttttatagactaatttttttagtacatctattttattctattttagcctctaaattaagaaaactaaaactctattttagtttttttatttaataatttagatataaaatagaataaaataaagtgactaaaaattaaacaaataccctttaagaaattaaaaaaactaaggaaacatttttcttgtttcgagtagataatgccagcctgttaaacgccgtcgacgagtctaacggacaccaaccagcgaaccagcagcgtcgcgtcgggccaagcgaagcagacggcacggcatctctgtcgctgcctctggacccctctcgagagttccgctccaccgttggacttgctccgctgtcggcatccagaaattgcgtggcggagcggcagacgtgagccggcacggcaggcggcctcctcctcctctcacggcaccggcagctacgggggattcctttcccaccgctccttcgctttcccttcctcgcccgccgtaataaatagacaccccctccacaccctctttccccaacctcgtgttgttcggagcgcacacacacacaaccagatctcccccaaatccacccgtcggcacctccgcttcaaggtacgccgctcgtcctcccccccccccctctctaccttctctagatcggcgttccggtccatgcatggttagggcccggtagttctacttctgttcatgtttgtgttagatccgtgtttgtgttagatccgtgctgctagcgttcgtacacggatgcgacctgtacgtcagacacgttctgattgctaacttgccagtgtttctctttggggaatcctgggatggctctagccgttccgcagacgggatcgatttcatgattttttttgtttcgttgcatagggtttggtttgcccttttcctttatttcaatatatgccgtgcacttgtttgtcgggtcatcttttcatgcttttttttgtcttggttgtgatgatgtggtctggttgggcggtcgttctagatcggagtagaattctgtttcaaactacctggtggatttattaattttggatctgtatgtgtgtgccatacatattcatagttacgaattgaagatgatggatggaaatatcgatctaggataggtatacatgttgatgcgggttttactgatgcatatacagagatgctttttgttcgcttggttgtgatgatgtggtgtggttgggcggtcgttcattcgttctagatcggagtagaatactgtttcaaactacctggtgtatttattaattttggaactgtatgtgtgtgtcatacatcttcatagttacgagtttaagatggatggaaatatcgatctaggataggtatacatgttgatgtgggttttactgatgcatatacatgatggcatatgcagcatctattcatatgctctaaccttgagtacctatctattataataaacaagtatgttttataattattttgatcttgatatacttggatgatggcatatgcagcagctatatgtggatttttttagccctgccttcatacgctatttatttgcttggtactgtttcttttgtcgatgctcaccctgttgtttggtgttacttctgcaggtcgactctagaggatccatggcaccgaagaagaagcgcaaggtgatgagcgacctcgtcctcggactcgacatcggaataggcagcgtcggagtcggtatcctgaacaaggtcaccggcgagatcatccataaaaacagcaggatcgtaagtttctgcttctacctttgatatatatataataattatcattaattagtagtaatataatatttcaaatatttttttcaaaataaaagaatgtagtatatagcaattgcttttctgtagtttataagtgtgtatattttaatttataacttttctaatatatgaccaaaacatggtgatgtgcagttcccagcagcacaagctgaaaataacctcgtcagaaggaccaaccgccaaggcaggaggcttgcacgcaggaagaagcacagaagggtgaggctcaaccgcctcttcgaagagagcggattaatcacagacttcaccaagatctcaattaatctcaacccctaccagctcagagtcaaggggctcacagacgagctcagcaacgaggagctcttcatcgccctcaaaaatatggtcaagcacaggggcatcagctacctcgacgacgcatcagacgacggaaacagcagcgtcggcgactacgcccagatcgtcaaggaaaatagtaagcagctcgagaccaagaccccaggacagatccagctcgaacgctaccagacatacggccagctcagaggcgacttcaccgtcgaaaaggacggcaagaagcaccgcctcattaatgtcttccccacaagcgcctacaggagcgaagcactgcggattctccagacccagcaggagttcaacccccagatcaccgacgagttcattaatcgctacctagagatcctcaccggcaagcgcaaatactatcacggaccagggaatgaaaagagccgcacagactacggacgctacagaaccagcggcgagaccctcgacaacatattcggcatcctcatcggcaagtgcaccttctaccccgacgagttcagagccgccaaggcatcctataccgcccaagagttcaacctactaaacgaccttaacaacctcacagtccccaccgaaaccaaaaagctcagcaaggagcagaagaatcaaatcattaattacgtcaagaatgaaaaggcgatgggcccagccaagctcttcaagtacatcgccaagctcctcagctgcgatgtcgccgacatcaagggataccgcatcgacaaaagcggcaaggccgaaatccacaccttcgaagcctaccgcaagatgaaaaccctcgagaccctcgacatcgagcaaatggaccgcgagaccctcgacaagctcgcctacgtcctcacattaaacacagagcgcgaaggcatccaggaggcactcgaacacgagttcgcagacggctccttcagccaaaagcaggtcgacgaactcgtccaattccgcaaggccaacagcagcatcttcggaaaaggctggcacaacttcagcgtcaagctcatgatggaactcatccccgagctctacgaaaccagcgaggagcaaatgaccatcctcacaaggctcggcaagcagaagaccaccagcagcagcaataaaacaaaatatatcgatgaaaaactcctcacagaggaaatctacaaccccgtcgtcgcaaagagcgtcaggcaggccataaaaatcgtcaacgccgccattaaagagtacggcgacttcgacaacatcgtcatcgagatggcaagggagaccaacgaggacgatgaaaagaaagccatccagaagatacagaaggccaacaaggatgaaaaagacgcagccatgctcaaggcagccaaccaatataatggcaaggccgagctcccacactcagtcttccacggccacaagcaactagccaccaagatacgcctgtggcaccaacaaggcgaacgctgcctctacacaggcaagaccatcagcatccacgacctcatcaataatagcaaccagttcgaggtcgaccacatcctcccactcagcatcaccttcgacgacagcctcgccaacaaggtcctcgtctacgcaaccgcaaaccaagagaagggacaaagaaccccgtaccaagccctcgacagcatggacgacgcctggagcttccgcgaattaaaagccttcgtcagggagagcaagaccctcagcaacaagaagaaagagtacctcctcaccgaggaggacatcagcaaattcgacgtccgcaagaagttcatcgaacgcaacctcgtcgacacaaggtacgccagcagagtcgtcctcaacgcactccaggagcacttcagagcccacaagatcgacaccaaggtcagcgtcgtcagaggacagttcaccagccaactcagacgccactgggggatcgagaagacacgcgacacctaccaccaccacgccgtcgacgccctcatcatcgcagcaagcagccaactcaacctctggaaaaagcagaagaacaccctcgtcagctacagcgaagaccagctcctcgacatagagaccggcgagctcatcagcgacgacgaatacaaggagagcgtcttcaaggccccctaccagcacttcgtcgatacattgaagagcaaagagttcgaggacagcatactcttcagctaccaggtcgacagcaaattcaaccgcaaaataagcgacgccaccatctacgccaccagacaggccaaggtcggaaaggacaaggccgatgaaacttacgtcctcggcaaaatcaaagacatatacacccaggacggatacgacgcattcatgaagatctacaagaaggacaagagcaagttcctcatgtacagacacgacccacagacattcgagaaggtcatcgagcccatcctcgaaaactaccccaacaagcaaataaatgaaaaaggaaaggaggtcccatgcaaccccttcctaaaatataaagaggagcacggctacatcaggaagtacagcaagaaaggaaacggccccgaaatcaagagcctcaaatactatgacagcaagctcggcaaccacatcgacatcacccccaaggacagcaacaataaagtcgtcctccaaagcgtcagcccctggagagccgacgtctacttcaacaagaccaccggaaaatacgagatcctcggcctaaagtacgccgacctccaattcgaaaaaggcaccggcacatataagatcagccaggaaaaatacaatgacatcaagaagaaggaaggagtcgacagcgacagcgaattcaagttcaccctctataaaaatgacctcctcctcgtcaaggacaccgagaccaaggagcagcagctcttccgcttcctcagcagaaccatgcccaagcagaagcattacgtcgaattaaaaccctacgacaagcagaagttcgaaggcggcgaagccttaattaaagtcctcggcaacgtcgccaacagcggacagtgcaaaaagggcctcggcaaatcaaatatcagcatatacaaggtccgcacagacgtcctcggaaaccaacacatcatcaagaacgaaggagacaagcccaagctcgacttcaagagaccacgggaccgccacgatggcgagctgggaggccgcaagcgggcaaggtaggtaccgttaacctagacttgtccatcttctggattggccaacttaattaatgtatgaaataaaaggatgcacacatagtgacatgctaatcactataatgtgggcatcaaagttgtgtgttatgtgtaattactagttatctgaataaaagagaaagagatcatccatatttcttatcctaaatgaatgtcacgtgtctttataattctttgatgaaccagatgcatttcattaaccaaatccatatacatataaatattaatcatatataattaatatcaattgggttagcaaaacaaatctagtctaggtgtgttttgc

SEQ ID NO: 73 - DNA, 4377 bp, synthetic construct
  misc_feature 1..4377: note = Sp Cas9 used in Example 4
  source 1..4377: mol_type = other DNA
atggcaccgaagaagaagcgcaaggtgatggacaagaagtacagcatcggcctcgacatcggcaccaactcggtgggctgggccgtcatcacggacgaatataaggtcccgtcgaagaagttcaaggtcctcggcaatacagaccgccacagcatcaagaaaaacttgatcggcgccctcctgttcgatagcggcgagaccgcggaggcgaccaggctcaagaggaccgccaggagacggtacactaggcgcaagaacaggatctgctacctgcaggagatcttcagcaacgagatggcgaaggtggacgactccttcttccaccgcctggaggaatcattcctggtggaggaggacaagaagcatgagcggcacccaatcttcggcaacatcgtcgacgaggtaagtttctgcttctacctttgatatatatataataattatcattaattagtagtaatataatatttcaaatatttttttcaaaataaaagaatgtagtatatagcaattgcttttctgtagtttataagtgtgtatattttaatttataacttttctaatatatgaccaaaacatggtgatgtgcaggtggcctaccacgagaagtacccgacaatctaccacctccggaagaaactggtggacagcacagacaaggcggacctccggctcatctaccttgccctcgcgcatatgatcaagttccgcggccacttcctcatcgagggcgacctgaacccggacaactccgacgtggacaagctgttcatccagctcgtgcagacgtacaatcaactgttcgaggagaaccccataaacgctagcggcgtggacgccaaggccatcctctcggccaggctctcgaaatcaagaaggctggagaaccttatcgcgcagttgccaggcgaaaagaagaacggcctcttcggcaaccttattgcgctcagcctcggcctgacgccgaacttcaaatcaaacttcgacctcgcggaggacgccaagctccagctctcaaaggacacctacgacgacgacctcgacaacctcctggcccagataggagaccagtacgcggacctcttcctcgccgccaagaacctctccgacgctatcctgctcagcgacatccttcgggtcaacaccgaaattaccaaggcaccgctgtccgccagcatgattaaacgctacgacgagcaccatcaggacctcacgctgctcaaggcactcgtccgccagcagctccccgagaagtacaaggagatcttcttcgaccaatcaaaaaacggctacgcgggatatatcgacggcggtgccagccaggaagagttctacaagttcatcaaaccaatcctggagaagatggacggcaccgaggagttgctggtcaagctcaacagggaggacctcctcaggaagcagaggaccttcgacaacggctccatcccgcatcagatccacctgggcgaactgcatgccatcctgcggcgccaggaggacttctacccgttcctgaaggataaccgggagaagatcgagaagatcttgacgttccgcatcccatactacgtgggcccgctggctcgcggcaactcccggttcgcctggatgacccggaagtcggaggagaccatcacaccctggaactttgaggaggtggtcgataagggcgctagcgctcagagcttcatcgagcgcatgaccaacttcgataaaaacctgcccaatgaaaaagtcctccccaagcactcgctgctctacgagtacttcaccgtgtacaacgagctcaccaaggtcaaatacgtcaccgagggcatgcggaagccggcgttcctgagcggcgagcagaagaaggcgatagtggacctcctcttcaagaccaacaggaaggtgaccgtgaagcaattaaaagaggactacttcaagaaaatagagtgcttcgactccgtggagatctcgggcgtggaggatcggttcaacgcctcactcggcacgtatcacgacctcctcaagatcattaaagacaaggacttcctcgacaacgaggagaacgaggacatcctcgaggacatcgtcctcaccctgaccctgttcgaggaccgcgaaatgatcgaggagaggctgaagacctacgcgcacctgttcgacgacaaggtcatgaaacagctcaagaggcgccgctacactggttggggaaggctgtcccgcaagctcattaatggcatcagggacaagcagagcggcaagaccatcctggacttcctcaagtccgacgggttcgccaaccgcaacttcatgcagctcattcacgacgactcgctcacgttcaaggaagacatccagaaggcacaggtgagcgggcagggtgactccctccacgaacacatcgccaacctggccggctcgccggccattaaaaagggcatcctgcagacggtcaaggtcgtcgacgagctcgtgaaggtgatgggccggcacaagcccgaaaatatcgtcatagagatggccagggagaaccagaccacccaaaaagggcagaagaactcgcgcgagcggatgaaacggatcgaggagggcattaaagagctcgggtcccagatcctgaaggagcaccccgtggaaaatacccagctccagaatgaaaagctctacctctactacctgcagaacggccgcgacatgtacgtggaccaggagctggacattaatcggctatcggactacgacgtcgaccacatcgtgccgcagtcgttcctcaaggacgatagcatcgacaacaaggtgctcacccggtcggataaaaatcggggcaagagcgacaacgtgcccagcgaggaggtcgtgaagaagatgaaaaactactggcgccagctcctcaacgcgaaactgatcacccagcgcaagttcgacaacctgacgaaggcggaacgcggtggcttgagcgaactcgataaggcgggcttcataaaaaggcagctggtcgagacgcgccagatcacgaagcatgtcgcccagatcctggacagccgcatgaatactaagtacgatgaaaacgacaagctgatccgggaggtgaaggtgatcacgctgaagtccaagctcgtgtcggacttccgcaaggacttccagttctacaaggtccgcgagatcaacaactaccaccacgcccacgacgcctacctgaatgcggtggtcgggaccgccctgatcaagaagtacccgaagctggagtcggagttcgtgtacggcgactacaaggtctacgacgtgcgcaaaatgatcgccaagtccgagcaggagatcggcaaggccacggcaaaatacttcttctactcgaacatcatgaacttcttcaagaccgagatcaccctcgcgaacggcgagatccgcaagcgcccgctcatcgaaaccaacggcgagacgggcgagatcgtctgggataagggccgggatttcgcgacggtccgcaaggtgctctccatgccgcaagtcaatatcgtgaaaaagacggaggtccagacgggcgggttcagcaaggagtccatcctcccgaagcgcaactccgacaagctcatcgcgaggaagaaggattgggacccgaaaaaatatggcggcttcgacagcccgaccgtcgcatacagcgtcctcgtcgtggcgaaggtggagaagggcaagtcaaagaagctcaagtccgtgaaggagctgctcgggatcacgattatggagcggtcctccttcgagaagaacccgatcgacttcctagaggccaagggatataaggaggtcaagaaggacctgattattaaactgccgaagtactcgctcttcgagctggaaaacggccgcaagaggatgctcgcctccgcaggcgagttgcagaagggcaacgagctcgccctcccgagcaaatacgtcaatttcctgtacctcgctagccactatgaaaagctcaagggcagcccggaggacaacgagcagaagcagctcttcgtggagcagcacaagcattacctggacgagatcatcgagcagatcagcgagttctcgaagcgggtgatcctcgccgacgcgaacctggacaaggtgctgtcggcatataacaagcaccgcgacaaaccaatacgcgagcaggccgaaaatatcatccacctcttcaccctcaccaacctcggcgctccggcagccttcaagtacttcgacaccacgattgaccggaagcggtacacgagcacgaaggaggtgctcgatgcgacgctgatccaccagagcatcacagggctctatgaaacacgcatcgacctgagccagctgggcggagacaagagaccacgggaccgccacgatggcgagctgggaggccgcaagcgggcaaggtag

SEQ ID NO: 74 - DNA, 18 bp, synthetic construct
  misc_feature 1..18: note = ZM-U6:08CR1
  source 1..18: mol_type = other DNA
gtacgtaacgtgcagtac

SEQ ID NO: 75 - DNA, 21 bp, synthetic construct
  misc_feature 1..21: note = ZM-U6:45CR1
  source 1..21: mol_type = other DNA
gcataatgaggatcgaggatg

SEQ ID NO: 76 - DNA, 18 bp, synthetic construct
  misc_feature 1..18: note = ZM-U6:10CR3
  source 1..18: mol_type = other DNA
gctcgtgttggagataca

SEQ ID NO: 77 - DNA, 14124 bp, synthetic construct
  misc_feature 1..14124: note = CTL1-TS8 DNA repair template
  source 1..14124: mol_type = other DNA
cagaatttacggtccagcacgggcatgccgcgcgggctgactttgctccactgactcgatcatgtgcggattccatcgcggcgtagcgtagccaaccgcaacgcaaaccgacttcatcttttttttttattatgaacaaaaggagatcgagagaaacgtgaacggtaaataatatatctgatcccatgcatgcacgctgcctgggtcgatctcgctctcgctccgcccagacgaacatgcatgctggtcaggctcaacgctcaggcgggcaagctgtgggaggacatgggatgggagaggaggacacatgcatgctggccagtcaggcactgtgctggcacatgaggtagggataggggggccctcggccagtgtccaggccgcatgcatgcatgccccccctgctgctcgaccgaacaacgttggatgcctggattgatgcaacagtttggacggacggaccatacgttatgtaccagtatctaacgccgacaccgtcgacgagtaagaggtcgtggccggctgcccacacgtctgtgtgaacctcaccatcgacaccaccgtccgcctgcggcctacggcctcgaactccaacatcacattcctctacaactgcatgaagaacattaccctaccctctgtcatggaactgagtgggttcccacaacaacaagaagatagatgtaggtcgtacgtgctgtgggatggcgggatcacgggtgctcaggcgtacgggtatgggtgcgaggacttggtggtagcgtcggagctggatgtacacaaaaagggagaaggcgatccacctccggaacggatcgctccatcgggttgccgcatgacgggatcgagctgaactacgacactcactctaagcagtgggacctagggatgaaaacggtcggtaaacactaaagcaattaccgttttcatattttttttatcgaaaacaaaatcgaaaacggtaactccggaaatggaaacgatatcggtatttcggaaacatcgcaaacgaaagttcggtgcgaaaaatacacaagtaacggtcgaaatctaaaatacgatcgataaacatatcaaacttcataatacaacaaagttgacaaaagatcacaaagaccacaagttcacaattcatgatataacaagtttaaaatataacaagttcacaaggatcacaaatttataatataaaaaaattacaaagatcacaagttcacaatataacaagttcacagtataacaagttcataaagatcacaagttcacaaactcaaggttcacaattcacaatatccactcgatttagctgacatggcatgcttactcatgaaatattttttcctcaaataaagagtttttcacagactcgtaggaaaaccctaaaatctagtatgtggaaaagacagactgtcggctctatcattatatattactaatacataacatgtggacagaaaatggtggattcgttcgagagaccaaatcgttaatctcaactgccttccaacaccatctatcaaaaaaaatcttaaggcgtccaaaaaatacaaaaaataagtaatccttatctagagacgtacaggcgatgcgaaaaaaatcacatgctgaataattccgaaaaaaattccggaaaattctgagacataaatccggtaatttccgacaaaaaccggtaaccgaaggaaacagtcggtaaaacaccacgccgattccgataccgactctaatagaaatttccgaaaaccgatttcgttttcgaaaaatactgttaccggtgaatacaatcgaaaaatttcgaaatcggtttccggaataccaaaaaattgtgaaactgttttcatcactagtgggaccgatgtgatggctccgacggatggtgtggctaccagcgtgatgagacgcccaccggcgggatgacattcgcatgtttttgcaaacgcagcccgatcacatgtgcacaatcgttagtggcgcgttttaaaaaagacgtaactacgaaaaaaaatagcgacatgtttttagccagtgtcacaaacgtcatcttcgagcacttttgatgtagtgtatacaatctactagtcaaattaaaaagaataacatacacgaaatggttcataacttttatatagttaaacaataataaatttataaaaatccctaaacaaacaacaaaacgttggacacctccccgctatttatggcggatggcccgcccaattgacgtaatttccacatcgaagtcgaagaaccggtcgctgtgaccagtcaccccaacctccgtcacttgtctctcacgcgcgcgcaacatcgccgagaaaaccagaacagacctccggattggtctctcccccgttcacacgagcacattgcgatggctcctctgctcctgctgctcctcttccccgtccagctccccctcgcagtagccgacgccgtctccggtccctgcaccagagccacatgcgccggccaggacgtccattacccgttctggctcaagtcctccgcgcccgactgcgtctatcccggtgtcggccttgtggcccttgtctgcgagggcaactcgacgctgatcctccccttcaagtcccacagatacgtagtgctcagcatcgactacaagacgcgtaccgtgctggtctccgacgccgacatcgtccacgagtacgacgcggccggctgcccgcgcgtccgcgtgaacctcaccatcgacaccgcctggctgcggcccacggcctccgactccaacatcaccttcctctacaactgcaagaagaacatcaccctgccctccgccgtggaactgagcgggtgccagcagcagcagcaacaagacggcagcaggtcgtattcgtacgtgctgccggacggcggggtcacgggcgctgaggcgcaccagtacgggtgcgaggacttggtggtggcgccggtgctggacgtccacaggagggcgatcttgagggcgcctggcggcccgactctggagaacgggtcgctccgtcggttgctgcagggcgggttcgagctgaactacgacactcactccgagcagtgcgaccgatgcgaggcctccggcgggtggtgtggctaccagcgcgacgagacgcccgccggctggatgacgttcgcctgcttctgcgacggcgggccgacgaccacggcccgatgcggtgccggtatgtcttttttttttcttcgaacaaggtgtggcatgtgttctaccgtttcaactagtaaatgattacattgagctaggcagctagccacacattttcttgaatgattttctttgatgaacctgctgtttgcttttatgacgtgaacaacggggcctgcaagctgccacatacctagggagactagttcgtgaccttctttacacgtcttctctactcgccactgggagttgacgccgctcggtcgtcccactttgtgacgttcaaccagagtctagagatgtaattctctgcgaatacaggactagttggagctaacaacgcagcttgacgagggtgaacccagctccacctcgtctaccacgtcttctcctcgccatggctgctcacctaccacgcctccccgtcctcctcctcgtcctcctcgctgctcatgtcgtctccacctccgcccatgccgagcctcctcttccgagcccttacagcacctccgcccatggcgagcctcctcttccgagcacttacaacgtctccatgtgctcggaatcgttctggtgcggcggcgtcgaaatccgctacccgttctatcttgccaacgcaaccgccgactacagcgggagctactactcctgcggctacaccgacttgagcgtttcctgcaaactcgaggtcgaggggccgacgacgacatggacccctaccatccgtctcggcggcgacaactacaccgtcaagaacatcttgtacgactatcataccatctcactggcggacagcgatgtgctcggaggcggcgagtgccccgtcgtccaccacaacgtcagcttcgacgagacgtggctgcacaaccccagcgccttcgacaacctcaccttcttcttcggatgccactgggggccacgcgatacactgcctgaatttgccggcaacaacatcagctgcgccgggttcagtactccagctatcagcggtggaggctccttcgtgttcaagcctgaagatcttgacgaacatgcggagcaggagttggcttcacactgcgacgaggttttctccgtgccagtgagaagcgaggctctgcagcaggcgatcgtcagcaacctcagcctcggggacgggtacggcgagctgcttaggcaggggatcgagttggaatggaaacggacatcggaggatcagtgtggccagtgcgaggaatcgggctccggcggacggtgcgcctacagccagaagagagaattccttggctgcttgtgcagcggagggaaggcgggcaacccgttctgcaaaccatcaagtaaagtcctgaaccgagcctcccttatttttttttcattttttgcaatccaccagagagcacgcatcggttgcgtcagtatcttgcaacctcgtagctagccccgcagtgtcccctgtgtgcgagtaccgcgctgctccagcttgcctcctgctaacgcctaacggtgaatgcttcatgcttgacatgatctagctagtctacactttgcttggggtttgcctgggagctggaaattctggctcctgtttgcatcactcgacaaggacgctttcagacttgcgactctcgttctgcttttgcaccaaatccgtgtttttttcatttcgtgatcgagattaatctagcttagagatgacaatgggtatccgaaactcgaaacttgatggatttttactccattagggtataggtttgaatcaattttcatatttatggatttgttaataggcataaatatatatccaacaggtttatagatacgagtttgtttctacagtactcaaatccgtgaacacatgaggtttttaaacccgaccaaacctagtgcatattgtcattttattttataaacgaacaacaaaattgttatctctatttacttcctattttttatcgattggtgaatgtataagtagttggtgagaatgtttcttgcttgctattatagttttactagcgttatatatgttgtgggtggataacttagtgcaatgtcacttgattatacaacttattatttgtattcattctctctactaataatttttataccaaatcatgaactcggtgtttattatataaattttggaccataatctcattaatcatcacgatagttattgattatgagaaaaaacaagcatattggagataaaaccctcggctaacccgttaacccgatgggtacgggtttgaacaaaatttcaaacctattatgaatataagttttttaacaagtatagatatatttcacggatagagtttaagatgacaaaatccaacggatttgtatccattgccatctctatccggcggcccttacccggcggcccttaccgtgctccacgagcagaggtcgtatcgtccctcttcccgtgtcgcctgcttcgcgttgccgaacggagacgtttggtagcgttggccggctctagcagtcgggtcaactctttttgttgttgttttcgatgttgttggatttttgttccgtataagccatgttttagtaatttatttagtccagccgaatccgaagacgtgtttgctgggttggagactttggagttgctagtcatgatatgctttctactcggtttgatttcaacccagttaggctatatttaatactctagtatttatttcaatataaatggtttgaaacggattaaggtataaattagtttaatttatatatttaattcctctcaatccatatgtattgggctgaatactgaggtagtgtttggttgaagagccatatagaacggagccgttctgttccagttttgttgttgtttggttataaagtaactagaacggaatgacttcaattaaggaatattcttctcagatccagaaccattccgctctaaaaaatcaaccggacggagccgctccgtttccatcctgctcttacagtcacgctccgttccgttcactctgcaaccaaacaaaaaacagagccgctccgttccaaattaccaaacacagaacagagcggcttcattcctagaattaggaatggaacgactctgttctacttgactcctcaaccaaacactacctaagtatccaaacaagcccttatttaagatgcatttcctttacagttacacatgaccactattgtgtgggggcaggctgaacaagcccttatttaagatgcatttcctttagagttacacgtggccactattgtgggggggggggggggggggcaggccgatcctactcgtcagtgctcattcgagagcaaagataccgaaggagattagagagactaaaaactttttactatttaaaattagataataagacgatttaatcccgttccatatctttgctctaaacaaaccctcaatgatcatatatctcggaagatccggccggctgttctttatttatcaagtgatgactgctgaccgcttatagaatatatattttaaagcaaaatttcttctacagcagtaaaaggactagacgaaacaatgatgcatttctctaacaaaagaaagtagaattatcaagcggagagccaagaccaaaagccttacttctatgggcgtcaacaaatgataccgcgacggaaccatcccagcaggtctatactgtctgtcacgacccagcgagtaatcgtgtggctacgctattagacttaggattggatgaaatgctcggtttattaatgagccagctcgtgagttaagagtgtttggtttgatgaatgaagtaattcatcttcttttcactccccacttttttatttggtttgtgtaatagaatgagttgatccatcaccaccacattcatcataagctaataattagtatatacatgagtagtgagttgattccaccaaaattgatgaaatgaacttatgatgcatcatctcatgaagcatagagtgactccacaaaccaaacacaccataaatgatctattacataacgaaattatatgcatatcatttatcagggcgacgacagggggcatagggaggcaatatccccctaatgctccccaaattctatagggattgttagtttcttttagctaattctcatgtaaacaatataaaaaatgcttctaacagtccctcctaattataatttggtccaccctaatcttagatcctggcttcgtccgtgccatttacgtaacaattggtaaatatgttatacatgtgtggtatctatggcctatgaattgaactaatgattgatgaattgtgcttatgtgttaaattggtctatgcgaatataactatgggttaaacggatgaacatgtgtgttcattgttaattcatgagtgatgaattatgtataatttggtgttatattgatgtgttttgtgaaactatgtgtataattattattttctataattaaatttgtttgaaattaactagaaattgattattatatatatatatatatatatattgtttttctgctctagtctgcaagctaaacgagcaagctcaagctcgtaaacgatccgaaccgagctgactttgtggctcattaacttaacaagccgagttgggccaacttgttagcttaacgagtcagctcgaatacggacaagttgagccgagttggcatgatatccagccctaattaggcttgtaccagtgcaacatatccctctcgcctttgtcacgtccagacatgtcaatgggccccgattcccgcaaggaatttctctattaagggatgaggatgggaaagtttctccccccacagaaaaattctctcccgacggataagcggggacaacactccccatccccattccccgtggggacctattagacttacatatggtgatgttttcatgtaaaagttaatgataaaaataaacaattaccttgttgtcggcgtttcgaccccggagggtccctggaccgacgagtaaattgtcgctgcgtgtcccagcccagatgggtcgacgcgagacggaacacaagggggaaacaataaggggaatcgcggcctcgtgttgtcctgcgcccagggcggatgcgcttgcagtaaggggttacaagcgttcgcgagggagagagagagagagcctgtgcgccagcccgtcctcccgcgcggccaccttctcgtacgagggccctggacctttcttttatagatgtaaggagagggtccaggtgtacaacagggagcgtagcaatgtgctaacgtgtctagcagagggaagccagaatcctatgtacaggccgacgtgactgtcgaagaggttttggcgccctgttcatgtgatgtcgtggccgtcggaggagcgcttgagccctgtaggagcacagctgtcggagctgtcgggtccttgctgacgtctcattgcttccatagggagctgagaaccgccgtcgtcatggagcacgcggggtgccatcattacttgttttaccgggacgagccagatgggacgctggtcttgttcccagtagcctgaggtagctagaggtagggtaatgatgtgccctcctgcgacgtggtcggtccgagcccaaggtcgggcgaggcggaggctcctccgaggtcgaggctgagtccgagacctggggtcgggcgaggcggagaccgtcgtccgaggtcgaggttgagtccgagccctggggtcgggcgaggcagagtccatcgtccgaggtcgaggttgagtccgagccctggggtcgggcgaggcggagacagtcgtccgaggtcaaggttgagtccgagccctggggtcgggcgaggcggagttcgtcttccgaggtcgaggtggagtctgagccctagggtcaggcgaggcggagaccgtcgtccgaggtcgaggttgagtccgagctctggggtcgggcgaggtggagcttcctatggcgcctgaggccggacttggcggctgtcagcctcaacctgacgggtggcacagcagtcgaagcagcgcaggcggcgctgtttttctatcaggtcagccagtggaggggcgaagtgactgcggtcacttcggctctgtcgactgaagagcgtgcgtcaggataaggtgtcaggcgatccttgcattgaatgctcctgcgatccggtcggctggcgaggcgatcttggctaaggttgcttctccgcgaagcctgcctgagctgggcctcgggcgagtcggaggtgcgcccgttgcttgaggaggccctcgggcgaggcgtgaacctgcctgggcctgctgtttctgcccgaggctgggctcgggtgaggcgagatcgtgtcccttgagcggacagagctttgtcctgtgttgcgcccatcaggcctttgcagctttgtgctgatggtgtttaccagccgagtttaagagtcttgggggtacccctaattatggtccccgacacttgtcaagagatcactttttgtacaaatatattcattctgatgtacacatatttttttcttacatctaacaatgtgtataagtgagaatgttttatattaataacaaatgaagtatgtcctaattagacttctcacattgagcagcaacaaaacattttatgaattagtaaccattttacttactaaaataattactattgtatcttaatcattttgtgcaaaataaagaatgaaccaaattttgggtcaggtgtgggtcactcgcaggttgaaataaaaacccgcacccacactcgtgaaactttgggtcagatgcgggttacacccgcggattaaaatctctacccatacccacactcatcagatcgagtacccaaagattttaagtttgcgggttaaattgtcatccctcgacaccaacgtgttggaggatttggaagtttcgcgatgcgtacttaccaagtgtttggttctatgataaaagtttagcctgtgtcgcattagatgattgaatgtctattatgagtattaaatattgtctaattattaatcaaattacacaagtgaaggctaaacaacgagacaaatttattaagcctaattaatctatgattagcaaatgtttacagtagcaccatctagtagcaccatctgagcgaatcatgaactaattaggtttaataggttcgtcttaacgtttaattcttatctatgtaattagttttataagtaaattatatttaatacttctaattagcctccaaacattcgatataacatagactaaaatttagtcagtggtgctgctgctggctcttttccttcatccgacgtaatgttttcctcccaatttattgtgttgttttgtttgtgctttaaaactgacttgctctctgcttgctgtatcaaagtcgtgatgtgtgcttagcttattcccttccttgctagctgcccttagcatctatatagggatatttggttatagggactaaagtttagtttagtccgtgtccaattataaaactaattacataactgaatactaaaagacgagaaaattttattaaacttaattaatttatgattagcaaatgtttattgtaacatcacataagtaaattatagactaattttgtttaataggttcatcttatcatttagtcttcatctatgtaattagttttgtaattagactatatttactatttctaactagtatctaaacattaaatgtgacatggattaaaatttagttagagcaactccagtagttttctaaaagacttcctaaatcaataatttaggtagttaacatgaaaactattctccaacagttctctaaataaactttctaaatttaacaacttgtcatctaacctcattttctctctacatttggcaaccatttaataactccctaatcaaaaatgttgactgcattatatagtttttgtgacttattttttatgtggataaatacaaaataaaattacaacctatatttagagaactattggagaacccacttatttttatttcaaaagtcatttagcaacttcttaaatctgtaatttagaaagctaaaatttacataactattagagttgctcttagtgacgttaggcttttagagttgagttggtcgtagcttggtttagttacgtgtttgttctcttgcgtttatttaggacctctctataatgttttatcaccttcttaatacaaattaaaatacgcagctctcttgcgtattggaggcgtgtgttcctatattttttaggctcaattatgaatgaaattattctcagcgagcatataaccgttttcgaggtaaaatgaactaaaagcatatgggcctgcctgttcgcataagtacaccctccgtctaaaaaagaataaaaatatcatttcttgatgagtcaaaaaagttcaaatttaagaaaatatatgttacgacaccaatatttataatgtgtaataagtactgctgattaattttaaaataaaattttcataataaacctatttgaagatacaagtattggtactatttctaataaatctaatcaaactggtgttatatcttttgtaacaaatttgtgctttgtgtttctggttgacgtgaatcagcttaatcttgctgaaatctaacattgtcttttgttcgttggcatacaggatcaaaaaggaaagaagcatctattgttggtaagagcctatagtcaatacccatgttcatttcgtctaaaagagcagaagaaaagcatatgatgaattattgccatgtcatgtttaaaatacagaattctcaaaaacaaaaacaaaaaaaacttggaatccactaaccagtaaccactgatagcattgtagaaaatttcatcctccctttgggcaatacactgatgagtttacatgctgactagtggtgcatttgttctttgccaattgaatttttagaatgctttgcagctgaattcacttgtgatttttttttgtgatgcaggtgctgttgccgttgcattcctgtgtctagtcattctcacatgcttcttggcttgtagacatggttcgctgcccttcaaatcggagaacaaaccagggacaaggattgagtccttcctacagaagaacgagagtatacatccgaaaagatacacctacacggacgtgaaaagaatgacaaaatccttcgctgtgaagctaggccaaggtgggtttggtgctgtatacaaaggcagcctccacgatggccgacaggtagcagtcaagatgctcaaggacacccaaggtgacggcgaggaattcatgaacgaggtggctagcatcagcaggacttctcatgtcaacgtcgtgacacttctagggttttgcttgcaagggtcgaaaagagcactgatctacgagtacatgcccaatggttcgctcgaaaggtatgccttcaccggtgacatgaacagtgagaatttgctaacctgggaaaggctatttgacatagcaattggcacggccagagggctcgaatacctacaccggggatgcaacactcggatcgtgcattttgacatcaagccacacaacatcctgttagaccaggatttctgtcctaagatctctgactttggactggccaagctatgtctgaacaaagagagcgctatctccattgttggcgcaagagggacgatagggtatatcgccccggaggtctactcaaagcaatttggaacaatcagcagcaagtctgatgtctatagctatgggatgatggtccttgagatggttggagcaagggaaaggaatacaagcgcaagcgcagatagtgaccatagcagccaatatttccctcagtggatttatgaacatttggacgactattgtgttggtgcttccgagattaatggtgagaccacagagctcgtgaggaagatgatagttgtaggtctgtggtgcatacaagtgattccgactgatcgaccaacaatgacgagagtcgtcgagatgttggaagggagcacgagtaatctagagttgccacccagagttctcttgagctgacaaagcgtagatatttttcctatcaaatgttgcttccaggtcacacaaatgcaaaatatttgtggagacgagtgcctatttacctcatacactgtatctgtatgacaaaagtcccacgactcactggacgcggaaatgtcgcttgactacgccaattttctaaaaagattggcagcaattaatggaggcttatagcggtaactttggttcgcattaatcctaggactagggttgaatatcgatctaactcgacgcggcttggtcaagctcaagctagctccactcatctcattaaagaatccagctagaaaatcaacccaagtcgtttacgaaacgagtttgagctgactcgtttagatcgtaaatcacaacaaaaacaatatgcacatatatacaataatataatcaatactagttaattctagactagtttaacactagaaaagagtaatgatactcataatttcacatacaatgtcaatccaacaccaatttaacacacttcatcacttattagttcatccaaccaagtgtaggctttgatttactaacaaatggttgctcgttcgagctagcgagcttgcttgttaacaaactgagttgagatgctagcttaacttgtgacaaaattaaaacgagccgagtcgagtcaagttgagctcacgatgagtcgagcaagctcacaatccacgagtatttttttagtcctatctaagactaaagtttaatcctaaaactaaattttaatctctatttgtttggttctataaactaaacaggttcagaaaacataaaatacattatagaaaacctgaaatacccttctatacttaaggcatcactaagagagagcaataaataaagggtagagagaggaataaatctgctttattcccttttagctaccctttgagagagtaaacactaaaatgaaaggatccttgaggattttgatgttttggatgacaactaacacaattaaaggtctaattaggatgttaa

SEQ ID NO: 78 - DNA, 14471 bp, synthetic construct
  misc_feature 1..14471: note = CTL1-TS45 DNA repair template
  source 1..14471: mol_type = other DNA
cggatagatggcgtctagcatatcgataggacatgacaagtggtacgatccccgtcacatgtccatggaggcatctgatatggacacggcgtgtatctatcgcggctggaacagaaccagcgctcgcgcggcggtcggcgggagggacagaccttggctccgtgcgttcaggttgtgcttgtgccgcgcgccacgcacggtctccgccgcctgcagctgaaattttagatttacatcctatccctttattttttttatttgtcacaattcagttcaaaaatgaagaacggaggtagtgcatcctttgtgagactaatgaaaatcacatctggatcctgaaatcggcgtcgtaacctacaaggccacggactggattagatagtggtccatggtgcataatgaggatcgaggtctaacgccgacaccgtcgacgagtaagaggtcgtggccggctgcccacacgtctgtgtgaacctcaccatcgacaccaccgtccgcctgcggcctacggcctcgaactccaacatcacattcctctacaactgcatgaagaacattaccctaccctctgtcatggaactgagtgggttcccacaacaacaagaagatagatgtaggtcgtacgtgctgtgggatggcgggatcacgggtgctcaggcgtacgggtatgggtgcgaggacttggtggtagcgtcggagctggatgtacacaaaaagggagaaggcgatccacctccggaacggatcgctccatcgggttgccgcatgacgggatcgagctgaactacgacactcactctaagcagtgggacctagggatgaaaacggtcggtaaacactaaagcaattaccgttttcatattttttttatcgaaaacaaaatcgaaaacggtaactccggaaatggaaacgatatcggtatttcggaaacatcgcaaacgaaagttcggtgcgaaaaatacacaagtaacggtcgaaatctaaaatacgatcgataaacatatcaaacttcataatacaacaaagttgacaaaagatcacaaagaccacaagttcacaattcatgatataacaagtttaaaatataacaagttcacaaggatcacaaatttataatataaaaaaattacaaagatcacaagttcacaatataacaagttcacagtataacaagttcataaagatcacaagttcacaaactcaaggttcacaattcacaatatccactcgatttagctgacatggcatgcttactcatgaaatattttttcctcaaataaagagtttttcacagactcgtaggaaaaccctaaaatctagtatgtggaaaagacagactgtcggctctatcattatatattactaatacataacatgtggacagaaaatggtggattcgttcgagagaccaaatcgttaatctcaactgccttccaacaccatctatcaaaaaaaatcttaaggcgtccaaaaaatacaaaaaataagtaatccttatctagagacgtacaggcgatgcgaaaaaaatcacatgctgaataattccgaaaaaaattccggaaaattctgagacataaatccggtaatttccgacaaaaaccggtaaccgaaggaaacagtcggtaaaacaccacgccgattccgataccgactctaatagaaatttccgaaaaccgatttcgttttcgaaaaatactgttaccggtgaatacaatcgaaaaatttcgaaatcggtttccggaataccaaaaaattgtgaaactgttttcatcactagtgggaccgatgtgatggctccgacggatggtgtggctaccagcgtgatgagacgcccaccggcgggatgacattcgcatgtttttgcaaacgcagcccgatcacatgtgcacaatcgttagtggcgcgttttaaaaaagacgtaactacgaaaaaaaatagcgacatgtttttagccagtgtcacaaacgtcatcttcgagcacttttgatgtagtgtatacaatctactagtcaaattaaaaagaataacatacacgaaatggttcataacttttatatagttaaacaataataaatttataaaaatccctaaacaaacaacaaaacgttggacacctccccgctatttatggcggatggcccgcccaattgacgtaatttccacatcgaagtcgaagaaccggtcgctgtgaccagtcaccccaacctccgtcacttgtctctcacgcgcgcgcaacatcgccgagaaaaccagaacagacctccggattggtctctcccccgttcacacgagcacattgcgatggctcctctgctcctgctgctcctcttccccgtccagctccccctcgcagtagccgacgccgtctccggtccctgcaccagagccacatgcgccggccaggacgtccattacccgttctggctcaagtcctccgcgcccgactgcgtctatcccggtgtcggccttgtggcccttgtctgcgagggcaactcgacgctgatcctccccttcaagtcccacagatacgtagtgctcagcatcgactacaagacgcgtaccgtgctggtctccgacgccgacatcgtccacgagtacgacgcggccggctgcccgcgcgtccgcgtgaacctcaccatcgacaccgcctggctgcggcccacggcctccgactccaacatcaccttcctctacaactgcaagaagaacatcaccctgccctccgccgtggaactgagcgggtgccagcagcagcagcaacaagacggcagcaggtcgtattcgtacgtgctgccggacggcggggtcacgggcgctgaggcgcaccagtacgggtgcgaggacttggtggtggcgccggtgctggacgtccacaggagggcgatcttgagggcgcctggcggcccgactctggagaacgggtcgctccgtcggttgctgcagggcgggttcgagctgaactacgacactcactccgagcagtgcgaccgatgcgaggcctccggcgggtggtgtggctaccagcgcgacgagacgcccgccggctggatgacgttcgcctgcttctgcgacggcgggccgacgaccacggcccgatgcggtgccggtatgtcttttttttttcttcgaacaaggtgtggcatgtgttctaccgtttcaactagtaaatgattacattgagctaggcagctagccacacattttcttgaatgattttctttgatgaacctgctgtttgcttttatgacgtgaacaacggggcctgcaagctgccacatacctagggagactagttcgtgaccttctttacacgtcttctctactcgccactgggagttgacgccgctcggtcgtcccactttgtgacgttcaaccagagtctagagatgtaattctctgcgaatacaggactagttggagctaacaacgcagcttgacgagggtgaacccagctccacctcgtctaccacgtcttctcctcgccatggctgctcacctaccacgcctccccgtcctcctcctcgtcctcctcgctgctcatgtcgtctccacctccgcccatgccgagcctcctcttccgagcccttacagcacctccgcccatggcgagcctcctcttccgagcacttacaacgtctccatgtgctcggaatcgttctggtgcggcggcgtcgaaatccgctacccgttctatcttgccaacgcaaccgccgactacagcgggagctactactcctgcggctacaccgacttgagcgtttcctgcaaactcgaggtcgaggggccgacgacgacatggacccctaccatccgtctcggcggcgacaactacaccgtcaagaacatcttgtacgactatcataccatctcactggcggacagcgatgtgctcggaggcggcgagtgccccgtcgtccaccacaacgtcagcttcgacgagacgtggctgcacaaccccagcgccttcgacaacctcaccttcttcttcggatgccactgggggccacgcgatacactgcctgaatttgccggcaacaacatcagctgcgccgggttcagtactccagctatcagcggtggaggctccttcgtgttcaagcctgaagatcttgacgaacatgcggagcaggagttggcttcacactgcgacgaggttttctccgtgccagtgagaagcgaggctctgcagcaggcgatcgtcagcaacctcagcctcggggacgggtacggcgagctgcttaggcaggggatcgagttggaatggaaacggacatcggaggatcagtgtggccagtgcgaggaatcgggctccggcggacggtgcgcctacagccagaagagagaattccttggctgcttgtgcagcggagggaaggcgggcaacccgttctgcaaaccatcaagtaaagtcctgaaccgagcctcccttatttttttttcattttttgcaatccaccagagagcacgcatcggttgcgtcagtatcttgcaacctcgtagctagccccgcagtgtcccctgtgtgcgagtaccgcgctgctccagcttgcctcctgctaacgcctaacggtgaatgcttcatgcttgacatgatctagctagtctacactttgcttggggtttgcctgggagctggaaattctggctcctgtttgcatcactcgacaaggacgctttcagacttgcgactctcgttctgcttttgcaccaaatccgtgtttttttcatttcgtgatcgagattaatctagcttagagatgacaatgggtatccgaaactcgaaacttgatggatttttactccattagggtataggtttgaatcaattttcatatttatggatttgttaataggcataaatatatatccaacaggtttatagatacgagtttgtttctacagtactcaaatccgtgaacacatgaggtttttaaacccgaccaaacctagtgcatattgtcattttattttataaacgaacaacaaaattgttatctctatttacttcctattttttatcgattggtgaatgtataagtagttggtgagaatgtttcttgcttgctattatagttttactagcgttatatatgttgtgggtggataacttagtgcaatgtcacttgattatacaacttattatttgtattcattctctctactaataatttttataccaaatcatgaactcggtgtttattatataaattttggaccataatctcattaatcatcacgatagttattgattatgagaaaaaacaagcatattggagataaaaccctcggctaacccgttaacccgatgggtacgggtttgaacaaaatttcaaacctattatgaatataagttttttaacaagtatagatatatttcacggatagagtttaagatgacaaaatccaacggatttgtatccattgccatctctatccggcggcccttacccggcggcccttaccgtgctccacgagcagaggtcgtatcgtccctcttcccgtgtcgcctgcttcgcgttgccgaacggagacgtttggtagcgttggccggctctagcagtcgggtcaactctttttgttgttgttttcgatgttgttggatttttgttccgtataagccatgttttagtaatttatttagtccagccgaatccgaagacgtgtttgctgggttggagactttggagttgctagtcatgatatgctttctactcggtttgatttcaacccagttaggctatatttaatactctagtatttatttcaatataaatggtttgaaacggattaaggtataaattagtttaatttatatatttaattcctctcaatccatatgtattgggctgaatactgaggtagtgtttggttgaagagccatatagaacggagccgttctgttccagttttgttgttgtttggttataaagtaactagaacggaatgacttcaattaaggaatattcttctcagatccagaaccattccgctctaaaaaatcaaccggacggagccgctccgtttccatcctgctcttacagtcacgctccgttccgttcactctgcaaccaaacaaaaaacagagccgctccgttccaaattaccaaacacagaacagagcggcttcattcctagaattaggaatggaacgactctgttctacttgactcctcaaccaaacactacctaagtatccaaacaagcccttatttaagatgcatttcctttacagttacacatgaccactattgtgtgggggcaggctgaacaagcccttatttaagatgcatttcctttagagttacacgtggccactattgtgggggggggggggggggggcaggccgatcctactcgtcagtgctcattcgagagcaaagataccgaaggagattagagagactaaaaactttttactatttaaaattagataataagacgatttaatcccgttccatatctttgctctaaacaaaccctcaatgatcatatatctcggaagatccggccggctgttctttatttatcaagtgatgactgctgaccgcttatagaatatatattttaaagcaaaatttcttctacagcagtaaaaggactagacgaaacaatgatgcatttctctaacaaaagaaagtagaattatcaagcggagagccaagaccaaaagccttacttctatgggcgtcaacaaatgataccgcgacggaaccatcccagcaggtctatactgtctgtcacgacccagcgagtaatcgtgtggctacgctattagacttaggattggatgaaatgctcggtttattaatgagccagctcgtgagttaagagtgtttggtttgatgaatgaagtaattcatcttcttttcactccccacttttttatttggtttgtgtaatagaatgagttgatccatcaccaccacattcatcataagctaataattagtatatacatgagtagtgagttgattccaccaaaattgatgaaatgaacttatgatgcatcatctcatgaagcatagagtgactccacaaaccaaacacaccataaatgatctattacataacgaaattatatgcatatcatttatcagggcgacgacagggggcatagggaggcaatatccccctaatgctccccaaattctatagggattgttagtttcttttagctaattctcatgtaaacaatataaaaaatgcttctaacagtccctcctaattataatttggtccaccctaatcttagatcctggcttcgtccgtgccatttacgtaacaattggtaaatatgttatacatgtgtggtatctatggcctatgaattgaactaatgattgatgaattgtgcttatgtgttaaattggtctatgcgaatataactatgggttaaacggatgaacatgtgtgttcattgttaattcatgagtgatgaattatgtataatttggtgttatattgatgtgttttgtgaaactatgtgtataattattattttctataattaaatttgtttgaaattaactagaaattgattattatatatatatatatatatatattgtttttctgctctagtctgcaagctaaacgagcaagctcaagctcgtaaacgatccgaaccgagctgactttgtggctcattaacttaacaagccgagttgggccaacttgttagcttaacgagtcagctcgaatacggacaagttgagccgagttggcatgatatccagccctaattaggcttgtaccagtgcaacatatccctctcgcctttgtcacgtccagacatgtcaatgggccccgattcccgcaaggaatttctctattaagggatgaggatgggaaagtttctccccccacagaaaaattctctcccgacggataagcggggacaacactccccatccccattccccgtggggacctattagacttacatatggtgatgttttcatgtaaaagttaatgataaaaataaacaattaccttgttgtcggcgtttcgaccccggagggtccctggaccgacgagtaaattgtcgctgcgtgtcccagcccagatgggtcgacgcgagacggaacacaagggggaaacaataaggggaatcgcggcctcgtgttgtcctgcgcccagggcggatgcgcttgcagtaaggggttacaagcgttcgcgagggagagagagagagagcctgtgcgccagcccgtcctcccgcgcggccaccttctcgtacgagggccctggacctttcttttatagatgtaaggagagggtccaggtgtacaacagggagcgtagcaatgtgctaacgtgtctagcagagggaagccagaatcctatgtacaggccgacgtgactgtcgaagaggttttggcgccctgttcatgtgatgtcgtggccgtcggaggagcgcttgagccctgtaggagcacagctgtcggagctgtcgggtccttgctgacgtctcattgcttccatagggagctgagaaccgccgtcgtcatggagcacgcggggtgccatcattacttgttttaccgggacgagccagatgggacgctggtcttgttcccagtagcctgaggtagctagaggtagggtaatgatgtgccctcctgcgacgtggtcggtccgagcccaaggtcgggcgaggcggaggctcctccgaggtcgaggctgagtccgagacctggggtcgggcgaggcggagaccgtcgtccgaggtcgaggttgagtccgagccctggggtcgggcgaggcagagtccatcgtccgaggtcgaggttgagtccgagccctggggtcgggcgaggcggagacagtcgtccgaggtcaaggttgagtccgagccctggggtcgggcgaggcggagttcgtcttccgaggtcgaggtggagtctgagccctagggtcaggcgaggcggagaccgtcgtccgaggtcgaggttgagtccgagctctggggtcgggcgaggtggagcttcctatggcgcctgaggccggacttggcggctgtcagcctcaacctgacgggtggcacagcagtcgaagcagcgcaggcggcgctgtttttctatcaggtcagccagtggaggggcgaagtgactgcggtcacttcggctctgtcgactgaagagcgtgcgtcaggataaggtgtcaggcgatccttgcattgaatgctcctgcgatccggtcggctggcgaggcgatcttggctaaggttgcttctccgcgaagcctgcctgagctgggcctcgggcgagtcggaggtgcgcccgttgcttgaggaggccctcgggcgaggcgtgaacctgcctgggcctgctgtttctgcccgaggctgggctcgggtgaggcgagatcgtgtcccttgagcggacagagctttgtcctgtgttgcgcccatcaggcctttgcagctttgtgctgatggtgtttaccagccgagtttaagagtcttgggggtacccctaattatggtccccgacacttgtcaagagatcactttttgtacaaatatattcattctgatgtacacatatttttttcttacatctaacaatgtgtataagtgagaatgttttatattaataacaaatgaagtatgtcctaattagacttctcacattgagcagcaacaaaacattttatgaattagtaaccattttacttactaaaataattactattgtatcttaatcattttgtgcaaaataaagaatgaaccaaattttgggtcaggtgtgggtcactcgcaggttgaaataaaaacccgcacccacactcgtgaaactttgggtcagatgcgggttacacccgcggattaaaatctctacccatacccacactcatcagatcgagtacccaaagattttaagtttgcgggttaaattgtcatccctcgacaccaacgtgttggaggatttggaagtttcgcgatgcgtacttaccaagtgtttggttctatgataaaagtttagcctgtgtcgcattagatgattgaatgtctattatgagtattaaatattgtctaattattaatcaaattacacaagtgaaggctaaacaacgagacaaatttattaagcctaattaatctatgattagcaaatgtttacagtagcaccatctagtagcaccatctgagcgaatcatgaactaattaggtttaataggttcgtcttaacgtttaattcttatctatgtaattagttttataagtaaattatatttaatacttctaattagcctccaaacattcgatataacatagactaaaatttagtcagtggtgctgctgctggctcttttccttcatccgacgtaatgttttcctcccaatttattgtgttgttttgtttgtgctttaaaactgacttgctctctgcttgctgtatcaaagtcgtgatgtgtgcttagcttattcccttccttgctagctgcccttagcatctatatagggatatttggttatagggactaaagtttagtttagtccgtgtccaattataaaactaattacataactgaatactaaaagacgagaaaattttattaaacttaattaatttatgattagcaaatgtttattgtaacatcacataagtaaattatagactaattttgtttaataggttcatcttatcatttagtcttcatctatgtaattagttttgtaattagactatatttactatttctaactagtatctaaacattaaatgtgacatggattaaaatttagttagagcaactccagtagttttctaaaagacttcctaaatcaataatttaggtagttaacatgaaaactattctccaacagttctctaaataaactttctaaatttaacaacttgtcatctaacctcattttctctctacatttggcaaccatttaataactccctaatcaaaaatgttgactgcattatatagtttttgtgacttattttttatgtggataaatacaaaataaaattacaacctatatttagagaactattggagaacccacttatttttatttcaaaagtcatttagcaacttcttaaatctgtaatttagaaagctaaaatttacataactattagagttgctcttagtgacgttaggcttttagagttgagttggtcgtagcttggtttagttacgtgtttgttctcttgcgtttatttaggacctctctataatgttttatcaccttcttaatacaaattaaaatacgcagctctcttgcgtattggaggcgtgtgttcctatattttttaggctcaattatgaatgaaattattctcagcgagcatataaccgttttcgaggtaaaatgaactaaaagcatatgggcctgcctgttcgcataagtacaccctccgtctaaaaaagaataaaaatatcatttcttgatgagtcaaaaaagttcaaatttaagaaaatatatgttacgacaccaatatttataatgtgtaataagtactgctgattaattttaaaataaaattttcataataaacctatttgaagatacaagtattggtactatttctaataaatctaatcaaactggtgttatatcttttgtaacaaatttgtgctttgtgtttctggttgacgtgaatcagcttaatcttgctgaaatctaacattgtcttttgttcgttggcatacaggatcaaaaaggaaagaagcatctattgttggtaagagcctatagtcaatacccatgttcatttcgtctaaaagagcagaagaaaagcatatgatgaattattgccatgtcatgtttaaaatacagaattctcaaaaacaaaaacaaaaaaaacttggaatccactaaccagtaaccactgatagcattgtagaaaatttcatcctccctttgggcaatacactgatgagtttacatgctgactagtggtgcatttgttctttgccaattgaatttttagaatgctttgcagctgaattcacttgtgatttttttttgtgatgcaggtgctgttgccgttgcattcctgtgtctagtcattctcacatgcttcttggcttgtagacatggttcgctgcccttcaaatcggagaacaaaccagggacaaggattgagtccttcctacagaagaacgagagtatacatccgaaaagatacacctacacggacgtgaaaagaatgacaaaatccttcgctgtgaagctaggccaaggtgggtttggtgctgtatacaaaggcagcctccacgatggccgacaggtagcagtcaagatgctcaaggacacccaaggtgacggcgaggaattcatgaacgaggtggctagcatcagcaggacttctcatgtcaacgtcgtgacacttctagggttttgcttgcaagggtcgaaaagagcactgatctacgagtacatgcccaatggttcgctcgaaaggtatgccttcaccggtgacatgaacagtgagaatttgctaacctgggaaaggctatttgacatagcaattggcacggccagagggctcgaatacctacaccggggatgcaacactcggatcgtgcattttgacatcaagccacacaacatcctgttagaccaggatttctgtcctaagatctctgactttggactggccaagctatgtctgaacaaagagagcgctatctccattgttggcgcaagagggacgatagggtatatcgccccggaggtctactcaaagcaatttggaacaatcagcagcaagtctgatgtctatagctatgggatgatggtccttgagatggttggagcaagggaaaggaatacaagcgcaagcgcagatagtgaccatagcagccaatatttccctcagtggatttatgaacatttggacgactattgtgttggtgcttccgagattaatggtgagaccacagagctcgtgaggaagatgatagttgtaggtctgtggtgcatacaagtgattccgactgatcgaccaacaatgacgagagtcgtcgagatgttggaagggagcacgagtaatctagagttgccacccagagttctcttgagctgacaaagcgtagatatttttcctatcaaatgttgcttccaggtcacacaaatgcaaaatatttgtggagacgagtgcctatttacctcatacactgtatctgtatgacaaaagtcccacgactcactggacgcggaaatgtcgcttgactacgccaattttctaaaaagattggcagcaattaatggaggcttatagcggtaactttggttcgcattaatcctaggactagggttgaatatcgatctaactcgacgcggcttggtcaagctcaagctagctccactcatctcattaaagaatccagctagaaaatcaacccaagtcgtttacgaaacgagtttgagctgactcgtttagatcgtaaatcacaacaaaaacaatatgcacatatatacaataatataatcaatactagttaattctagactagtttaacactagaaaagagtaatgatactcataatttcacatacaatgtcaatccaacaccaatttaacacacttcatcacttattagttcatccaaccaagtgtaggctttgatttactaacaaatggttgctcgttcgagctagcgagcttgcttgttaacaaactgagttgagatgctagcttaacttgtgacaaaattaaaacgagccgagtcgagtcaagttgagctcacgatgagtcgagcaagctcacaatccacgagtatttttttagtcctatctaagactaaagtttaatcctaaaactaaattttaatctctatttgtttggttctataaactaaacaggttcagaaaacataaaatacattatagaaaacctgaaatacccttctatacttaaggcatcactaagagagagcaataaataaagggtagagagaggaataaatctgctttattcccttttagctaccctttgagagagtaaacactaaaatgaaaggatccttgaggattttgatgttttggatgacaactaacacaattaaaggtctaattaggatgttaaatgaggagcaatcattgttcaagacatgatgcaaagctagaaaactttgattgtggccgtcctaattgtgaagtttaggccggggggaacttcatgaaccctatcgaagcttaattagttcttttttgttgttagccatgtttgtattgtagtttaggtgaacaacatgacgccgcacccgcgatctcagggctcgtccccacacaggagggcacgtcgtcgtcttcgccgccgagcatcagagattcagagcacgtacacgcacatctcaagcaaacggagtagtacgtcctactcctacgtacatacctagccgacgacctttatgtgcacaccaccactgctctgctgcccggcctctccgtcgtccgttcatcaccagctggtctggtccttcaatttccatgcgtcggtccg

SEQ ID NO: 79 - DNA, 7154 bp, synthetic construct
  misc_feature 1..7154: note = CTL1-TS10 DNA repair template
  source 1..7154: mol_type = other DNA
aaatagtaaacgggaggggaggtcgctagtagtaaacgctaggtagctaggataatccgtctcgtgttggacggaaggttttggacgcatctgcgtgcacagcccgctgatacagatctgatcgactagctagctagatgccgaggccccagagcaaggcccggatactcctgcacagtccctgagatttcagcacagcaggtgctgttgcatcaatatataaatccctgctttattaatttaatctctgtgcatgtatccatacatcgtcagcggctcagcgctatcacactgcagtgcacgcagctagttgagcgcctgggtcagtatatatatagctagtagggacaaaggggggcactgtacgttggtttggtttggcacgcacgcgatcgagagtggtggaatggactgcagatcatcgatcgctgcactgtacgcacgcgcaccggactgcatttgcatgcccctgaaggaggaaaggggaaggaaagaaaagaaataggagaaagaagaagaagcagagaaatacgtcacagtccaagaagagtgagccgccctagctagcttcaaccctgacgaacccggcagccacacttccggccatgtatgcatgcatgcatggcttagcttcagatgtccaatcgaatccatcaagacctggccggttttccatggccgcctcgccttcgctagttaagggccaagtacttgctgtccctgtgatattgaatccaattcaattctataacctccaaaatcgatatcctaacatagcatgatagtttttttgagaggtgtgatttaacatattagatgaattttctttttttaatacgctatgttctagatgtctgacgatgaatggagccgctctgcatataccaaacgctatctaagtttgtgaacaaatgactaaattatccacacgaccacaattgggcgctgataagatccacacttgctggttttaattcatccggtctttatcaactgtcacatcagttatagatcattatcaacttttatctacaattgatgttgtaatacacggtcacttaagaccatgtttaggtacaatgtctctcaaaactatgattttacttatgatgacaataccgtagttttgaatagctctaaaaatatcatggttctaaaaatattgtttggattcaacattataaatcgtggtattaagcaaaagctagtcatgttataaaaactttaggttgaagtagagttttcaatactaaaaaaatatcatggtatttagaatatcatgattttaaaaatatagttcttacgaatgcaaccaaacaccttatgatataaaataatatggtattgcctacaaactacaaaaataaatcactcccaagcattacataaacatcatttttataaactttttagtaaaataaagcgcaatgtttttattaaatagaaatttatacaagtatatataattaagcaaataaaaactacgttattcataaaaagctaataaaaagtaaaaagtaaaaactatataattcataaaaaaatcgttatctttctcttccatcttattatctatttttagttgttttgtcaaatttaaggctattttatgggttctttttatctttgtacatgtcgtgagccaataacttattgaattggtcaatcaatttaggttgagttttacttttaactaacctagtatagtttgttcaacacctttttttcataatcggggactcattccacttgttgttgacccattttttcttctactgagttcttgcccttttgcaatcaataggacgtggtgagcccatatttttaggtgttatggatttataatcaccgttcaaatttgaatgaatattttgtttttattattgaagtcttcgtcaatcgttatcatgcctcgcataccacttagaccgacgaagtccaacatatttctcccccgacgaggagagattcttcgtaaaattgctactggtattactggtattgaatagaagataagggtgcgtttggttgcatgcatctacgcgtgcttgcatcacggaatgcgggttggtgctgtttggttgctataagctagactatacatatgcaagttttgtgtttggttggctgcatgcagatttcgatccaaactcgcacgatccacacagcaccctgggccaggcttaccagatacgagtagattggtcgcatctttggagccaggctttagcggtccgcggtcctggctgacacggccagattgccgagagaaaccaaccaaacagggtctaaatgtccaatcgtttgactgctactggatgaaaaaagaatgtcacaactttaaaatgtgtatttatttatactcctacacatgaaataactactatactcagatttcttttacattcagattttttctcagccactgaaacataccagccctttactaccaaaaacaggaactccacggtccaatgattatgtgagtcggaggagaggggaggaagaatcgcctgtgaaggagggagggagggagggacgtccgatccgaagatggaaggagctggggaggggagcgccttgacggggatgatgggtcctgcgctcgacaagctcgctagcctcgttgacaagtacaccgagctcagaaacgtgaggaagaagatggagcagctgaggaaggagctgattgcgatcaacctcgcgcttgagaagcacgcggccatggagaacccagacgcgcaggcgaaggcgtgggcggcggagatgcgcgagctggcctacgacatggaggacagcatcgatctcttcacccaccacgtcgaccacgaaccggccgacaccgccaccaccggcgtcaagaggttcttcctccggatcatccggaagcttaagaaactccactaccgccacaggtttgttcaggagatcaaacaactccacgaccttgccaacgaatcgtaccggcgtaggaagaggtacaggattgaggagggcggttcaagcctctcgcacgcggagatcgatcctcggttagaggcgctctacgtggaggtggagaaactcgtgggcatccagggcccaagccaggagatcattggacagctcgtcggcgagaacgcagcggagcgacggagggttgtcgccgttgttggatctggaggttcaggcaagaccacacttgccaaacaggtgtacgagaaaatcaggtgccaattctcttgtgcagcctttgtgtctgtgtcgcaaaagcccaacatgaatagcctcctgtgggagttgctatctcaaatcgggaaccatggtggagatttaggaatgatggcagtaggatattgcagtgacaaacaactgatcgacagactaagatcacatcttgaaaagcagaggttagtttaccttttcattccggttagcttaattcggtacaccaactagagatttgtgatttgctattaattacaccaaatttctcctacacaacaataactggtttagcatgatggcgatccaaagtcaaaactatcttctactactagtgtatgccatactcatatagatattttcttttcataaactctcgtagcatttttacatgcattcatattcctattgcctttatacagaactgatttttcactgcttcacaatctgctcttaggtatctcgttgtgatagatgatgtttggacaaactcagcgtgggagaccatacaatgtgcgctccctaaaaatgcccatgcaagtaaaataattctgacaacacgaatcaacagtgtaggccagttctcctgcactccagatgagggttttatctatcagatgaagcctctttgcagaaacgattctgaaaatctgtttctgaaaaggacactatgtgataaagataagtttcctgctcagctggaggggattaaaaacgagataatcgagaaatgcgatggtttgccactggctattgttactctagctagcatgttagctactaaacagagaacaagggaagaatgggagagggcacttgattcaatccattctatgcacaagaaagatagtggcctggaagtgatggacaagatactgtctctgagttacagggatctacctcacaacatgagaaattgcttgctgtatctcagtacatttccagaggaccacacgatttacaaagatgccctagtatggagatggatggctgaagggtttatcgctgaaacacaaggctttactttggagcaggttgccgagggctacttctacgagtttgtgaacaggagtttggttcagcccataaccttgcgttcaagatatgaaatgcgtggagaaggaggttgccgagtccatgacattgtactgaacttcctcatctctcgtgcagctgaagagaactttttaactacgctgtatggcgcccagggggttccatcttcagaccgaaggattcgccggctctctgtctgggacagtccagaacacgcactggcagtctctagagcgaccatgaatctgtcccatctccggtcagttagaatatgcaacgttggagactggcccgtgcctgctgttctagacttacctgtccttcgagtgttagatctagagggatgccgtgatctgaggatcgacgaacctgactgcattctaagcttgtttcatctgagatacctgggtttccgcagcgcaagtggtgtcgtgctaccggctcaaatcggaaatttacaccatctgcagaccatcgatttaagcgggactggagtgacacagctgccagaaagcattgtccagctcaagcgactgatgcatcttgttgggcaacggctcatcatgccagacgggtttggtagcatggaatcccttgaggagttaggtactatcgactgctgcaagtgccccgtcagttttggggaagacctagcacttctgagcaggctgagggtgctccgagtggctttcatcggggtcgaaacaagtgacatggaaaccagaaggaaatctttgatgtcatccctctgcaaactcggaggagacaaccttcggcgtgtcactattatcgacctcgctggcggtggagattgctttgtggagtcgtggcaccctcctcctcgtctcctccagaagttcatccatatcagtcagcaacagcacttctccaggtttccagaatggatcagttcctgcctatgtgatctcacccacctggatataaaggccgaaaagatggaaagggagcatctaagtgttcttgaacacctgcccgccatccgttgcctataccttttcgtgaagcgagtctccgaagacgggctcgccatcagccacggcgcgttccgatgtctacggcgtctcgagttctgcaacgtagatggacctggtttgatgtttgcaggaggcgttccaatgttggaatggctgaggctcgggttcgacgcggatagagcgcaatcgacatacggcggtctggaggttggcatccagcgcctctcgtctctcaaacatgtcgtgctcattgtatggatggtttctgaaggcggtgatgatccagcggagcaagccgtctggtctgccatcaatggccaagtagagatgctccccaactctccgacggttgatatccggtttcgtagacggagtcagctgcaggcaagctcagaataaggagcacgaaaaagacgatgatgttggatgtcgcctgctagctgtagtatgttgctgcttctgcttgttgccaacacattttttttgggttagggtggggtacaaccataaaatgtgtgtggatgtgcttgtaagcattacttgtatgtttttttttgtaaagcacaatatagatagatgcatatatgtgtgcgtgcaaagctatgattatcgacactcacacttgtacattagctagatgaaggtctcgacagagcagagcatagtacacatctctgggagttggactggacactataacggggatgctgcagccgaaactcaaaagctacatgcatgtcacttggctcatcggcgcaggaagcaacgcaggtccatcacgcgcagcaccttgaacccgtccaggctacaccccagcagcagcctcggcttcttcggcgccggcgggcagcgcggggggcgttcggttccagcgccactcgccgtcgccgacgacagcggcgagagctgccgtggaccttcttcgtcctcgtcgccgccgcgggagtaagaccgcttcagcttcagcggccgcagctccaccagctgcggaatgctaacatcttcttcaggcacctgccgggtggttctctttcccagaatcttccgctggagacccatggcgagctcggttcggtttaacctgcaattaatgcgcaatagcggagtaggaagcgagattgttagctcaggcgagcagagatgaaccggctaggaaagtttagttgctcgtgcatgctaccagctagcttgttggaggctcttgctttggacaccaagcaacggatatgacagcagaatgtgcgtgcttataagcaagcaagcagagcagcagttgcaaagaagggaaaaggtggagtggaaaaaggagttgccattgaagtgcacgagtgagcgagcatcatgtcaaggaaccaggagggaagttgcacaacagatgaaaagcggagagctgtttccgatctccaacacgagccttgattcctgccggccggtgatggcaatggccgctagtagtctccgctagctagggagcggcgatccgacgcgacgccaccatgtgtctagaaaagaagtttcttgctttgcatgcagacttattagcgcggtcgacacctgtggggaccccgtgtcttgagacaatgagactgcctgtccgcccaagacactacttgtagccatgaagccatcgactcctctccttgctctccagtaatccagtggatggatccatcatcgatagtttagtttatcagtcttcttgaggccggtgtcccccatgcataatgatgacagaaagcctgggccaggtaaaagccaaaaagtttgaccctctaggtactggggccagccctggcgtttgaacaaaaaaaaaatctgagcgtgtcgccccggcctgttttcgaactcctaaacgacgtcgcaactttttttatacacacactaccggtacatggcttt

SEQ ID NO: 80 - protein, 18 aa, Agrobacterium tumefaciens
KRPRDRHDGELGGRKRAR

SEQ ID NO: 81 - DNA, 341 bp, Zea mays
  source 1..341: mol_type = genomic DNA
ttgtgaggtctattaaggcatgtttggttttggaccctagttgtatagaatggcttcgttcgaggcctccaacttatgagaatgaaatgactcgtttgaaagatagaatgactttggtccattgtgagccaaaaggtttgataacccgtttggatgtagatattggagcactaaattggaaatttgaatcaatttttctgaattctattgtttggttgcacatggaattgagattagaaattagatattcaatttcagggaattggtaaattctctctcaatatatagcatcatccctttgaattgcgtttaactagaccacataattctaaactccaatc

SEQ ID NO: 82 - DNA, 276 bp, Zea mays
  source 1..276: mol_type = genomic DNA
ctgatcacgtgagcagcagctagccaaagtgaaggtgaaagaggaataaaggaaaaagaggacgacgagaaaagcacagctttgtctttgttgaaaaggaaacaataaaaaaacacaaagaaaaacacggggaatgtgcaaaaggaagccttatttggctggatgcgttcttgagtgcactgttttggagggaatgagaataccaagggcttgttcggttaggggtggattgaggaggacaaaccccttcaaaccgaacaaaccctaataggggtg

SEQ ID NO: 83 - DNA, 403 bp, Zea mays
  source 1..403: mol_type = genomic DNA
gaagactgggttgtgaggtctattaaggcatgtttggttttggaccctagttgtatagaatggcttcgttcgaggcctccaacttatgagaatgaaatgactcgtttgaaagatagaatgactttggtccattgtgagccaaaaggtttgataacccgtttggatgtagatattggagcactaaattggaaatttgaatcaatttttctgaattctattgtttggttgcacatggaattgagattagaaattagatattcaatttcagggaattggtaaattctctctcaatatatagcatcatccctttgaattgcgtttaactagaccacataattctaaactccaatcatgtgacatccaaacaatataattaaaatgtctgacgatgaatgagccgctc

SEQ ID NO: 84 - DNA, 368 bp, Zea mays
  source 1..368: mol_type = genomic DNA
actaggcgatcttctttccgtaacacagcatatgatgaaaacggaacgatgaaagcgccatttgagaggggaggggagggaaaatgccttggctgatcacgtgagcagcagctagccaaagtgaaggtgaaagaggaataaaggaaaaagaggacgacgagaaaagcacagctttgtctttgttgaaaaggaaacaataaaaaaacacaaagaaaaacacggggaatgtgcaaaaggaagccttatttggctggatgcgttcttgagtgcactgttttggagggaatgagaataccaagggcttgttcggttaggggtggattgaggaggacaaaccccttcaaaccgaacaaaccctaataggggtg

SEQ ID NO: 85 - DNA, 481 bp, Zea mays
  source 1..481: mol_type = genomic DNA
cagaatttacggtccagcacgggcatgccgcgcgggctgactttgctccactgactcgatcatgtgcggattccatcgcggcgtagcgtagccaaccgcaacgcaaaccgacttcatcttttttttttattatgaacaaaaggagatcgagagaaacgtgaacggtaaataatatatctgatcccatgcatgcacgctgcctgggtcgatctcgctctcgctccgcccagacgaacatgcatgctggtcaggctcaacgctcaggcgggcaagctgtgggaggacatgggatgggagaggaggacacatgcatgctggccagtcaggcactgtgctggcacatgaggtagggataggggggccctcggccagtgtccaggccgcatgcatgcatgccccccctgctgctcgaccgaacaacgttggatgcctggattgatgcaacagtttggacggacggaccatacgttatgtaccagta

SEQ ID NO: 86 - DNA, 486 bp, Zea mays
  source 1..486: mol_type = genomic DNA
ctgcacgttacgtacgtacgaactaatatactccaccagctgatcactgatgagccgagccgccatgcattgtaatttataacatgtgcggctgtacgcttccatctcaaatacctttttatatatatattgtactttatagtctacgacataatctgccatggtaatttataagatgtgctttattgctcgttgttctgttctcatctgtgtccatggcatggcatggatacaaaatgtatgtatggccacgcatccaatctgtgacgttgtcaaggcagaggtccaaccgtccaagaccctcttgtgccgccctgtacttgcagtcagtgacgttgtgagaaaaagctgtgggtggtctccgcagagcgcgcgggccacgagagggagccccatctctcggccgaggggtacgggggctccagacacggtcctttggtttcttctgcctgtagcgagcggccccgccccccaccgcgctgctag

SEQ ID NO: 87 - DNA, 411 bp, Zea mays
  source 1..411: mol_type = genomic DNA
cggatagatggcgtctagcatatcgataggacatgacaagtggtacgatccccgtcacatgtccatggaggcatctgatatggacacggcgtgtatctatcgcggctggaacagaaccagcgctcgcgcggcggtcggcgggagggacagaccttggctccgtgcgttcaggttgtgcttgtgccgcgcgccacgcacggtctccgccgcctgcagctgaaattttagatttacatcctatccctttattttttttatttgtcacaattcagttcaaaaatgaagaacggaggtagtgcatcctttgtgagactaatgaaaatcacatctggatcctgaaatcggcgtcgtaacctacaaggccacggactggattagatagtggtccatggtgcataatgaggatcgagg

SEQ ID NO: 88 - DNA, 417 bp, Zea mays
  source 1..417: mol_type = genomic DNA
atgaggagcaatcattgttcaagacatgatgcaaagctagaaaactttgattgtggccgtcctaattgtgaagtttaggccggggggaacttcatgaaccctatcgaagcttaattagttcttttttgttgttagccatgtttgtattgtagtttaggtgaacaacatgacgccgcacccgcgatctcagggctcgtccccacacaggagggcacgtcgtcgtcttcgccgccgagcatcagagattcagagcacgtacacgcacatctcaagcaaacggagtagtacgtcctactcctacgtacatacctagccgacgacctttatgtgcacaccaccactgctctgctgcccggcctctccgtcgtccgttcatcaccagctggtctggtccttcaatttccatgcgtcggtccg

SEQ ID NO: 89 - DNA, 724 bp, Zea mays
  source 1..724: mol_type = genomic DNA
aaatagtaaacgggaggggaggtcgctagtagtaaacgctaggtagctaggataatccgtctcgtgttggacggaaggttttggacgcatctgcgtgcacagcccgctgatacagatctgatcgactagctagctagatgccgaggccccagagcaaggcccggatactcctgcacagtccctgagatttcagcacagcaggtgctgttgcatcaatatataaatccctgctttattaatttaatctctgtgcatgtatccatacatcgtcagcggctcagcgctatcacactgcagtgcacgcagctagttgagcgcctgggtcagtatatatatagctagtagggacaaaggggggcactgtacgttggtttggtttggcacgcacgcgatcgagagtggtggaatggactgcagatcatcgatcgctgcactgtacgcacgcgcaccggactgcatttgcatgcccctgaaggaggaaaggggaaggaaagaaaagaaataggagaaagaagaagaagcagagaaatacgtcacagtccaagaagagtgagccgccctagctagcttcaaccctgacgaacccggcagccacacttccggccatgtatgcatgcatgcatggcttagcttcagatgtccaatcgaatccatcaagacctggccggttttccatggccgcctcgccttcgctagttaagggccaagtacttgctgtccctgt

SEQ ID NO: 90 - DNA, 500 bp, Zea mays
  source 1..500: mol_type = genomic DNA
atctccaacacgagccttgattcctgccggccggtgatggcaatggccgctagtagtctccgctagctagggagcggcgatccgacgcgacgccaccatgtgtctagaaaagaagtttcttgctttgcatgcagacttattagcgcggtcgacacctgtggggaccccgtgtcttgagacaatgagactgcctgtccgcccaagacactacttgtagccatgaagccatcgactcctctccttgctctccagtaatccagtggatggatccatcatcgatagtttagtttatcagtcttcttgaggccggtgtcccccatgcataatgatgacagaaagcctgggccaggtaaaagccaaaaagtttgaccctctaggtactggggccagccctggcgtttgaacaaaaaaaaaatctgagcgtgtcgccccggcctgttttcgaactcctaaacgacgtcgcaactttttttatacacacactaccggtacatggcttt